European Patent Application EP 4 205 764 A1, published July 5, 2023. Title: Bispecific antibodies that bind to cleaved form of mutant CALR-CD3 , and Pharmaceutical composition. Applicant: JUNTENDO EDUCATIONAL FOUNDATION Meiji Seika Pharma Co. Ltd. The sequence listing filed with the application follows.

SEQUENCE LISTING (212 sequences)

SEQ ID NO: 1 - protein, 13 aa, Homo sapiens
RRMMRTKMRMRRM

SEQ ID NO: 2 - protein, 119 aa, Rattus norvegicus
QVQLQQSGAELVKPGSSVKISCKASGYTFTRNFIHWIKQQPGNGLEWIGWIFPGDGDTEYNQKFNGKATLTADKSSSTAYMQLSSLTSEDSAVYFCARGNYNYEYFDYWGQGVMVTVSS

SEQ ID NO: 3 - protein, 107 aa, Rattus norvegicus
DIQMTQSPASLSASLGETVSIECLASEDIYSYLAWYQQKPGKSPQLLIFAANRLQDGVPSRFSGSGSGTQFSLKISGMQPEDEGDYFCLQGSKFPYTFGPGTKLELN

SEQ ID NO: 4 - protein, 121 aa, Rattus norvegicus
QVQLQQSGAELVKPGSSVKISCKASGYTFTSYFVHWIKQQPGDGLEWIGWIYPGDGDTEYNHKFNGKSTLTADRSSSTAYMQLSSLTSEDSAVYFCARGNYYDGREVMDAWGQGASVTVSS

SEQ ID NO: 5 - protein, 112 aa, Rattus norvegicus
DVVLTQTPPTLSATIGQSVSISCRSSQSLLDSDGETYLNWLLQRPGQSPQLLIYSVSNLESGVPNRFSGSGSETDFTLKISGMEAEDLGVYYCMQATHGPYTFGAGTKLELK

SEQ ID NO: 6 - protein, 121 aa, Rattus norvegicus
QVQLQQSGAELVKPGSSVKISCKASGYTFTSYFVHWIKQQPGDGLEWIGWIYPGDGDTEYNQKFNGKATLTADRSSSTAYMQLSSLTSEDSAVYFCARGNYYDGREVMDAWGQGASVTVSS

SEQ ID NO: 7 - protein, 112 aa, Rattus norvegicus
DVVLTQTPPTLSATIGQSVSISCRSSQSLLDSDGETYLNWLLQRPGQCPQLLIYSVSNLESGVPNRFSGSGSETDFTLKISGVEAEDLGVYYCMQGTHGPYTFGAGTKLELK

SEQ ID NO: 8 - protein, 119 aa, Artificial Sequence
QVQLVQSGGGVVQPGRSLRLSCKASGYTFTRYTMHWVRQAPGKGLEWIGYINPSRGYTNYNQKVKDRFTISRDNSKNTAFLQMDSLRPEDTGVYFCARYYDDHYSLDYWGQGTPVTVSS

SEQ ID NO: 9 - protein, 107 aa, Artificial Sequence
DIQMTQSPSSLSASVGDRVTITCSASSSVSYMNWYQQTPGKAPKRWIYDTSKLASGVPSRFSGSGSGTDYTFTISSLQPEDIATYYCQQWSSNPFTFGQGTKLQITR

SEQ ID NO: 10 - protein, 10 aa, Rattus norvegicus
GYTFTRNFIH

SEQ ID NO: 11 - protein, 17 aa, Rattus norvegicus
WIFPGDGDTEYNQKFNG

SEQ ID NO: 12 - protein, 10 aa, Rattus norvegicus
GNYNYEYFDY

SEQ ID NO: 13 - protein, 11 aa, Rattus norvegicus
LASEDIYSYLA

SEQ ID NO: 14 - protein, 7 aa, Rattus norvegicus
AANRLQD

SEQ ID NO: 15 - protein, 9 aa, Rattus norvegicus
LQGSKFPYT

SEQ ID NO: 16 - protein, 10 aa, Rattus norvegicus
GYTFTSYFVH

SEQ ID NO: 17 - protein, 17 aa, Rattus norvegicus
WIYPGDGDTEYNHKFNG

SEQ ID NO: 18 - protein, 12 aa, Rattus norvegicus
GNYYDGREVMDA

SEQ ID NO: 19 - protein, 16 aa, Rattus norvegicus
RSSQSLLDSDGETYLN

SEQ ID NO: 20 - protein, 7 aa, Rattus norvegicus
SVSNLES

SEQ ID NO: 21 - protein, 9 aa, Rattus norvegicus
MQATHGPYT

SEQ ID NO: 22 - protein, 10 aa, Rattus norvegicus
GYTFTSYFVH

SEQ ID NO: 23 - protein, 17 aa, Rattus norvegicus
WIYPGDGDTEYNQKFNG

SEQ ID NO: 24 - protein, 12 aa, Rattus norvegicus
GNYYDGREVMDA

SEQ ID NO: 25 - protein, 16 aa, Rattus norvegicus
RSSQSLLDSDGETYLN

SEQ ID NO: 26 - protein, 7 aa, Rattus norvegicus
SVSNLES

SEQ ID NO: 27 - protein, 9 aa, Rattus norvegicus
MQGTHGPYT

SEQ ID NO: 28 - protein, 5 aa, Mus musculus
RYTMH

SEQ ID NO: 29 - protein, 17 aa, Mus musculus
YINPSRGYTNYNQKVKD

SEQ ID NO: 30 - protein, 10 aa, Mus musculus
YYDDHYSLDY

SEQ ID NO: 31 - protein, 10 aa, Mus musculus
SASSSVSYMN

SEQ ID NO: 32 - protein, 7 aa, Mus musculus
DTSKLAS

SEQ ID NO: 33 - protein, 9 aa, Mus musculus
QQWSSNPFT

SEQ ID NO: 34 - protein, 714 aa, Artificial Sequence
QVQLQQSGAELVKPGSSVKISCKASGYTFTRNFIHWIKQQPGNGLEWIGWIFPGDGDTEYNQKFNGKATLTADKSSSTAYMQLSSLTSEDSAVYFCARGNYNYEYFDYWGQGVMVTVSSGGGGSGGGGSGGGGSDIQMTQSPASLSASLGETVSIECLASEDIYSYLAWYQQKPGKSPQLLIFAANRLQDGVPSRFSGSGSGTQFSLKISGMQPEDEGDYFCLQGSKFPYTFGPGTKLELNGGGGSQVQLVQSGGGVVQPGRSLRLSCKASGYTFTRYTMHWVRQAPGKGLEWIGYINPSRGYTNYNQKVKDRFTISRDNSKNTAFLQMDSLRPEDTGVYFCARYYDDHYSLDYWGQGTPVTVSSGGGGSGGGGSGGGGSDIQMTQSPSSLSASVGDRVTITCSASSSVSYMNWYQQTPGKAPKRWIYDTSKLASGVPSRFSGSGSGTDYTFTISSLQPEDIATYYCQQWSSNPFTFGQGTKLQITRDKTHTCPPCPAPEAAGGPSVFLFPPKPKDTLMISRTPEVTCVVVDVSHEDPEVKFNWYVDGVEVHNAKTKPREEQYNSTYRVVSVLTVLHQDWLNGKEYKCKVSNKALPAPIEKTISKAKGQPREPQVYTLPPSRDELTKNQVSLTCLVKGFYPSDIAVEWESNGQPENNYKTTPPVLDSDGSFFLYSKLTVDKSRWQQGNVFSCSVMHEALHNHYTQKSLSLSPGK

SEQ ID NO: 35 - protein, 722 aa, Artificial Sequence
DIQMTQSPASLSASLGETVSIECLASEDIYSYLAWYQQKPGKSPQLLIFAANRLQDGVPSRFSGSGSGTQFSLKISGMQPEDEGDYFCLQGSKFPYTFGPGTKLELNGGGGSGGGGSGGGGSQVQLQQSGAELVKPGSSVKISCKASGYTFTRNFIHWIKQQPGNGLEWIGWIFPGDGDTEYNQKFNGKATLTADKSSSTAYMQLSSLTSEDSAVYFCARGNYNYEYFDYWGQGVMVTVSSGGGGSQVQLVQSGGGVVQPGRSLRLSCKASGYTFTRYTMHWVRQAPGKGLEWIGYINPSRGYTNYNQKVKDRFTISRDNSKNTAFLQMDSLRPEDTGVYFCARYYDDHYSLDYWGQGTPVTVSSGGGGSGGGGSGGGGSDIQMTQSPSSLSASVGDRVTITCSASSSVSYMNWYQQTPGKAPKRWIYDTSKLASGVPSRFSGSGSGTDYTFTISSLQPEDIATYYCQQWSSNPFTFGQGTKLQITRLEVLFQGPDKTHTCPPCPAPELLGGPSVFLFPPKPKDTLMISRTPEVTCVVVDVSHEDPEVKFNWYVDGVEVHNAKTKPREEQYNSTYRVVSVLTVLHQDWLNGKEYKCKVSNKALPAPIEKTISKAKGQPREPQVYTLPPSRDELTKNQVSLTCLVKGFYPSDIAVEWESNGQPENNYKTTPPVLDSDGSFFLYSKLTVDKSRWQQGNVFSCSVMHEALHNHYTQKSLSLSPGK

SEQ ID NO: 36 - protein, 714 aa, Artificial Sequence
QVQLVQSGGGVVQPGRSLRLSCKASGYTFTRYTMHWVRQAPGKGLEWIGYINPSRGYTNYNQKVKDRFTISRDNSKNTAFLQMDSLRPEDTGVYFCARYYDDHYSLDYWGQGTPVTVSSGGGGSGGGGSGGGGSDIQMTQSPSSLSASVGDRVTITCSASSSVSYMNWYQQTPGKAPKRWIYDTSKLASGVPSRFSGSGSGTDYTFTISSLQPEDIATYYCQQWSSNPFTFGQGTKLQITRGGGGSQVQLQQSGAELVKPGSSVKISCKASGYTFTRNFIHWIKQQPGNGLEWIGWIFPGDGDTEYNQKFNGKATLTADKSSSTAYMQLSSLTSEDSAVYFCARGNYNYEYFDYWGQGVMVTVSSGGGGSGGGGSGGGGSDIQMTQSPASLSASLGETVSIECLASEDIYSYLAWYQQKPGKSPQLLIFAANRLQDGVPSRFSGSGSGTQFSLKISGMQPEDEGDYFCLQGSKFPYTFGPGTKLELNDKTHTCPPCPAPEAAGGPSVFLFPPKPKDTLMISRTPEVTCVVVDVSHEDPEVKFNWYVDGVEVHNAKTKPREEQYNSTYRVVSVLTVLHQDWLNGKEYKCKVSNKALPAPIEKTISKAKGQPREPQVYTLPPSRDELTKNQVSLTCLVKGFYPSDIAVEWESNGQPENNYKTTPPVLDSDGSFFLYSKLTVDKSRWQQGNVFSCSVMHEALHNHYTQKSLSLSPGK

SEQ ID NO: 37 - protein, 714 aa, Artificial Sequence
QVQLVQSGGGVVQPGRSLRLSCKASGYTFTRYTMHWVRQAPGKGLEWIGYINPSRGYTNYNQKVKDRFTISRDNSKNTAFLQMDSLRPEDTGVYFCARYYDDHYSLDYWGQGTPVTVSSGGGGSGGGGSGGGGSDIQMTQSPSSLSASVGDRVTITCSASSSVSYMNWYQQTPGKAPKRWIYDTSKLASGVPSRFSGSGSGTDYTFTISSLQPEDIATYYCQQWSSNPFTFGQGTKLQITRGGGGSDIQMTQSPASLSASLGETVSIECLASEDIYSYLAWYQQKPGKSPQLLIFAANRLQDGVPSRFSGSGSGTQFSLKISGMQPEDEGDYFCLQGSKFPYTFGPGTKLELNGGGGSGGGGSGGGGSQVQLQQSGAELVKPGSSVKISCKASGYTFTRNFIHWIKQQPGNGLEWIGWIFPGDGDTEYNQKFNGKATLTADKSSSTAYMQLSSLTSEDSAVYFCARGNYNYEYFDYWGQGVMVTVSSDKTHTCPPCPAPEAAGGPSVFLFPPKPKDTLMISRTPEVTCVVVDVSHEDPEVKFNWYVDGVEVHNAKTKPREEQYNSTYRVVSVLTVLHQDWLNGKEYKCKVSNKALPAPIEKTISKAKGQPREPQVYTLPPSRDELTKNQVSLTCLVKGFYPSDIAVEWESNGQPENNYKTTPPVLDSDGSFFLYSKLTVDKSRWQQGNVFSCSVMHEALHNHYTQKSLSLSPGK

SEQ ID NO: 38 - protein, 717 aa, Artificial Sequence
QVQLVQSGGGVVQPGRSLRLSCKASGYTFTRYTMHWVRQAPGKGLEWIGYINPSRGYTNYNQKVKDRFTISRDNSKNTAFLQMDSLRPEDTGVYFCARYYDDHYSLDYWGQGTPVTVSSGGGGSDIQMTQSPASLSASLGETVSIECLASEDIYSYLAWYQQKPGKSPQLLIFAANRLQDGVPSRFSGSGSGTQFSLKISGMQPEDEGDYFCLQGSKFPYTFGPGTKLELNGGGGSGGGGSGGGGSGGGGSQVQLQQSGAELVKPGSSVKISCKASGYTFTRNFIHWIKQQPGNGLEWIGWIFPGDGDTEYNQKFNGKATLTADKSSSTAYMQLSSLTSEDSAVYFCARGNYNYEYFDYWGQGVMVTVSSGGGGSDIQMTQSPSSLSASVGDRVTITCSASSSVSYMNWYQQTPGKAPKRWIYDTSKLASGVPSRFSGSGSGTDYTFTISSLQPEDIATYYCQQWSSNPFTFGQGTKLQITRLEVLFQGPDKTHTCPPCPAPEAAGGPSVFLFPPKPKDTLMISRTPEVTCVVVDVSHEDPEVKFNWYVDGVEVHNAKTKPREEQYNSTYRVVSVLTVLHQDWLNGKEYKCKVSNKALPAPIEKTISKAKGQPREPQVYTLPPSRDELTKNQVSLTCLVKGFYPSDIAVEWESNGQPENNYKTTPPVLDSDGSFFLYSKLTVDKSRWQQGNVFSCSVMHEALHNHYTQKSLSLSPGK

SEQ ID NO: 39 - protein, 709 aa, Artificial Sequence
DIQMTQSPSSLSASVGDRVTITCSASSSVSYMNWYQQTPGKAPKRWIYDTSKLASGVPSRFSGSGSGTDYTFTISSLQPEDIATYYCQQWSSNPFTFGQGTKLQITRGGGGSQVQLQQSGAELVKPGSSVKISCKASGYTFTRNFIHWIKQQPGNGLEWIGWIFPGDGDTEYNQKFNGKATLTADKSSSTAYMQLSSLTSEDSAVYFCARGNYNYEYFDYWGQGVMVTVSSGGGGSGGGGSGGGGSGGGGSDIQMTQSPASLSASLGETVSIECLASEDIYSYLAWYQQKPGKSPQLLIFAANRLQDGVPSRFSGSGSGTQFSLKISGMQPEDEGDYFCLQGSKFPYTFGPGTKLELNGGGGSQVQLVQSGGGVVQPGRSLRLSCKASGYTFTRYTMHWVRQAPGKGLEWIGYINPSRGYTNYNQKVKDRFTISRDNSKNTAFLQMDSLRPEDTGVYFCARYYDDHYSLDYWGQGTPVTVSSDKTHTCPPCPAPEAAGGPSVFLFPPKPKDTLMISRTPEVTCVVVDVSHEDPEVKFNWYVDGVEVHNAKTKPREEQYNSTYRVVSVLTVLHQDWLNGKEYKCKVSNKALPAPIEKTISKAKGQPREPQVYTLPPSRDELTKNQVSLTCLVKGFYPSDIAVEWESNGQPENNYKTTPPVLDSDGSFFLYSKLTVDKSRWQQGNVFSCSVMHEALHNHYTQKSLSLSPGK

SEQ ID NO: 40 - protein, 709 aa, Artificial Sequence
QVQLQQSGAELVKPGSSVKISCKASGYTFTRNFIHWIKQQPGNGLEWIGWIFPGDGDTEYNQKFNGKATLTADKSSSTAYMQLSSLTSEDSAVYFCARGNYNYEYFDYWGQGVMVTVSSGGGGSDIQMTQSPSSLSASVGDRVTITCSASSSVSYMNWYQQTPGKAPKRWIYDTSKLASGVPSRFSGSGSGTDYTFTISSLQPEDIATYYCQQWSSNPFTFGQGTKLQITRGGGGSGGGGSGGGGSGGGGSQVQLVQSGGGVVQPGRSLRLSCKASGYTFTRYTMHWVRQAPGKGLEWIGYINPSRGYTNYNQKVKDRFTISRDNSKNTAFLQMDSLRPEDTGVYFCARYYDDHYSLDYWGQGTPVTVSSGGGGSDIQMTQSPASLSASLGETVSIECLASEDIYSYLAWYQQKPGKSPQLLIFAANRLQDGVPSRFSGSGSGTQFSLKISGMQPEDEGDYFCLQGSKFPYTFGPGTKLELNDKTHTCPPCPAPEAAGGPSVFLFPPKPKDTLMISRTPEVTCVVVDVSHEDPEVKFNWYVDGVEVHNAKTKPREEQYNSTYRVVSVLTVLHQDWLNGKEYKCKVSNKALPAPIEKTISKAKGQPREPQVYTLPPSRDELTKNQVSLTCLVKGFYPSDIAVEWESNGQPENNYKTTPPVLDSDGSFFLYSKLTVDKSRWQQGNVFSCSVMHEALHNHYTQKSLSLSPGK

SEQ ID NO: 41 - protein, 717 aa, Artificial Sequence
DIQMTQSPASLSASLGETVSIECLASEDIYSYLAWYQQKPGKSPQLLIFAANRLQDGVPSRFSGSGSGTQFSLKISGMQPEDEGDYFCLQGSKFPYTFGPGTKLELNGGGGSQVQLVQSGGGVVQPGRSLRLSCKASGYTFTRYTMHWVRQAPGKGLEWIGYINPSRGYTNYNQKVKDRFTISRDNSKNTAFLQMDSLRPEDTGVYFCARYYDDHYSLDYWGQGTPVTVSSGGGGSGGGGSGGGGSGGGGSDIQMTQSPSSLSASVGDRVTITCSASSSVSYMNWYQQTPGKAPKRWIYDTSKLASGVPSRFSGSGSGTDYTFTISSLQPEDIATYYCQQWSSNPFTFGQGTKLQITRGGGGSQVQLQQSGAELVKPGSSVKISCKASGYTFTRNFIHWIKQQPGNGLEWIGWIFPGDGDTEYNQKFNGKATLTADKSSSTAYMQLSSLTSEDSAVYFCARGNYNYEYFDYWGQGVMVTVSSLEVLFQGPDKTHTCPPCPAPEAAGGPSVFLFPPKPKDTLMISRTPEVTCVVVDVSHEDPEVKFNWYVDGVEVHNAKTKPREEQYNSTYRVVSVLTVLHQDWLNGKEYKCKVSNKALPAPIEKTISKAKGQPREPQVYTLPPSRDELTKNQVSLTCLVKGFYPSDIAVEWESNGQPENNYKTTPPVLDSDGSFFLYSKLTVDKSRWQQGNVFSCSVMHEALHNHYTQKSLSLSPGK

SEQ ID NO: 42 - protein, 493 aa, Artificial Sequence
QVQLQQSGAELVKPGSSVKISCKASGYTFTRNFIHWIKQQPGNGLEWIGWIFPGDGDTEYNQKFNGKATLTADKSSSTAYMQLSSLTSEDSAVYFCARGNYNYEYFDYWGQGVMVTVSSGGGGSGGGGSGGGGSDIQMTQSPASLSASLGETVSIECLASEDIYSYLAWYQQKPGKSPQLLIFAANRLQDGVPSRFSGSGSGTQFSLKISGMQPEDEGDYFCLQGSKFPYTFGPGTKLELNGGGGSQVQLVQSGGGVVQPGRSLRLSCKASGYTFTRYTMHWVRQAPGKGLEWIGYINPSRGYTNYNQKVKDRFTISRDNSKNTAFLQMDSLRPEDTGVYFCARYYDDHYSLDYWGQGTPVTVSSGGGGSGGGGSGGGGSDIQMTQSPSSLSASVGDRVTITCSASSSVSYMNWYQQTPGKAPKRWIYDTSKLASGVPSRFSGSGSGTDYTFTISSLQPEDIATYYCQQWSSNPFTFGQGTKLQITRHHHHHH

SEQ ID NO: 43 - protein, 493 aa, Artificial Sequence
DIQMTQSPASLSASLGETVSIECLASEDIYSYLAWYQQKPGKSPQLLIFAANRLQDGVPSRFSGSGSGTQFSLKISGMQPEDEGDYFCLQGSKFPYTFGPGTKLELNGGGGSGGGGSGGGGSQVQLQQSGAELVKPGSSVKISCKASGYTFTRNFIHWIKQQPGNGLEWIGWIFPGDGDTEYNQKFNGKATLTADKSSSTAYMQLSSLTSEDSAVYFCARGNYNYEYFDYWGQGVMVTVSSGGGGSQVQLVQSGGGVVQPGRSLRLSCKASGYTFTRYTMHWVRQAPGKGLEWIGYINPSRGYTNYNQKVKDRFTISRDNSKNTAFLQMDSLRPEDTGVYFCARYYDDHYSLDYWGQGTPVTVSSGGGGSGGGGSGGGGSDIQMTQSPSSLSASVGDRVTITCSASSSVSYMNWYQQTPGKAPKRWIYDTSKLASGVPSRFSGSGSGTDYTFTISSLQPEDIATYYCQQWSSNPFTFGQGTKLQITRHHHHHH

SEQ ID NO: 44 - protein, 493 aa, Artificial Sequence
QVQLVQSGGGVVQPGRSLRLSCKASGYTFTRYTMHWVRQAPGKGLEWIGYINPSRGYTNYNQKVKDRFTISRDNSKNTAFLQMDSLRPEDTGVYFCARYYDDHYSLDYWGQGTPVTVSSGGGGSGGGGSGGGGSDIQMTQSPSSLSASVGDRVTITCSASSSVSYMNWYQQTPGKAPKRWIYDTSKLASGVPSRFSGSGSGTDYTFTISSLQPEDIATYYCQQWSSNPFTFGQGTKLQITRGGGGSQVQLQQSGAELVKPGSSVKISCKASGYTFTRNFIHWIKQQPGNGLEWIGWIFPGDGDTEYNQKFNGKATLTADKSSSTAYMQLSSLTSEDSAVYFCARGNYNYEYFDYWGQGVMVTVSSGGGGSGGGGSGGGGSDIQMTQSPASLSASLGETVSIECLASEDIYSYLAWYQQKPGKSPQLLIFAANRLQDGVPSRFSGSGSGTQFSLKISGMQPEDEGDYFCLQGSKFPYTFGPGTKLELNHHHHHH

SEQ ID NO: 45 - protein, 493 aa, Artificial Sequence
QVQLVQSGGGVVQPGRSLRLSCKASGYTFTRYTMHWVRQAPGKGLEWIGYINPSRGYTNYNQKVKDRFTISRDNSKNTAFLQMDSLRPEDTGVYFCARYYDDHYSLDYWGQGTPVTVSSGGGGSGGGGSGGGGSDIQMTQSPSSLSASVGDRVTITCSASSSVSYMNWYQQTPGKAPKRWIYDTSKLASGVPSRFSGSGSGTDYTFTISSLQPEDIATYYCQQWSSNPFTFGQGTKLQITRGGGGSDIQMTQSPASLSASLGETVSIECLASEDIYSYLAWYQQKPGKSPQLLIFAANRLQDGVPSRFSGSGSGTQFSLKISGMQPEDEGDYFCLQGSKFPYTFGPGTKLELNGGGGSGGGGSGGGGSQVQLQQSGAELVKPGSSVKISCKASGYTFTRNFIHWIKQQPGNGLEWIGWIFPGDGDTEYNQKFNGKATLTADKSSSTAYMQLSSLTSEDSAVYFCARGNYNYEYFDYWGQGVMVTVSSHHHHHH

SEQ ID NO: 46 - protein, 449 aa, Artificial Sequence
QVQLQQSGAELVKPGSSVKISCKASGYTFTRNFIHWIKQQPGNGLEWIGWIFPGDGDTEYNQKFNGKATLTADKSSSTAYMQLSSLTSEDSAVYFCARGNYNYEYFDYWGQGVMVTVSSASTKGPSVFPLAPSSKSTSGGTAALGCLVKDYFPEPVTVSWNSGALTSGVHTFPAVLQSSGLYSLSSVVTVPSSSLGTQTYICNVNHKPSNTKVDKRVEPKSCDKTHTCPPCPAPEAAGGPSVFLFPPKPKDTLMISRTPEVTCVVVDVSHEDPEVKFNWYVDGVEVHNAKTKPREEQYNSTYRVVSVLTVLHQDWLNGKEYKCKVSNKALPAPIEKTISKAKGQPREPQVYTLPPCREEMTKNQVSLWCLVKGFYPSDIAVEWESNGQPENNYKTTPPVLDSDGSFFLYSKLTVDKSRWQQGNVFSCSVMHEALHNHYTQKSLSLSPGK

SEQ ID NO: 47 - protein, 695 aa, Artificial Sequence
QVQLQQSGAELVKPGSSVKISCKASGYTFTRNFIHWIKQQPGNGLEWIGWIFPGDGDTEYNQKFNGKATLTADKSSSTAYMQLSSLTSEDSAVYFCARGNYNYEYFDYWGQGVMVTVSSASTKGPSVFPLAPSSKSTSGGTAALGCLVKDYFPEPVTVSWNSGALTSGVHTFPAVLQSSGLYSLSSVVTVPSSSLGTQTYICNVNHKPSNTKVDKRVEPKSCDKTHTCPPCPAPEAAGGPSVFLFPPKPKDTLMISRTPEVTCVVVDVSHEDPEVKFNWYVDGVEVHNAKTKPREEQYNSTYRVVSVLTVLHQDWLNGKEYKCKVSNKALPAPIEKTISKAKGQPREPQVCTLPPSREEMTKNQVSLSCAVKGFYPSDIAVEWESNGQPENNYKTTPPVLDSDGSFFLVSKLTVDKSRWQQGNVFSCSVMHEALHNHYTQKSLSLSPGKGGGGSQVQLVQSGGGVVQPGRSLRLSCKASGYTFTRYTMHWVRQAPGKGLEWIGYINPSRGYTNYNQKVKDRFTISRDNSKNTAFLQMDSLRPEDTGVYFCARYYDDHYSLDYWGQGTPVTVSSGGGGSGGGGSGGGGSDIQMTQSPSSLSASVGDRVTITCSASSSVSYMNWYQQTPGKAPKRWIYDTSKLASGVPSRFSGSGSGTDYTFTISSLQPEDIATYYCQQWSSNPFTFGQGTKLQITR

SEQ ID NO: 48 - protein, 214 aa, Artificial Sequence
DIQMTQSPASLSASLGETVSIECLASEDIYSYLAWYQQKPGKSPQLLIFAANRLQDGVPSRFSGSGSGTQFSLKISGMQPEDEGDYFCLQGSKFPYTFGPGTKLELNRTVAAPSVFIFPPSDEQLKSGTASVVCLLNNFYPREAKVQWKVDNALQSGNSQESVTEQDSKDSTYSLSSTLTLSKADYEKHKVYACEVTHQGLSSPVTKSFNRGEC

SEQ ID NO: 49 - protein, 695 aa, Artificial Sequence
QVQLQQSGAELVKPGSSVKISCKASGYTFTRNFIHWIKQQPGNGLEWIGWIFPGDGDTEYNQKFNGKATLTADKSSSTAYMQLSSLTSEDSAVYFCARGNYNYEYFDYWGQGVMVTVSSASTKGPSVFPLAPSSKSTSGGTAALGCLVKDYFPEPVTVSWNSGALTSGVHTFPAVLQSSGLYSLSSVVTVPSSSLGTQTYICNVNHKPSNTKVDKRVEPKSCDKTHTCPPCPAPEAAGGPSVFLFPPKPKDTLMISRTPEVTCVVVDVSHEDPEVKFNWYVDGVEVHNAKTKPREEQYNSTYRVVSVLTVLHQDWLNGKEYKCKVSNKALPAPIEKTISKAKGQPREPQVYTLPPSREEMTKNQVSLTCLVKGFYPSDIAVEWESNGQPENNYKTTPPVLDSDGSFFLYSKLTVDKSRWQQGNVFSCSVMHEALHNHYTQKSLSLSPGKGGGGSQVQLVQSGGGVVQPGRSLRLSCKASGYTFTRYTMHWVRQAPGKGLEWIGYINPSRGYTNYNQKVKDRFTISRDNSKNTAFLQMDSLRPEDTGVYFCARYYDDHYSLDYWGQGTPVTVSSGGGGSGGGGSGGGGSDIQMTQSPSSLSASVGDRVTITCSASSSVSYMNWYQQTPGKAPKRWIYDTSKLASGVPSRFSGSGSGTDYTFTISSLQPEDIATYYCQQWSSNPFTFGQGTKLQITR

SEQ ID NO: 50 - protein, 473 aa, Artificial Sequence
QVQLVQSGGGVVQPGRSLRLSCKASGYTFTRYTMHWVRQAPGKGLEWIGYINPSRGYTNYNQKVKDRFTISRDNSKNTAFLQMDSLRPEDTGVYFCARYYDDHYSLDYWGQGTPVTVSSGGGGSGGGGSGGGGSDIQMTQSPSSLSASVGDRVTITCSASSSVSYMNWYQQTPGKAPKRWIYDTSKLASGVPSRFSGSGSGTDYTFTISSLQPEDIATYYCQQWSSNPFTFGQGTKLQITREPKSCDKTHTCPPCPAPEAAGGPSVFLFPPKPKDTLMISRTPEVTCVVVDVSHEDPEVKFNWYVDGVEVHNAKTKPREEQYNSTYRVVSVLTVLHQDWLNGKEYKCKVSNKALPAPIEKTISKAKGQPREPQVCTLPPSREEMTKNQVSLSCAVKGFYPSDIAVEWESNGQPENNYKTTPPVLDSDGSFFLVSKLTVDKSRWQQGNVFSCSVMHEALHNHYTQKSLSLSPGK

SEQ ID NO: 51 - protein, 474 aa, Artificial Sequence
QVQLQQSGAELVKPGSSVKISCKASGYTFTRNFIHWIKQQPGNGLEWIGWIFPGDGDTEYNQKFNGKATLTADKSSSTAYMQLSSLTSEDSAVYFCARGNYNYEYFDYWGQGVMVTVSSASTKGPSVFPLAPSSKSTSGGTAALGCLVKDYFPEPVTVSWNSGALTSGVHTFPAVLQSSGLYSLSSVVTVPSSSLGTQTYICNVNHKPSNTKVDKRVEPKSCGGGGSQVQLVQSGGGVVQPGRSLRLSCKASGYTFTRYTMHWVRQAPGKGLEWIGYINPSRGYTNYNQKVKDRFTISRDNSKNTAFLQMDSLRPEDTGVYFCARYYDDHYSLDYWGQGTPVTVSSGGGGSGGGGSGGGGSDIQMTQSPSSLSASVGDRVTITCSASSSVSYMNWYQQTPGKAPKRWIYDTSKLASGVPSRFSGSGSGTDYTFTISSLQPEDIATYYCQQWSSNPFTFGQGTKLQITRHHHHHH

SEQ ID NO: 52 - protein, 695 aa, Artificial Sequence
QVQLQQSGAELVKPGSSVKISCKASGYTFTRNFIHWIKQQPGNGLEWIGWIFPGDGDTEYNQKFNGKATLTADKSSSTAYMQLSSLTSEDSAVYFCARGNYNYEYFDYWGQGVMVTVSSASTKGPSVFPLAPSSKSTSGGTAALGCLVKDYFPEPVTVSWNSGALTSGVHTFPAVLQSSGLYSLSSVVTVPSSSLGTQTYICNVNHKPSNTKVDKRVEPKSCGGGGSQVQLVQSGGGVVQPGRSLRLSCKASGYTFTRYTMHWVRQAPGKGLEWIGYINPSRGYTNYNQKVKDRFTISRDNSKNTAFLQMDSLRPEDTGVYFCARYYDDHYSLDYWGQGTPVTVSSGGGGSGGGGSGGGGSDIQMTQSPSSLSASVGDRVTITCSASSSVSYMNWYQQTPGKAPKRWIYDTSKLASGVPSRFSGSGSGTDYTFTISSLQPEDIATYYCQQWSSNPFTFGQGTKLQITRDKTHTCPPCPAPEAAGGPSVFLFPPKPKDTLMISRTPEVTCVVVDVSHEDPEVKFNWYVDGVEVHNAKTKPREEQYNSTYRVVSVLTVLHQDWLNGKEYKCKVSNKALPAPIEKTISKAKGQPREPQVYTLPPSREEMTKNQVSLTCLVKGFYPSDIAVEWESNGQPENNYKTTPPVLDSDGSFFLYSKLTVDKSRWQQGNVFSCSVMHEALHNHYTQKSLSLSPGK

SEQ ID NO: 53 - protein, 580 aa, Artificial Sequence
QVQLQQSGAELVKPGSSVKISCKASGYTFTRNFIHWIKQQPGNGLEWIGWIFPGDGDTEYNQKFNGKATLTADKSSSTAYMQLSSLTSEDSAVYFCARGNYNYEYFDYWGQGVMVTVSSASTKGPSVFPLAPSSKSTSGGTAALGCLVKDYFPEPVTVSWNSGALTSGVHTFPAVLQSSGLYSLSSVVTVPSSSLGTQTYICNVNHKPSNTKVDKRVEPKSCGGGGSQVQLVQSGGGVVQPGRSLRLSCKASGYTFTRYTMHWVRQAPGKGLEWIGYINPSRGYTNYNQKVKDRFTISRDNSKNTAFLQMDSLRPEDTGVYFCARYYDDHYSLDYWGQGTPVTVSSGGGGSGGGGSGGGGSDIQMTQSPSSLSASVGDRVTITCSASSSVSYMNWYQQTPGKAPKRWIYDTSKLASGVPSRFSGSGSGTDYTFTISSLQPEDIATYYCQQWSSNPFTFGQGTKLQITRAAAGGGQPREPQVYTLPPSREEMTKNQVSLTCLVKGFYPSDIAVEWESNGQPENNYKTTPPVLDSDGSFFLYSKLTVDKSRWQQGNVFSCSVMHEALHNHYTQKSLSLSPGK

SEQ ID NO: 54 - protein, 701 aa, Artificial Sequence
QVQLQQSGAELVKPGSSVKISCKASGYTFTRNFIHWIKQQPGNGLEWIGWIFPGDGDTEYNQKFNGKATLTADKSSSTAYMQLSSLTSEDSAVYFCARGNYNYEYFDYWGQGVMVTVSSASTKGPSVFPLAPSSKSTSGGTAALGCLVKDYFPEPVTVSWNSGALTSGVHTFPAVLQSSGLYSLSSVVTVPSSSLGTQTYICNVNHKPSNTKVDKRVEPKSCGGGGSQVQLVQSGGGVVQPGRSLRLSCKASGYTFTRYTMHWVRQAPGKGLEWIGYINPSRGYTNYNQKVKDRFTISRDNSKNTAFLQMDSLRPEDTGVYFCARYYDDHYSLDYWGQGTPVTVSSGGGGSGGGGSGGGGSDIQMTQSPSSLSASVGDRVTITCSASSSVSYMNWYQQTPGKAPKRWIYDTSKLASGVPSRFSGSGSGTDYTFTISSLQPEDIATYYCQQWSSNPFTFGQGTKLQITRGGGGSQVQLQQSGAELVKPGSSVKISCKASGYTFTRNFIHWIKQQPGNGLEWIGWIFPGDGDTEYNQKFNGKATLTADKSSSTAYMQLSSLTSEDSAVYFCARGNYNYEYFDYWGQGVMVTVSSASTKGPSVFPLAPSSKSTSGGTAALGCLVKDYFPEPVTVSWNSGALTSGVHTFPAVLQSSGLYSLSSVVTVPSSSLGTQTYICNVNHKPSNTKVDKRVEPKSCHHHHHH

SEQ ID NO: 55 - protein, 474 aa, Artificial Sequence
QVQLVQSGGGVVQPGRSLRLSCKASGYTFTRYTMHWVRQAPGKGLEWIGYINPSRGYTNYNQKVKDRFTISRDNSKNTAFLQMDSLRPEDTGVYFCARYYDDHYSLDYWGQGTPVTVSSGGGGSGGGGSGGGGSDIQMTQSPSSLSASVGDRVTITCSASSSVSYMNWYQQTPGKAPKRWIYDTSKLASGVPSRFSGSGSGTDYTFTISSLQPEDIATYYCQQWSSNPFTFGQGTKLQITRGGGGSQVQLQQSGAELVKPGSSVKISCKASGYTFTRNFIHWIKQQPGNGLEWIGWIFPGDGDTEYNQKFNGKATLTADKSSSTAYMQLSSLTSEDSAVYFCARGNYNYEYFDYWGQGVMVTVSSASTKGPSVFPLAPSSKSTSGGTAALGCLVKDYFPEPVTVSWNSGALTSGVHTFPAVLQSSGLYSLSSVVTVPSSSLGTQTYICNVNHKPSNTKVDKRVEPKSCHHHHHH

SEQ ID NO: 56 - protein, 695 aa, Artificial Sequence
QVQLVQSGGGVVQPGRSLRLSCKASGYTFTRYTMHWVRQAPGKGLEWIGYINPSRGYTNYNQKVKDRFTISRDNSKNTAFLQMDSLRPEDTGVYFCARYYDDHYSLDYWGQGTPVTVSSGGGGSGGGGSGGGGSDIQMTQSPSSLSASVGDRVTITCSASSSVSYMNWYQQTPGKAPKRWIYDTSKLASGVPSRFSGSGSGTDYTFTISSLQPEDIATYYCQQWSSNPFTFGQGTKLQITRGGGGSQVQLQQSGAELVKPGSSVKISCKASGYTFTRNFIHWIKQQPGNGLEWIGWIFPGDGDTEYNQKFNGKATLTADKSSSTAYMQLSSLTSEDSAVYFCARGNYNYEYFDYWGQGVMVTVSSASTKGPSVFPLAPSSKSTSGGTAALGCLVKDYFPEPVTVSWNSGALTSGVHTFPAVLQSSGLYSLSSVVTVPSSSLGTQTYICNVNHKPSNTKVDKRVEPKSCDKTHTCPPCPAPEAAGGPSVFLFPPKPKDTLMISRTPEVTCVVVDVSHEDPEVKFNWYVDGVEVHNAKTKPREEQYNSTYRVVSVLTVLHQDWLNGKEYKCKVSNKALPAPIEKTISKAKGQPREPQVYTLPPSREEMTKNQVSLTCLVKGFYPSDIAVEWESNGQPENNYKTTPPVLDSDGSFFLYSKLTVDKSRWQQGNVFSCSVMHEALHNHYTQKSLSLSPGK

SEQ ID NO: 57 - protein, 580 aa, Artificial Sequence
QVQLVQSGGGVVQPGRSLRLSCKASGYTFTRYTMHWVRQAPGKGLEWIGYINPSRGYTNYNQKVKDRFTISRDNSKNTAFLQMDSLRPEDTGVYFCARYYDDHYSLDYWGQGTPVTVSSGGGGSGGGGSGGGGSDIQMTQSPSSLSASVGDRVTITCSASSSVSYMNWYQQTPGKAPKRWIYDTSKLASGVPSRFSGSGSGTDYTFTISSLQPEDIATYYCQQWSSNPFTFGQGTKLQITRGGGGSQVQLQQSGAELVKPGSSVKISCKASGYTFTRNFIHWIKQQPGNGLEWIGWIFPGDGDTEYNQKFNGKATLTADKSSSTAYMQLSSLTSEDSAVYFCARGNYNYEYFDYWGQGVMVTVSSASTKGPSVFPLAPSSKSTSGGTAALGCLVKDYFPEPVTVSWNSGALTSGVHTFPAVLQSSGLYSLSSVVTVPSSSLGTQTYICNVNHKPSNTKVDKRVEPKSCAAAGGGQPREPQVYTLPPSREEMTKNQVSLTCLVKGFYPSDIAVEWESNGQPENNYKTTPPVLDSDGSFFLYSKLTVDKSRWQQGNVFSCSVMHEALHNHYTQKSLSLSPGK

SEQ ID NO: 58 - protein, 228 aa, Artificial Sequence
QVQLQQSGAELVKPGSSVKISCKASGYTFTRNFIHWIKQQPGNGLEWIGWIFPGDGDTEYNQKFNGKATLTADKSSSTAYMQLSSLTSEDSAVYFCARGNYNYEYFDYWGQGVMVTVSSASTKGPSVFPLAPSSKSTSGGTAALGCLVKDYFPEPVTVSWNSGALTSGVHTFPAVLQSSGLYSLSSVVTVPSSSLGTQTYICNVNHKPSNTKVDKRVEPKSCHHHHHH

SEQ ID NO: 59 - protein, 460 aa, Artificial Sequence
QVQLVQSGGGVVQPGRSLRLSCKASGYTFTRYTMHWVRQAPGKGLEWIGYINPSRGYTNYNQKVKDRFTISRDNSKNTAFLQMDSLRPEDTGVYFCARYYDDHYSLDYWGQGTPVTVSSGGGGSGGGGSGGGGSDIQMTQSPSSLSASVGDRVTITCSASSSVSYMNWYQQTPGKAPKRWIYDTSKLASGVPSRFSGSGSGTDYTFTISSLQPEDIATYYCQQWSSNPFTFGQGTKLQITRGGGGSDIQMTQSPASLSASLGETVSIECLASEDIYSYLAWYQQKPGKSPQLLIFAANRLQDGVPSRFSGSGSGTQFSLKISGMQPEDEGDYFCLQGSKFPYTFGPGTKLELNRTVAAPSVFIFPPSDEQLKSGTASVVCLLNNFYPREAKVQWKVDNALQSGNSQESVTEQDSKDSTYSLSSTLTLSKADYEKHKVYACEVTHQGLSSPVTKSFNRGEC

SEQ ID NO: 60 - protein, 449 aa, Artificial Sequence
QVQLQQSGAELVKPGSSVKISCKASGYTFTRNFIHWIKQQPGNGLEWIGWIFPGDGDTEYNQKFNGKATLTADKSSSTAYMQLSSLTSEDSAVYFCARGNYNYEYFDYWGQGVMVTVSSASTKGPSVFPLAPSSKSTSGGTAALGCLVKDYFPEPVTVSWNSGALTSGVHTFPAVLQSSGLYSLSSVVTVPSSSLGTQTYICNVNHKPSNTKVDKRVEPKSCDKTHTCPPCPAPEAAGGPSVFLFPPKPKDTLMISRTPEVTCVVVDVSHEDPEVKFNWYVDGVEVHNAKTKPREEQYNSTYRVVSVLTVLHQDWLNGKEYKCKVSNKALPAPIEKTISKAKGQPREPQVYTLPPSREEMTKNQVSLTCLVKGFYPSDIAVEWESNGQPENNYKTTPPVLDSDGSFFLYSKLTVDKSRWQQGNVFSCSVMHEALHNHYTQKSLSLSPGK

SEQ ID NO: 61 - protein, 334 aa, Artificial Sequence
QVQLQQSGAELVKPGSSVKISCKASGYTFTRNFIHWIKQQPGNGLEWIGWIFPGDGDTEYNQKFNGKATLTADKSSSTAYMQLSSLTSEDSAVYFCARGNYNYEYFDYWGQGVMVTVSSASTKGPSVFPLAPSSKSTSGGTAALGCLVKDYFPEPVTVSWNSGALTSGVHTFPAVLQSSGLYSLSSVVTVPSSSLGTQTYICNVNHKPSNTKVDKRVEPKSCAAAGGGQPREPQVYTLPPSREEMTKNQVSLTCLVKGFYPSDIAVEWESNGQPENNYKTTPPVLDSDGSFFLYSKLTVDKSRWQQGNVFSCSVMHEALHNHYTQKSLSLSPGK

SEQ ID NO: 62 - DNA, 2142 bp, Artificial Sequence
caggtgcaactgcagcagtccggggctgagctggtgaagcctggtagctctgtaaagatctcttgcaaggcaagcggctacacttttacccgaaacttcatccattggatcaaacagcaaccaggcaatggactagagtggattggatggatctttcctggcgatggggacaccgaatacaatcagaaattcaacgggaaagccaccttaactgctgataagtcttcctcaaccgcatacatgcagttaagcagcctgacatccgaggattcagccgtgtacttttgtgctagaggcaactacaattacgagtatttcgattattggggccagggcgttatggtcaccgtgtcatccggtggtggcgggagtggcggaggtggctctggtggtggaggatctgatatacagatgacgcagagtcccgccagcttatctgcgtccctgggggaaaccgtgtcgattgaatgcctagcaagtgaggacatctatagctaccttgcatggtaccaacagaaacccggtaaaagtcctcagttgttgatatttgccgccaaccggttacaggacggagtccccagcaggttttctgggtcagggagcggtacacagttttccctgaagatctcagggatgcagccagaagacgagggcgattacttctgtctgcagggttctaagttcccgtacaccttcggacctggcactaagctggaactcaatggcggcggcggtagccaggtccagcttgttcagtctgggggaggggtagtgcaaccaggaagatccctgaggctgtcatgcaaagcctccgggtatacattcacccgctatacgatgcattgggtgagacaggcaccgggaaaggggcttgaatggatcggctatattaacccatcaagaggctacactaactataaccagaaagtgaaagaccggtttactatctcgcgtgataacagcaaaaacactgccttcttgcagatggatagcctgaggccagaggacacaggcgtgtatttttgtgcgcggtattatgacgaccattactcgctcgactattgggggcaaggcactcctgtcaccgtcagctctggaggcgggggaagtggaggaggagggtccggtggcgggggatcagacatccaaatgactcagagcccctcaagtctgtcagcttcggtgggcgatcgcgtcacgattacttgtagcgccagtagtagcgttagctacatgaactggtatcagcaaacaccaggtaaagcccccaaacgctggatttatgacaccagcaaattggcttctggagtgcctagtcgttttagcggatctggatcaggcacagactacaccttcaccatttcctcccttcaacccgaggacatagcgacatactactgtcagcagtggagttccaatccattcacgtttggtcaaggaacgaagctgcagataaccagagacaagactcacacttgccctccttgtcctgcccccgaagccgccggcggcccttcagtatttctctttccaccgaaacctaaggacacattgatgatctcacgcactccagaagtgacctgcgtggtggttgatgtctcacacgaagatcctgaggtgaaattcaactggtacgtagatggcgtggaagtccataacgcgaagacaaagcccagagaggagcagtataattcgacctatcgggtggtttcggtactgaccgtcctgcatcaggactggcttaacggcaaggagtacaagtgcaaggtttctaataaagccctcccagctcccatcgagaaaacaatcagcaaggctaagggccaacccagggaaccccaagtctacactttgccaccgagtcgtgacgagctcacaaaaaatcaggtgtctttaacttgcctcgtaaagggcttttatcccagcgacattgccgtcgagtgggaatcgaatggccagccagaaaacaactacaagactactccacccgtgctcgactcagacggctcctttttcctgtactccaaacttactgtggataagagtagatggcagcagggcaatgtgttctcctgttcagtgatgcatgaagcccttcacaaccattacacacagaaatccttgtctctgtccccaggcaag

SEQ ID NO: 63 - DNA, 2166 bp, Artificial Sequence
gatatccagatgacgcagagccctgcttccctgtccgccagcttgggcgaaacagtgagcatcgaatgtctggcgtccgaggatatctacagctacctggcttggtaccagcagaaacccgggaagtcacctcagttgctgatatttgccgctaacaggctccaggatggggtgccaagcagattttcagggtccgggagtgggacgcagttcagcctcaaaatctccgggatgcagcccgaagacgaaggggactacttttgcctccaaggatctaagtttccgtacactttcggacctggaaccaaacttgagctgaatggcggcggcggctccggcggcggtggatccggggggggcgggagccaggtccaactgcagcagtctggcgccgaactcgtcaagccgggcagtagtgtgaagatctcttgtaaagcaagcggctatacctttacccggaattttattcactggattaagcagcaaccaggcaatggcctagagtggataggatggatctttccaggcgatggtgacacagaatacaatcagaagttcaatggcaaagcaacactgactgccgacaaaagcagtagcactgcctacatgcagctctcatccttaacctcagaggactcagccgtctacttctgcgctagaggaaactacaactacgagtacttcgactactggggccaaggcgtaatggtgactgtgtcttcgggagggggaggttcacaggttcagctggtgcagtctggaggcggagtggtccaaccaggtcgctccctgaggctgagttgcaaggcatccggttataccttcacccgctacactatgcactgggttcgacaagctccaggtaaagggctcgaatggattgggtatatcaacccttctcgggggtataccaactataaccagaaggttaaagaccggttcaccattagccgggataactctaagaacactgcatttctgcagatggattccctcagacccgaagatacgggtgtgtacttctgtgccagatactacgatgaccactacagcttggactattgggggcaaggaactcctgtaaccgtgagcagtggaggagggggctctggtggaggtggatctggcggaggaggctccgacatacagatgacccagtctccctcgtccttgtccgcctccgtaggagatcgggtgactatcacctgttcagcatcctcgtcagtgagctatatgaactggtatcaacaaacaccagggaaagctccgaagcgctggatctacgataccagcaagttagcgtcaggcgtcccctctcgatttagtggctctgggtcagggacagactatacatttacgatctcaagccttcaacctgaggacattgccacgtattattgccagcagtggtcttctaatccattcacctttggtcaggggactaaactgcagattactaggttggaggtactcttccaaggtcctgacaagacacatacttgtcccccatgtcccgctccagaattgcttggtggtccaagcgtattcctatttcccccgaaacccaaggatactctcatgatatcacgtacacccgaagtgacatgcgttgtcgtagacgttagtcatgaggatcctgaggtgaaattcaactggtatgtggacggcgttgaagtgcacaatgccaagacaaagccacgtgaggaacagtacaatagcacctatagggtggtttcagtgttaacagtcctgcatcaggattggcttaatggcaaggagtacaagtgcaaagtctcgaacaaggcactgcctgctccgattgagaagacaatctcgaaagcgaagggacagcctagagaaccacaggtgtacacactccctcccagtagggacgagctaacaaagaatcaggtgagcttaacctgcctcgtgaaaggcttttatccctccgatattgcagtcgagtgggagtccaacggtcaacccgagaacaactataagacaactccccctgtgttggacagtgacggatccttcttcctgtatagcaaacttaccgtcgataaaagtcgctggcagcagggaaatgttttcagttgcagcgtgatgcatgaggccctgcacaatcactatacccagaagagtctttctctatctcctggcaaa

SEQ ID NO: 64 - DNA, 2142 bp, Artificial Sequence
caggttcaactggtgcagtccggcggtggcgtggtgcaacctggcagatccttacggctgtcttgtaaggcatctggctacactttcacccggtatacgatgcattgggtgaggcaggcaccaggaaaggggttggagtggatcggttacattaatcccagccgaggctataccaactataaccagaaggtcaaagacaggtttacaatcagccgagacaatagcaagaataccgcctttcttcagatggactccctaagacctgaggacactggcgtgtatttctgcgcccgttattacgatgaccactactccctggactattggggccaggggaccccggtaacagtgtcttccggaggcggcggatctggcggaggtggatccggcggcggtgggtccgatatccaaatgactcagtcaccgagcagtctgtccgccagcgttggggacagagtgaccatcacatgcagtgctagttcctccgtctcttacatgaattggtatcagcagactccgggtaaggcgcctaaaaggtggatttacgatacctccaagctcgcatccggtgttccttccagatttagcgggtccggctctgggactgactacacattcaccataagtagcctacaacccgaagatatcgcaacctattactgtcagcagtggtcttcgaatccttttacgtttggacagggaaccaaactgcagattacacggggagggggcggctctcaagtgcagttacaacagtcgggcgctgaacttgtgaaaccaggctcttcagtcaagatcagttgcaaagcctctggctatacattcactcgcaatttcatccactggataaagcagcaacctggaaatggcctggaatggataggatggattttccccggtgatggcgatacagagtacaaccagaagttcaacgggaaagctaccctcactgccgataagtccagttctaccgcatacatgcagcttagtagcttgacaagtgaagatagcgctgtctacttttgcgccagaggaaactacaattacgagtattttgactactggggccaaggggtcatggtcacagttagctcagggggaggcgggtcaggagggggagggagcggaggcggtggcagcgacattcagatgactcagagccccgcttctctttccgcctcactcggggagactgtgagcatcgagtgtctcgcaagcgaggatatctattcctatctggcttggtaccagcagaaacccggcaaatcgccacagctcttgattttcgccgcgaaccggctgcaggatggggttcctagccgcttcagcggttccgggagcggaacacagttctcactgaaaatttcagggatgcagcccgaggacgaaggtgactacttttgtctgcaagggtcgaagttcccctatacgttcggtccaggaaccaagctggagctcaacgacaagactcacacttgccctccttgtcctgcccccgaagccgccggcggcccttcagtatttctctttccaccgaaacctaaggacacattgatgatctcacgcactccagaagtgacctgcgtggtggttgatgtctcacacgaagatcctgaggtgaaattcaactggtacgtagatggcgtggaagtccataacgcgaagacaaagcccagagaggagcagtataattcgacctatcgggtggtttcggtactgaccgtcctgcatcaggactggcttaacggcaaggagtacaagtgcaaggtttctaataaagccctcccagctcccatcgagaaaacaatcagcaaggctaagggccaacccagggaaccccaagtctacactttgccaccgagtcgtgacgagctcacaaaaaatcaggtgtctttaacttgcctcgtaaagggcttttatcccagcgacattgccgtcgagtgggaatcgaatggccagccagaaaacaactacaagactactccacccgtgctcgactcagacggctcctttttcctgtactccaaacttactgtggataagagtagatggcagcagggcaatgtgttctcctgttcagtgatgcatgaagcccttcacaaccattacacacagaaatccttgtctctgtccccaggcaag

SEQ ID NO: 65 - DNA, 2142 bp, Artificial Sequence
caagtgcaactcgtccagtccggtggaggcgtagtacagccaggcagatcattgagactgagctgcaaggccagcgggtacacttttacgcgctacactatgcattgggtgagacaggcaccaggcaaggggttggaatggatagggtacatcaatcccagccgcggatataccaattacaatcagaaggtcaaagatcggttcaccatttctagggataacagcaagaacactgccttcctgcagatggactctctgcggcctgaggatactggggtgtacttctgtgctcgctactacgacgaccactattccctagattactggggacagggcaccccagtcacagtttcgtcaggaggaggtgggtccggcggagggggtagcgggggcggaggctcagatatccagatgactcagagtccctcgagcctttctgcttccgtaggcgatcgggtgaccatcacttgttctgcgtccagcagtgtcagttacatgaactggtatcaacagactccagggaaagctcccaaaaggtggatctatgacacaagtaagttggccagcggcgtcccctcgcgcttcagtgggtctggctccggcaccgactatacctttacaatctcaagccttcagcccgaagacattgctacatactactgtcagcagtggtcaagtaacccattcaccttcgggcagggcacaaagctccagattacacgagggggaggaggcagcgacatccaaatgacccagagccccgctagcttgagcgccagtcttggcgagactgtgtctatagagtgcttagcctctgaggatatctactcttatctggcatggtatcagcagaagcctgggaaatcccctcagctgctgatctttgccgcgaatcggctacaggatggagtcccttctcgttttagtggctctggcagtggtacgcaattttccctgaagatctcaggcatgcagccggaagacgagggcgactatttctgcttacagggcagcaaatttccctataccttcggtccgggtacaaaacttgagctgaatggtggggggggctccgggggtggcgggtcaggcggcggcggatcccaggttcagctgcagcagtcaggagctgaactggtgaaacccggatcgagcgttaagatttcttgcaaagcatcagggtatacgtttacgcgaaacttcatccactggattaagcagcagccaggtaacggcttggagtggataggctggatttttcccggagacggagacaccgagtataaccagaagttcaatggcaaggcaacactgacagctgacaagtccagtagcacagcctacatgcaactgtcttcactgactagcgaagattcagccgtctacttttgcgcacgggggaattacaactacgagtacttcgactattggggtcaaggcgttatggtgactgtgagttccgataagacacatacctgtcctccatgccctgctcctgaagctgctggaggtcccagcgtctttttgtttcctccaaaaccgaaagacacactgatgatttcccgtaccccggaagttacctgtgtggtggtggatgtttctcacgaggatccggaagtgaagttcaactggtatgttgatggtgtagaggtccacaatgcgaagaccaaacctagggaggagcaatacaactccacctatagggtggtcagcgtgctaactgtgctccatcaggactggctgaatgggaaggagtacaagtgcaaagtctccaataaagcattacctgcaccaatcgagaaaaccatctccaaggccaaaggacaaccaagagaacctcaggtgtacacactgcccccatccagagatgagctcaccaaaaaccaggtgtctctgacttgcctcgtaaagggattctatcccagtgacattgccgtggaatgggagtccaatggacaacccgaaaacaactacaagacaaccccacctgtgctggactcggatggtagcttcttcctgtattctaagctcacggtggataaatctaggtggcagcaggggaatgtgtttagttgtagcgtaatgcatgaagccttacacaaccactatacgcagaaatccctttcactgtcacctggtaag

SEQ ID NO: 66 - DNA, 2151 bp, Artificial Sequence
caggtccagttggtccaatctggaggcggtgtagttcagcctgggaggtctttacgcctgagctgtaaagcaagcggatatacattcacccggtacaccatgcactgggtgagacaggctcccggaaagggacttgagtggatagggtatatcaacccgtctcgtggttataccaactacaaccagaaggtgaaagacagattcaccatctctagggacaactccaagaacacagcgtttctgcagatggatagcttacggccagaggatactggcgtgtatttctgcgccagatactacgatgaccactacagcctggattattggggccagggtacccctgtgactgtctcgtcaggcgggggaggtagtgatatccagatgacccagtccccagcttctctatccgcttcattgggagaaaccgtttccattgaatgtctggcttctgaggacatttacagctacctggcgtggtatcagcagaaacccgggaaatcccctcagctcctcattttcgctgccaatcgcctgcaagatggggttccatcccggtttagcgggagcgggtctggaacccagttctccctgaagatctccggcatgcaacctgaggatgagggggactacttttgcctgcaggggagcaaattcccctatacatttggtccgggtacgaaactggagctcaatggaggtgggggatccggaggcggaggaagcggcggagggggcagcggggggggtggtagtcaggtgcagctacaacagagtggagctgagctggtcaagcccgggagtagtgtcaagatttcctgcaaagccagtggatatacgttcacgcgaaatttcattcactggattaagcagcagccaggcaacggcttagagtggatcggatggatctttcctggggatggtgataccgagtataaccagaaattcaatggtaaagccactctaacagccgataagagcagtagcactgcctatatgcaattgtcatccctaacctctgaagacagtgcagtgtacttctgtgcacgagggaattacaattatgagtacttcgactattgggggcagggagttatggtaaccgtgagcagtggaggtggtgggagcgacatacagatgactcaatctcctagctctctgtcagcaagtgtgggagatcgagtgaccataacgtgcagcgcctccagctcagtctcatacatgaactggtaccaacagacgccaggaaaagcacccaaacggtggatttacgacacatcgaagctggccagtggggtgccgtctcgcttctccgggtctggctcaggcaccgactacacctttacaatctcatctctgcagcccgaagatatagccacatattattgtcaacagtggagcagcaatccctttacatttggccaaggcaccaagctccagattacgaggctggaagtgctgtttcaaggccctgacaagactcacacttgccctccttgtcctgcccccgaagccgccggcggcccttcagtatttctctttccaccgaaacctaaggacacattgatgatctcacgcactccagaagtgacctgcgtggtggttgatgtctcacacgaagatcctgaggtgaaattcaactggtacgtagatggcgtggaagtccataacgcgaagacaaagcccagagaggagcagtataattcgacctatcgggtggtttcggtactgaccgtcctgcatcaggactggcttaacggcaaggagtacaagtgcaaggtttctaataaagccctcccagctcccatcgagaaaacaatcagcaaggctaagggccaacccagggaaccccaagtctacactttgccaccgagtcgtgacgagctcacaaaaaatcaggtgtctttaacttgcctcgtaaagggcttttatcccagcgacattgccgtcgagtgggaatcgaatggccagccagaaaacaactacaagactactccacccgtgctcgactcagacggctcctttttcctgtactccaaacttactgtggataagagtagatggcagcagggcaatgtgttctcctgttcagtgatgcatgaagcccttcacaaccattacacacagaaatccttgtctctgtccccaggcaag

SEQ ID NO: 67 - DNA, 2127 bp, Artificial Sequence
gatatccagatgactcaaagtccctcctctcttagcgcaagcgtaggagatcgggtgaccattacatgctctgcatcgagctcagtatcatacatgaattggtaccagcagacaccaggaaaagccccgaagcggtggatttatgacactagtaaactcgcttctggagtcccaagccgcttcagtgggtctggaagtgggacagactatactttcacaatcagcagtctacagccagaggacattgctacttactactgccaacagtggtcttccaaccctttcacctttggccagggcactaaattgcagattaccagaggtggaggtggatcccaggtgcagttacagcagtctggcgctgaactggtgaaacccgggtcatctgtgaagatatcctgcaaggctagcggatatacattcacccgaaacttcatccactggataaagcagcagcctgggaatggcttggagtggattggttggatttttcccggcgacggggatactgagtacaatcagaagttcaacggcaaagccaccttaaccgcggataagtcgagtagcacagcttacatgcagttgtcatccctaacatctgaggatagcgccgtgtatttctgcgcaagagggaattataactacgaatacttcgattattgggggcaaggagttatggtgacagtgagctctggcggcgggggatccggtgggggaggctcaggaggaggaggcagcggaggagggggaagcgacatccaaatgactcagtcccctgcctcactcagtgccagtttgggagaaacggtgtccatcgaatgtttggcctctgaggacatatacagctacctcgcctggtatcagcagaagcctggcaagtcccctcaactgctcatttttgctgccaatcgcttacaggacggcgtacctagccggttttcaggttctggctcaggtactcaattcagtttaaagatatccggcatgcagccagaagatgagggcgattatttctgcttgcagggtagcaagtttccctacaccttcggtcccggcactaagctcgaactcaatggaggcggcgggtcacaggtccaactagtccagtccggtggcggcgtggttcagcctgggcgttcccttagactgagctgtaaggccagcgggtacaccttcaccagatacaccatgcactgggtgcgccaagcaccagggaaaggccttgagtggatcggttacatcaatccatcgaggggatacacgaactataaccagaaagtcaaagatcggtttacaatcagtcgggacaactctaagaacacggcctttctacaaatggactcacttagacccgaggatacaggggtctacttttgtgcacgctactatgacgaccactattccctggattactgggggcagggcacacccgtcaccgtgtcctcggacaaaacacacacgtgtccaccatgtccagcccctgaagccgccggtgggccgagcgtgtttctgtttccccccaaaccgaaagacaccctcatgatcagtcgaacacctgaagtaacctgtgtggttgtggacgtgtcccatgaggacccggaagtcaagtttaactggtatgtagacggtgttgaggttcacaacgccaagaccaaacccagggaagagcagtataacagcacgtatcgtgtcgtgagcgtcctgacagtcctgcatcaggattggctgaatggtaaggagtataagtgcaaagtgagcaacaaggctctgccagcgcccatcgaaaaaaccatttccaaggcaaaagggcagccaagggaaccccaagtgtacacgctgccaccttctagggacgagctgactaaaaatcaggtgtcactgacctgcctggttaagggcttctatcccagtgatattgcggttgagtgggagtctaatggccagccggaaaataactacaagacaactcctcctgttctggactccgatgggtcattcttcctgtattccaaactgactgtggataagagcaggtggcaacagggcaatgtcttctcatgctcggtgatgcatgaggcactgcataaccactacactcagaagtctctgagtctgtctcctgggaaa

SEQ ID NO: 68 - DNA, 2127 bp, Artificial Sequence
caagtacagctccagcagtcaggagctgagctggtaaaacctgggagtagcgtgaagattagctgcaaagctagtggatacacctttacccgtaacttcatccattggatcaagcaacagcctgggaatgggctcgaatggataggctggatctttccgggggatggggataccgagtacaatcagaagttcaatggcaaggccacactgaccgcagataagtcttcttccaccgcatacatgcagctgtccagccttacaagcgaggattctgccgtttatttttgcgccagaggaaactacaactatgagtactttgactattggggtcaaggtgtgatggtgaccgtctcctccgggggtgggggttcggacattcagatgactcagtcgccttcctcattaagtgcctcagttggggaccgggtaaccattacctgcagcgcatcttcaagcgtctcatacatgaactggtaccaacaaacgccaggcaaagcacccaaacgctggatctatgacacttcaaagctggcttccggggttccttcgcgattttctgggagtggctctggcactgattacaccttcacaatatcctcactgcaacccgaggatatcgccacttattactgccagcagtggtctagcaatcctttcacttttgggcaggggacaaaactccagattacccgaggtggcggcggatcaggtggcggtggcagcggaggcggagggtctgggggaggcgggagccaggtacagcttgtccagtctggcggaggcgttgtccagccaggcaggagtcttcgcttgagctgtaaggcttcaggctacactttcacccggtatactatgcactgggttagacaagccccagggaagggtctggagtggatcggctatatcaatcctagtagggggtacacgaattacaaccagaaagtgaaggaccggtttacaataagcagggacaattcgaaaaacaccgcttttctgcaaatggacagtctgcgacccgaagacacaggcgtgtatttctgtgccagatactatgatgaccactactcgctggattactgggggcagggaacacccgtgaccgtgagtagcggaggagggggctctgacatacaaatgactcagagtcctgcctccttgagcgcatctctgggagaaactgtgtccattgaatgccttgcgagtgaggacatctacagctatctagcctggtatcagcagaagcccggtaaatcacctcaattgctcatttttgccgcgaatcgcctacaggatggagtcccttccaggttcagcggctccggatctggaacacaattcagcctcaagatttcaggcatgcagccggaagatgaaggagattacttctgcctacagggaagcaaattcccctacacattcggacccggtacaaaacttgaactgaacgataagacacacacctgtccaccatgtcctgcaccagaagccgccggcggccctagtgtcttcctgtttcccccgaaaccgaaggacacactcatgatcagcaggactcccgaggtgacatgcgtggtggtcgacgtttcccatgaggacccagaagtcaaattcaattggtatgtggacggggtggaggtgcacaatgcgaagacgaagccacgcgaagagcagtataatagcacctatcgggttgtgtccgtcctcacagtcctgcatcaggattggctgaacggtaaagagtacaagtgcaaggtgagtaacaaggcattgcccgctcccattgagaagacaatctctaaggccaaaggtcagccacgggaaccgcaggtatatacgctcccacccagcagagatgagctgactaagaaccaggtatcactcacgtgtctggtgaaaggcttttatccatccgatattgctgttgaatgggagtcaaatggccagcctgaaaacaactacaagactacgcctccagtgttagactctgatggatccttctttctatattctaaactgaccgtggacaaatcccgttggcagcagggcaacgtgttttcctgttccgtgatgcatgaggctctgcacaaccactacacccagaagagtctgtctctgtcccccggtaaa

SEQ ID NO: 69 - DNA, 2151 bp, Artificial Sequence
gacattcagatgacacagagtccagcaagtctgtccgcaagccttggtgagactgtaagcatcgagtgcctggccagcgaagacatttattcctatctggcgtggtaccagcagaagccagggaagtcaccccagctcctcatttttgccgctaatcgcttacaggacggcgtgccctcacgattcagcgggagcggaagtggcactcagttttccctgaagatttccggaatgcagccagaagacgaaggggattatttctgcctacaaggatcaaagttcccgtatacgtttggccctggtactaaactggaactgaatggggggggagggtcccaggttcagctggtgcagtcaggagggggagtggttcaaccgggcagatctctgaggttatcctgcaaagctagtggctatacctttacacggtacacaatgcactgggtgaggcaggcacctggtaaggggctggagtggatagggtatatcaatcccagcagaggctatacgaattacaatcagaaggtgaaagaccgctttactataagccgtgacaacagtaagaacaccgcctttctccagatggactcgttgcgaccagaagatacaggggtctatttctgcgccagatactatgacgaccattactccctagactactggggtcaaggaacaccagtcaccgtcagtagcggcggaggaggctctggcggtggcgggtccggtggcggtggttccgggggaggaggatccgatatccagatgacccaaagcccttcttcactctcggcatccgtaggcgatagagtcaccataacatgcagtgcttcaagctccgtgtcctacatgaactggtatcagcaaactcctggtaaagcacccaagaggtggatttacgatacctcaaagctggcctctggcgtaccctccaggttttctggctcgggctccgggacagactatacgttcacgatcagttctctccagcctgaggatattgccacttactactgtcagcagtggagcagcaatccctttaccttcggccagggaacaaagttacagatcacgagaggtggcggcgggagtcaagtgcagctccaacagtctggcgccgaactcgtgaaacccggatctagcgtgaaaatctcatgcaaggccagcggctatacattcacccggaacttcatccactggattaagcaacagcctggaaatggtctagaatggatcggttggatttttccgggagatggagacaccgagtacaaccaaaaattcaacgggaaagcgactctgaccgccgataaatcgagctctacggcttacatgcagctgtcttctctcacttcagaggactcagccgtttacttttgtgctcgcggcaactacaactacgagtactttgattattggggtcagggcgtaatggtgaccgtctcctctctcgaagtgctgttccagggaccagacaaaactcacacatgtccaccttgtcccgctcctgaggccgccgggggcccatcggtctttctgttcccccctaaaccaaaagacaccctgatgatctctcgtacacccgaggtgacctgtgtcgttgtggacgttagccacgaggaccccgaagtgaagttcaactggtatgtggatggcgtggaggttcataatgccaaaacaaagcctcgggaagagcagtataattctacataccgcgttgtatcagtattgaccgtcctgcatcaggattggttgaatggaaaggagtacaagtgcaaggtgtctaacaaggcactgcctgcgcctatagagaagaccatctccaaggctaaagggcaaccacgggaaccacaagtctacacacttccccccagcagggatgaactcaccaaaaaccaggtgagtctgacttgcttggttaaaggcttctacccgtccgatattgccgtcgaatgggagagcaacggacagccggagaacaactataagaccacacctccagtgttggatagcgatgggagcttcttcctttacagtaagctgactgtcgacaagtctcgatggcaacaggggaatgtgtttagctgtagtgtgatgcatgaggcattacacaatcactatactcagaaatccttgagtctatcacccgggaaa

SEQ ID NO: 70 - DNA, 1479 bp, Artificial Sequence
caggtacagctgcaacagtctggggctgagttagtcaaaccagggtcctcggtgaagatctcttgcaaggcatcaggctacacattcacccgtaatttcattcactggattaagcagcagccaggaaatggcctcgagtggattgggtggatatttcccggggatggagataccgagtacaatcagaagtttaatggaaaggccacactgaccgctgacaagtcgagttcaactgcctatatgcagctgagttccctgaccagcgaggatagcgccgtttatttctgcgcaagagggaactacaactacgagtacttcgactattggggacagggtgtcatggtcacagtgagttctggggggggaggttcaggcggcggagggtctggcggaggcggctctgacattcagatgacacagagtcctgcaagtctgagtgcgtcccttggcgagactgtgtccatcgaatgtctcgcatctgaagacatctactcctatttggcgtggtaccagcaaaagccagggaaatcccctcagttactgatcttcgccgctaataggctgcaagatggagtgcctagccgattttctggtagcggatccggcacccagttctcgctcaagatctccggtatgcagcccgaagatgaaggagactacttctgcttgcagggcagcaagttcccctatacctttggaccggggaccaagttggagctcaatgggggcggaggtagccaggttcagctagttcagtcaggtgggggcgtagtgcaacccggaaggtcccttagactgagttgcaaagcttccggctatacatttacccggtatacgatgcattgggtgagacaagcgccaggcaaaggcttggaatggattggctacatcaacccttctcggggttatacaaactacaaccagaaggtgaaagatcggtttactatcagtcgcgacaacagcaaaaacaccgcatttctgcagatggacagccttagacccgaagacacaggcgtctatttctgtgccaggtattacgacgatcactacagcctagattactggggtcaaggcactcccgtcacagtgtctagcggaggtggaggctcagggggtggcgggtctggtggaggaggcagcgacatacagatgactcagtctcctagctccctttcagccagcgtaggcgatcgcgtgacaatcacttgtagcgccagcagctcagtgtcgtacatgaactggtatcagcagactcctgggaaagcccccaaacgatggatttatgacacatcaaagctggcatcaggggttccaagccgcttttccggcagtggtagtggaaccgactatacgttcacgatctcttccctccaaccagaggatattgccacttactactgtcaacagtggtcatctaatccgtttacctttggccaggggacgaaactccaaattaccaggcaccatcaccaccatcac

SEQ ID NO: 71 - DNA, 1479 bp, Artificial Sequence
gatatacagatgacccaatcaccagcatctctttccgctagccttggcgaaactgtgtccatcgaatgccttgcctccgaagacatctatagctatctggcctggtatcagcagaaacccggcaagtcacctcagctgctaatcttcgcggccaatagactccaggacggggtaccatctcgttttagcgggtccggctcgggaacacagtttagcctgaagatttcagggatgcagcctgaggacgaaggggactacttctgtctccagggatccaagttcccctacacatttggcccaggtaccaaactggagctgaatggtggggggggctctggaggcggtgggtctgggggcggtggcagtcaagtccagctacagcaaagtggggccgaattggtgaaaccaggcagcagcgtgaaaatctcctgcaaagccagtgggtatacgttcacaaggaacttcatccactggatcaaacagcagcctggcaatggcttagaatggattggctggatttttcccggggatggagacaccgagtataatcagaagttcaacgggaaggccactctcactgcggataagtcatcgagtactgcctatatgcagctgtcctcgctgacttctgaggatagcgctgtgtacttttgtgctcgcggcaactacaactacgagtactttgactactggggacagggtgtaatggtcacagtgtcgtccggcgggggaggatctcaggtacagctggttcaatccggaggaggagtggtgcaaccgggtagatctttgaggctgtcatgcaaggcctccgggtacacatttacccggtataccatgcattgggtgcgacaagcaccgggaaagggtttagagtggatcggatatatcaatcccagcagaggttacaccaattacaaccagaaagtcaaggacagattcaccatcagccgcgataactcaaagaacacggcttttctccagatggattccctgcgaccagaggatactggcgtgtatttctgtgctcggtattacgatgatcactatagtctcgactattggggccagggcacaccagtcaccgtgtctagtgggggagggggctcaggaggagggggatcaggcggcggtggttctgacattcagatgacgcaatctccttctagcttgagtgcttccgttggcgatcgcgtcactattacctgtagcgcaagcagcagtgtgtcctacatgaattggtaccagcaaacgcctggcaaagcaccgaaacggtggatttacgacactagcaagctcgcatcaggagttcccagcaggttttccggaagtggttctggcacagactacacattcaccataagctcccttcagcccgaggacattgccacctactattgccaacagtggtcaagtaaccctttcactttcgggcagggaaccaagctgcaaattaccaggcatcaccaccatcaccat

SEQ ID NO: 72 - DNA, 1479 bp, Artificial Sequence
caggtgcagctggttcagtctggtggcggagttgtgcagcctggcagatctctgagactgagctgtaaagccagcggctacaccttcaccagatacaccatgcactgggtccgacaggcccctggaaaaggactggaatggatcggctacatcaaccccagccggggctacaccaactacaaccagaaagtgaaggaccggttcaccatcagccgggacaacagcaagaataccgccttcctgcagatggacagcctgaggcctgaagataccggcgtgtacttctgcgcccggtactacgatgaccactacagcctggattactggggccagggcacacctgtgacagtttctagcggaggcggaggaagtggcggcggaggatctggcggtggtggttctgatatccagatgacacagagccctagcagcctgtctgcctctgtgggcgatagagtgaccatcacatgtagcgccagcagcagcgtgtcctacatgaactggtatcagcagacccctggcaaggcccctaagagatggatctacgataccagcaagctggcctccggcgtgccaagcagattttctggctctggcagcggaaccgattacacgttcaccattagctccctgcagccagaggatatcgccacctactactgccagcagtggtccagcaatcccttcacctttggacagggcaccaagctgcagatcacaagaggtggtggtggcagccaggttcagctgcaacaatctggcgccgagctggttaagcctggctctagcgtgaagatctcttgcaaggcctccggatacacattcacccggaacttcatccactggatcaagcagcagcccggcaatggactcgagtggatcggatggattttccccggcgacggcgacaccgagtacaatcagaagttcaacggcaaggccacactgaccgccgataagagcagcagcacagcctacatgcagctgagcagcctgacaagcgaggacagcgccgtgtatttctgtgccagaggcaactacaattacgagtacttcgactattggggacagggcgtgatggttaccgtttcatctggcggaggcggaagcggtggtggtggaagcggaggtggcggctcagatattcagatgacccagtctcctgccagcctgagcgcttctctgggagagacagtgtctatcgagtgcctggccagcgaggatatctacagctacctggcttggtatcaacagaagccaggcaagagccctcagctgctgatcttcgccgccaatagactgcaggatggcgtgccatctagattcagcggctctggctccggcacacagttcagcctgaaaatctctggcatgcagcccgaggacgagggcgattacttttgcctgcaaggcagcaagttcccctacacatttggccctggcacaaagctggaactgaaccaccatcatcaccaccac

SEQ ID NO: 73 - DNA, 1479 bp, Artificial Sequence
caggtccagctggtgcaatcgggtgggggagtggtgcaacctgggagatccttacggcttagttgcaaagcctccgggtatacgtttactaggtacaccatgcattgggtaagacaggcacctggaaagggactggaatggattggctacatcaaccccagtcgaggatataccaactacaatcagaaggtgaaggataggttcacaattagccgtgacaacagcaagaacaccgcctttctgcagatggattctctaagaccggaggatactggcgtctacttctgtgctcgctattatgacgaccactattccctggattattgggggcaaggcactccagtgaccgttagctctggaggagggggtagcggcggaggaggctctgggggaggggggtctgacatacagatgactcaatcccctagctcactgtcagcatcggttggcgacagagtgaccattacctgtagcgccagctctagtgtcagctacatgaactggtatcagcagacaccaggtaaagccccaaaaaggtggatctacgacacgagcaagttggcctctggtgtgcccagtcgcttctcagggtcaggttccgggactgattacacattcacaatcagctctctccaaccggaagacatagcgacttactattgccagcagtggtcatcgaatccattcacctttggccagggcactaagctacagattacacgggggggaggtggctcagacattcagatgacacaaagtcccgcttctctgagtgcttccctgggagaaaccgtgtctatcgagtgtctcgcgagtgaggacatttactcctatctggcatggtatcaacagaaacctgggaaatccccccagttgctgatctttgccgctaatcgactccaggatggcgtaccttcacgcttcagcggcagcggatccggaacgcagtttagtctcaagatatctgggatgcagccggaagatgagggggactatttctgcttacagggatctaaattcccctatacattcggccctggcaccaagctggagcttaatggcggtgggggtagtggtggtggcggttcgggaggcggtgggtcacaggtgcagcttcagcaatctggcgcagagttggtgaagccaggatcctcagtcaagatcagctgcaaggcttccggctatacctttaccaggaatttcattcactggatcaaacagcaacccggcaatggcctcgaatggatcgggtggatctttcccggggatggcgataccgagtacaaccagaagtttaacggcaaagccactcttacagccgacaaaagcagcagcacagcctacatgcagctctcctcactgacctccgaagactccgctgtgtacttttgcgcacggggaaactacaattacgagtacttcgattactggggccaaggcgtcatggttacggtatccagtcaccatcaccaccatcat

SEQ ID NO: 74 - DNA, 1347 bp, Artificial Sequence
caggtacagttgcagcaatctggggcagaactggtcaaacccgggagttctgtgaaaatctcctgtaaggccagtggatataccttcacccgtaatttcatccactggatcaaacaacagcctggcaatggcctcgaatggatcggatggatttttcccggtgatggcgataccgagtataaccagaagttcaatgggaaggcaacactaacagccgacaaatcctcatccacagcctatatgcaacttagtagcctcacatctgaagatagcgccgtgtacttttgcgcaaggggcaactataactacgagtatttcgactactggggtcagggggtgatggtgaccgtatcttccgctagtactaaaggacccagcgtgtttccactggcaccatcctctaaatctacaagcggaggcactgccgcacttggctgcctggtcaaagactattttcctgaacccgtcactgtgtcttggaactctggagctttgacatctggcgttcacacttttcccgcagtactccagtcatctggcctgtattctctgtcaagtgttgtgactgttcccagcagtagtctgggaacccagacctacatatgcaacgtcaaccataaacccagcaacacaaaggtggataagcgcgtcgagcctaagagctgcgataagacccatacatgcccaccatgtcccgctccagaggccgccggaggtccatccgtattcttgtttcctcccaaacccaaggataccctgatgatcagccggacacctgaagtcacttgtgtggttgtggacgtatcccatgaagatccagaggtgaagttcaactggtacgtcgacggtgtcgaagtccataatgccaaaaccaaacctagggaggaacagtacaacagtacctaccgagtagtgtcagtcctgactgtgttgcaccaggactggctgaatggtaaggagtacaagtgtaaggtgtccaataaggcccttcctgctcccattgaaaagaccatctccaaagcaaaagggcagccaagagagccccaggtgtatacactgcctccatgcagagaggagatgaccaagaatcaggttagtctgtggtgcctggttaaggggttttatccctcagatattgccgtggagtgggagtccaatggccaacccgagaataactacaagaccacgcctcccgtgcttgacagcgacgggagtttcttcctgtattccaagctgactgttgacaagtcccgttggcagcagggaaacgtgtttagctgttccgtgatgcacgaagccctgcacaaccactacacccagaaaagcctctctctctctccagggaag

SEQ ID NO: 75 - DNA, 2085 bp, Artificial Sequence
caggtccagttgcagcagagcggcgcggagctggtgaagcctggcagtagcgtcaagatctcttgcaaggcgagtggctataccttcacacggaacttcatccactggataaagcagcaacccggcaatggactagagtggattgggtggattttcccgggagatggcgataccgagtataaccagaagttcaatggtaaggcgacattaaccgccgataagtccagtagtaccgcctatatgcagttgtcttcattgacatctgaagactcagccgtgtatttttgcgctaggggcaactacaactatgagtactttgactactggggacaaggggtgatggtgactgtatcctccgcttccacaaagggtccatccgtatttccccttgctccaagcagcaaatcaacctctggtggtacagctgcccttggatgtcttgttaaggactattttcccgaaccggttacggtaagctggaacagtggcgcactgacatccggcgttcacacctttcctgccgtgcttcaaagtagcggactctattcactgagctccgtagtgaccgtaccatcctcctcccttgggacccagacttacatctgcaatgtgaaccataagccctctaataccaaggtcgacaagcgggtcgaacccaaatcgtgtgataagacccacacttgtcccccgtgtcctgctcctgaagccgcaggcgggccatccgtcttcctcttccctcccaaaccgaaggacacactgatgatctcccgtacgcctgaggtgacatgtgtggttgtcgatgtgagccatgaagatcctgaagtgaagtttaattggtatgttgacggagtcgaagtacacaacgcaaagaccaaacctagggaggagcagtataactccacataccgcgtcgtctcggtcttaactgtcctgcatcaggattggctgaatggcaaagagtacaagtgcaaggtttccaataaggcactacccgccccaatcgagaaaaccatcagcaaagccaaagggcagcctagagagccccaggtgtgcactttgcctcccagtagggaggaaatgaccaaaaatcaagtgtccctcagctgtgccgttaaaggcttttacccatctgacatagctgtggaatgggagtcaaacggacaaccagagaacaactataagacaacaccacccgtgctggactctgacgggtcattctttctggtgagcaaactcaccgtggacaaatctcgctggcaacaggggaatgtgttcagctgcagtgtgatgcatgaagcactgcacaaccactacacgcagaaaagcctctctctgtcacctgggaaagggggaggcggctcccaagttcagctcgttcagtccggagggggagtagtgcagccagggagaagccttcggctgagctgcaaagctagcggctacacttttacgcgatacaccatgcactgggttcgtcaggctcctggcaagggcctggagtggatcggctacatcaatccgagtcgagggtataccaactacaatcagaaagtcaaagatcgcttcacgatctcacgggacaactctaagaatacagcatttctccagatggattctttacggcctgaggatactggcgtgtacttttgcgccagatactatgacgatcactatagcctggactattggggtcaaggcactcccgtgacagtgtcctcagggggaggaggtagtggaggagggggttctgggggtggaggctcagatattcaaatgactcagtcaccctcctctctgagcgcgagcgtcggggacagagtgaccattacatgctctgcctctagtagcgtgagttacatgaactggtatcagcagacccccggaaaagccccaaagaggtggatctacgacacttcaaaactggcttcgggagtcccaagcagattctcaggttcgggctctggtacggattacaccttcaccataagcagtctacagccagaagacattgccacatactactgtcagcaatggtcctctaatcccttcacttttggtcagggcactaagctccagattacaagg

SEQ ID NO: 76 - DNA, 642 bp, Artificial Sequence
gatatacagatgacacagagccccgcaagcctatccgcctccctgggggagacagtgtctatagagtgcttagcttccgaggacatctatagctacttggcttggtatcagcaaaagcctgggaaatcaccacagctgttgatctttgcggccaacaggcttcaggacggagtccctagccggtttagtggatctggctcaggtacacagttcagtctgaagatctccgggatgcagcccgaagacgaaggagactacttctgcttgcagggatctaaattcccatacacttttggccctggcacgaaactggagttaaatcgcactgttgcagctccctcagtgttcatcttccctcccagcgatgagcagctgaaaagtggaactgccagtgttgtgtgcttgctgaacaacttttaccccagggaagccaaggtgcagtggaaggtagacaatgctcttcagtcagggaactctcaggaatccgtgactgagcaagacagcaaggattccacctacagtctcagcagcacactgaccctctccaaagcagactacgagaagcacaaggtgtatgcctgtgaggtaacccatcaagggcttagctccccagtcaccaagagtttcaataggggcgagtgt

SEQ ID NO: 77 - DNA, 2085 bp, Artificial Sequence
caagttcagcttcaacaaagtggtgcggagctagtgaaacccggatctagtgtcaagatctcttgtaaggcaagcggctatacgtttacccgcaacttcatacactggatcaaacagcaacctggtaatgggctggagtggatcgggtggatttttccgggagatggagacacagagtataatcagaaattcaatggcaaagctactctgacggccgataaaagctccagcacagcctacatgcagttatcttccctgacaagtgaggatagcgccgtgtacttttgcgcaagagggaactacaactacgagtatttcgactattggggccaaggcgtaatggtaaccgtatcctccgccagtacaaagggcccaagtgtgtttccactggcaccgtcttcaaagagcacatcaggtgggactgctgccttgggctgtctggtgaaggactactttccagaacccgtgaccgtgtcctggaatagtggggctttgacaagtggcgttcacacttttcccgctgtactgcagagttcagggctgtatagcttgtcgtccgttgtcactgttcctagcagcagcctaggaacccagacctacatttgcaatgtgaatcacaagccatctaataccaaggtggacaagagggtcgagccaaagtcttgcgacaagactcatacttgtcccccatgtccagcgcctgaagccgctggcggaccctctgtgtttctgttccctccaaagcccaaagatactctcatgatcagccggactccggaggtcacttgtgtcgttgtcgacgtgtcacatgaggatcctgaagtgaagttcaactggtatgtcgatggagtcgaggtgcacaatgccaagaccaaaccccgagaagagcagtacaacagcacataccgggtagtgtccgtgctgaccgtgctccatcaggattggttgaacggtaaggagtacaaatgcaaggtgagcaacaaagctctgccagcacccattgagaagaccatctccaaggccaaagggcagcctagagaaccccaagtgtacaccctccctccaagccgggaagagatgacaaagaatcaggttagcctcacatgccttgtcaagggcttttatccctccgacattgccgtagaatgggagtccaatggccaacccgaaaacaattacaaaaccacaccacccgtcctcgatagcgatggctccttctttctctactccaagttaacggttgacaaaagccggtggcagcaggggaatgtgttcagctgctccgtaatgcacgaggcccttcacaatcactatacccagaaatcgctgtctctttctcccgggaaaggcgggggcggatcacaggtgcaactcgtccagtctgggggaggtgtggtgcaacctggccggagtttacgactgagttgcaaggcatcgggctatacttttaccaggtatactatgcattgggtgagacaggcacccggcaaaggcctagaatggattggctacatcaacccttcaagggggtatactaactacaaccagaaggtgaaagacaggtttaccatatcgcgtgataacagcaaaaacacagccttcctgcagatggactcccttagacctgaagacacaggggtgtatttctgtgctcgttactacgacgaccactatagtctggactactgggggcagggtacaccggttaccgtttctagtggtggaggtggatcaggcggagggggatccggtggaggcggatccgatattcagatgacacagagcccctcttccctttccgcgtcagtgggagacagggtcaccattacctgttccgcctctagctccgtctcatacatgaactggtatcagcagacccctgggaaagcaccaaagcgctggatctatgatacgtcgaagttggcttctggagttccgtcacgcttctcaggatcaggttcaggtaccgactacacttttacgatctcttctctccagcctgaagatatagcgacgtactattgccagcagtggtctagtaaccctttcacattcggccaagggaccaaactgcagatcactcgc

SEQ ID NO: 78 - DNA, 1419 bp, Artificial Sequence
caggtccagttggtgcaatcgggcggcggcgttgtccagccgggtcgctctctacggctcagctgcaaagcaagtgggtatacctttactcgctatactatgcattgggtacgacaggctcccggtaaaggactggaatggattggctacatcaatcccagtcgcggctatacaaactacaaccaaaaggtcaaagacaggtttacgatttcccgggataactctaagaatacagcctttttgcagatggacagtctgaggccagaggatacaggcgtctacttttgtgccagatactatgacgatcactactcactcgactattggggccaagggacccccgtgactgtgagctcaggaggaggtggatctggcggcggagggagtgggggagggggttccgatatccagatgacccagtcccccagttcactgagcgcttctgtgggcgatcgggtcaccattacatgcagtgccagcagctccgtttcctacatgaattggtaccagcagacacccggaaaagcgccaaaacggtggatctatgacaccagtaaactggcaagcggcgtgcccagtcgattctcgggaagtgggtcaggtaccgactacacatttacgataagcagcctgcagcctgaggacatagccacatactactgccagcagtggtcgtcgaacccgtttactttcggccagggtacgaaactgcagattactcgagagcctaagagctgcgataagacccatacatgcccaccatgtcccgctccagaggccgccggaggtccatccgtattcttgtttcctcccaaacccaaggataccctgatgatcagccggacacctgaagtcacttgtgtggttgtggacgtatcccatgaagatccagaggtgaagttcaactggtacgtcgacggtgtcgaagtccataatgccaaaaccaaacctagggaggaacagtacaacagtacctaccgagtagtgtcagtcctgactgtgttgcaccaggactggctgaatggtaaggagtacaagtgtaaggtgtccaataaggcccttcctgctcccattgaaaagaccatctccaaagcaaaagggcagccaagagagccccaggtgtgtacactgcctccatctagagaggagatgaccaagaatcaggttagtctgagttgcgccgttaaggggttttatccctcagatattgccgtggagtgggagtccaatggccaacccgagaataactacaagaccacgcctcccgtgcttgacagcgacgggagtttcttcctggtttccaagctgactgttgacaagtcccgttggcagcagggaaacgtgtttagctgttccgtgatgcacgaagccctgcacaaccactacacccagaaaagcctctctctctctccagggaag

SEQ ID NO: 79 - DNA, 1422 bp, Artificial Sequence
caggtacagttgcagcaatctggggcagaactggtcaaacccgggagttctgtgaaaatctcctgtaaggccagtggatataccttcacccgtaatttcatccactggatcaaacaacagcctggcaatggcctcgaatggatcggatggatttttcccggtgatggcgataccgagtataaccagaagttcaatgggaaggcaacactaacagccgacaaatcctcatccacagcctatatgcaacttagtagcctcacatctgaagatagcgccgtgtacttttgcgcaaggggcaactataactacgagtatttcgactactggggtcagggggtgatggtgaccgtatcttccgctagtactaaaggacccagcgtgtttccactggcaccatcctctaaatctacaagcggaggcactgccgcacttggctgcctggtcaaagactattttcctgaacccgtcactgtgtcttggaactctggagctttgacatctggcgttcacacttttcccgcagtactccagtcatctggcctgtattctctgtcaagtgttgtgactgttcccagcagtagtctgggaacccagacctacatatgcaacgtcaaccataaacccagcaacacaaaggtggataagcgcgtcgagcctaagagctgcggaggtggaggctcacaggttcagctagttcagtcaggtgggggcgtagtgcaacccggaaggtcccttagactgagttgcaaagcttccggctatacatttacccggtatacgatgcattgggtgagacaagcgccaggcaaaggcttggaatggattggctacatcaacccttctcggggttatacaaactacaaccagaaggtgaaagatcggtttactatcagtcgcgacaacagcaaaaacaccgcatttctgcagatggacagccttagacccgaagacacaggcgtctatttctgtgccaggtattacgacgatcactacagcctagattactggggtcaaggcactcccgtcacagtgtctagcggaggtggaggctcagggggtggcgggtctggtggaggaggcagcgacatacagatgactcagtctcctagctccctttcagccagcgtaggcgatcgcgtgacaatcacttgtagcgccagcagctcagtgtcgtacatgaactggtatcagcagactcctgggaaagcccccaaacgatggatttatgacacatcaaagctggcatcaggggttccaagccgcttttccggcagtggtagtggaaccgactatacgttcacgatctcttccctccaaccagaggatattgccacttactactgtcaacagtggtcatctaatccgtttacctttggccaggggacgaaactccaaattaccaggcaccatcaccaccatcac

SEQ ID NO: 80 - DNA, 2085 bp, Artificial Sequence
caggtacagttgcagcaatctggggcagaactggtcaaacccgggagttctgtgaaaatctcctgtaaggccagtggatataccttcacccgtaatttcatccactggatcaaacaacagcctggcaatggcctcgaatggatcggatggatttttcccggtgatggcgataccgagtataaccagaagttcaatgggaaggcaacactaacagccgacaaatcctcatccacagcctatatgcaacttagtagcctcacatctgaagatagcgccgtgtacttttgcgcaaggggcaactataactacgagtatttcgactactggggtcagggggtgatggtgaccgtatcttccgctagtactaaaggacccagcgtgtttccactggcaccatcctctaaatctacaagcggaggcactgccgcacttggctgcctggtcaaagactattttcctgaacccgtcactgtgtcttggaactctggagctttgacatctggcgttcacacttttcccgcagtactccagtcatctggcctgtattctctgtcaagtgttgtgactgttcccagcagtagtctgggaacccagacctacatatgcaacgtcaaccataaacccagcaacacaaaggtggataagcgcgtcgagcctaagagctgcggaggtggaggctcacaggttcagctagttcagtcaggtgggggcgtagtgcaacccggaaggtcccttagactgagttgcaaagcttccggctatacatttacccggtatacgatgcattgggtgagacaagcgccaggcaaaggcttggaatggattggctacatcaacccttctcggggttatacaaactacaaccagaaggtgaaagatcggtttactatcagtcgcgacaacagcaaaaacaccgcatttctgcagatggacagccttagacccgaagacacaggcgtctatttctgtgccaggtattacgacgatcactacagcctagattactggggtcaaggcactcccgtcacagtgtctagcggaggtggaggctcagggggtggcgggtctggtggaggaggcagcgacatacagatgactcagtctcctagctccctttcagccagcgtaggcgatcgcgtgacaatcacttgtagcgccagcagctcagtgtcgtacatgaactggtatcagcagactcctgggaaagcccccaaacgatggatttatgacacatcaaagctggcatcaggggttccaagccgcttttccggcagtggtagtggaaccgactatacgttcacgatctcttccctccaaccagaggatattgccacttactactgtcaacagtggtcatctaatccgtttacctttggccaggggacgaaactccaaattaccagggataagacccatacatgcccaccatgtcccgctccagaggccgccggaggtccatccgtattcttgtttcctcccaaacccaaggataccctgatgatcagccggacacctgaagtcacttgtgtggttgtggacgtatcccatgaagatccagaggtgaagttcaactggtacgtcgacggtgtcgaagtccataatgccaaaaccaaacctagggaggaacagtacaacagtacctaccgagtagtgtcagtcctgactgtgttgcaccaggactggctgaatggtaaggagtacaagtgtaaggtgtccaataaggcccttcctgctcccattgaaaagaccatctccaaagcaaaagggcagccaagagagccccaggtgtatacactgcctccatctagagaggagatgaccaagaatcaggttagtctgacatgcctggttaaggggttttatccctcagatattgccgtggagtgggagtccaatggccaacccgagaataactacaagaccacgcctcccgtgcttgacagcgacgggagtttcttcctgtattccaagctgactgttgacaagtcccgttggcagcagggaaacgtgtttagctgttccgtgatgcacgaagccctgcacaaccactacacccagaaaagcctctctctctctccagggaag

SEQ ID NO: 81 - DNA, 1740 bp, Artificial Sequence
caggtacagttgcagcaatctggggcagaactggtcaaacccgggagttctgtgaaaatctcctgtaaggccagtggatataccttcacccgtaatttcatccactggatcaaacaacagcctggcaatggcctcgaatggatcggatggatttttcccggtgatggcgataccgagtataaccagaagttcaatgggaaggcaacactaacagccgacaaatcctcatccacagcctatatgcaacttagtagcctcacatctgaagatagcgccgtgtacttttgcgcaaggggcaactataactacgagtatttcgactactggggtcagggggtgatggtgaccgtatcttccgctagtactaaaggacccagcgtgtttccactggcaccatcctctaaatctacaagcggaggcactgccgcacttggctgcctggtcaaagactattttcctgaacccgtcactgtgtcttggaactctggagctttgacatctggcgttcacacttttcccgcagtactccagtcatctggcctgtattctctgtcaagtgttgtgactgttcccagcagtagtctgggaacccagacctacatatgcaacgtcaaccataaacccagcaacacaaaggtggataagcgcgtcgagcctaagagctgcggaggtggaggctcacaggttcagctagttcagtcaggtgggggcgtagtgcaacccggaaggtcccttagactgagttgcaaagcttccggctatacatttacccggtatacgatgcattgggtgagacaagcgccaggcaaaggcttggaatggattggctacatcaacccttctcggggttatacaaactacaaccagaaggtgaaagatcggtttactatcagtcgcgacaacagcaaaaacaccgcatttctgcagatggacagccttagacccgaagacacaggcgtctatttctgtgccaggtattacgacgatcactacagcctagattactggggtcaaggcactcccgtcacagtgtctagcggaggtggaggctcagggggtggcgggtctggtggaggaggcagcgacatacagatgactcagtctcctagctccctttcagccagcgtaggcgatcgcgtgacaatcacttgtagcgccagcagctcagtgtcgtacatgaactggtatcagcagactcctgggaaagcccccaaacgatggatttatgacacatcaaagctggcatcaggggttccaagccgcttttccggcagtggtagtggaaccgactatacgttcacgatctcttccctccaaccagaggatattgccacttactactgtcaacagtggtcatctaatccgtttacctttggccaggggacgaaactccaaattaccagggccgctgcaggcggtgggcagccaagagagccccaggtgtatacactgcctccatctagagaggagatgaccaagaatcaggttagtctgacatgcctggttaaggggttttatccctcagatattgccgtggagtgggagtccaatggccaacccgagaataactacaagaccacgcctcccgtgcttgacagcgacgggagtttcttcctgtattccaagctgactgttgacaagtcccgttggcagcagggaaacgtgtttagctgttccgtgatgcacgaagccctgcacaaccactacacccagaaaagcctctctctctctccagggaag

SEQ ID NO: 82 - DNA, 2103 bp, Artificial Sequence
caggtacagttgcagcaatctggggcagaactggtcaaacccgggagttctgtgaaaatctcctgtaaggccagtggatataccttcacccgtaatttcatccactggatcaaacaacagcctggcaatggcctcgaatggatcggatggatttttcccggtgatggcgataccgagtataaccagaagttcaatgggaaggcaacactaacagccgacaaatcctcatccacagcctatatgcaacttagtagcctcacatctgaagatagcgccgtgtacttttgcgcaaggggcaactataactacgagtatttcgactactggggtcagggggtgatggtgaccgtatcttccgctagtactaaaggacccagcgtgtttccactggcaccatcctctaaatctacaagcggaggcactgccgcacttggctgcctggtcaaagactattttcctgaacccgtcactgtgtcttggaactctggagctttgacatctggcgttcacacttttcccgcagtactccagtcatctggcctgtattctctgtcaagtgttgtgactgttcccagcagtagtctgggaacccagacctacatatgcaacgtcaaccataaacccagcaacacaaaggtggataagcgcgtcgagcctaagagctgcggaggtggaggctcacaggttcagctagttcagtcaggtgggggcgtagtgcaacccggaaggtcccttagactgagttgcaaagcttccggctatacatttacccggtatacgatgcattgggtgagacaagcgccaggcaaaggcttggaatggattggctacatcaacccttctcggggttatacaaactacaaccagaaggtgaaagatcggtttactatcagtcgcgacaacagcaaaaacaccgcatttctgcagatggacagccttagacccgaagacacaggcgtctatttctgtgccaggtattacgacgatcactacagcctagattactggggtcaaggcactcccgtcacagtgtctagcggaggtggaggctcagggggtggcgggtctggtggaggaggcagcgacatacagatgactcagtctcctagctccctttcagccagcgtaggcgatcgcgtgacaatcacttgtagcgccagcagctcagtgtcgtacatgaactggtatcagcagactcctgggaaagcccccaaacgatggatttatgacacatcaaagctggcatcaggggttccaagccgcttttccggcagtggtagtggaaccgactatacgttcacgatctcttccctccaaccagaggatattgccacttactactgtcaacagtggtcatctaatccgtttacctttggccaggggacgaaactccaaattaccaggggaggtggaggctcacaggtacagttgcagcaatctggggcagaactggtcaaacccgggagttctgtgaaaatctcctgtaaggccagtggatataccttcacccgtaatttcatccactggatcaaacaacagcctggcaatggcctcgaatggatcggatggatttttcccggtgatggcgataccgagtataaccagaagttcaatgggaaggcaacactaacagccgacaaatcctcatccacagcctatatgcaacttagtagcctcacatctgaagatagcgccgtgtacttttgcgcaaggggcaactataactacgagtatttcgactactggggtcagggggtgatggtgaccgtatcttccgctagtactaaaggacccagcgtgtttccactggcaccatcctctaaatctacaagcggaggcactgccgcacttggctgcctggtcaaagactattttcctgaacccgtcactgtgtcttggaactctggagctttgacatctggcgttcacacttttcccgcagtactccagtcatctggcctgtattctctgtcaagtgttgtgactgttcccagcagtagtctgggaacccagacctacatatgcaacgtcaaccataaacccagcaacacaaaggtggataagcgcgtcgagcctaagagctgccaccatcaccaccatcac

SEQ ID NO: 83 - DNA, 1422 bp, Artificial Sequence
caggttcaactcgtccagagtggaggcggggttgtacagccagggagaagcctcaggcttagttgtaaagcatctggctataccttcacacgctataccatgcactgggtgagacaggctccagggaagggactggagtggatagggtatatcaatccctctcgtggttatacaaactataaccagaaggtgaaggatcggttcactatcagccgagataattcaaagaacacagcatttctgcagatggatagcctgcgacctgaagataccggtgtctacttttgcgccaggtattacgacgatcattatagcttggactactggggccaaggcacccctgtgacggtttccagcggcggaggaggcagtggaggaggaggctccggaggtggcggatctgacatccaaatgacccaaagccccagttctttgagcgcctcagttggagatcgggtgaccattacttgcagcgccagcagtagcgtgtcttacatgaactggtatcagcagaccccggggaaggctccaaagcgctggatctacgatacgtccaagctggcttccggcgtgccctctagattctcagggtctggcagtggtactgactacactttcacgatctcctctttgcagccagaggatatagcgacctactactgtcagcagtggtcctctaatcccttcacttttggtcaaggtaccaagctgcagattacaagaggcggtggaggcagccaggtgcagctccagcagtcaggggccgagctggtaaaaccgggttcatcagtgaagattagctgcaaagcctccggttacacctttacaaggaacttcattcactggatcaagcagcaacccgggaatgggctcgagtggattgggtggatattcccaggggacggagacacagagtacaaccagaaatttaacggcaaagctacactgacagccgacaaatcatcaagtacagcatacatgcagctctcctcactgacttccgaggacagcgcggtgtacttctgtgcgcgcggaaattataactacgaatactttgactattggggtcaaggcgtgatggtaacagtcagttctgcatcaacgaaaggccctagcgtctttcctctggcccctagctctaagtctacttccggcggaacagccgctctggggtgtcttgtcaaggactatttccctgaacccgtcacagtgagctggaatagcggggcccttacttcaggcgtccacacctttcctgctgtgcttcagagttccggcctgtattccctgagttctgtggtcactgttccaagctccagcctggggacccagacctacatctgcaatgtgaatcataaaccgtccaacacgaaagtggataaacgggttgaacccaagagctgccaccatcaccatcatcac

SEQ ID NO: 84 - DNA, 2085 bp, Artificial Sequence
caggttcaactcgtccagagtggaggcggggttgtacagccagggagaagcctcaggcttagttgtaaagcatctggctataccttcacacgctataccatgcactgggtgagacaggctccagggaagggactggagtggatagggtatatcaatccctctcgtggttatacaaactataaccagaaggtgaaggatcggttcactatcagccgagataattcaaagaacacagcatttctgcagatggatagcctgcgacctgaagataccggtgtctacttttgcgccaggtattacgacgatcattatagcttggactactggggccaaggcacccctgtgacggtttccagcggcggaggaggcagtggaggaggaggctccggaggtggcggatctgacatccaaatgacccaaagccccagttctttgagcgcctcagttggagatcgggtgaccattacttgcagcgccagcagtagcgtgtcttacatgaactggtatcagcagaccccggggaaggctccaaagcgctggatctacgatacgtccaagctggcttccggcgtgccctctagattctcagggtctggcagtggtactgactacactttcacgatctcctctttgcagccagaggatatagcgacctactactgtcagcagtggtcctctaatcccttcacttttggtcaaggtaccaagctgcagattacaagaggcggtggaggcagccaggtgcagctccagcagtcaggggccgagctggtaaaaccgggttcatcagtgaagattagctgcaaagcctccggttacacctttacaaggaacttcattcactggatcaagcagcaacccgggaatgggctcgagtggattgggtggatattcccaggggacggagacacagagtacaaccagaaatttaacggcaaagctacactgacagccgacaaatcatcaagtacagcatacatgcagctctcctcactgacttccgaggacagcgcggtgtacttctgtgcgcgcggaaattataactacgaatactttgactattggggtcaaggcgtgatggtaacagtcagttctgcatcaacgaaaggccctagcgtctttcctctggcccctagctctaagtctacttccggcggaacagccgctctggggtgtcttgtcaaggactatttccctgaacccgtcacagtgagctggaatagcggggcccttacttcaggcgtccacacctttcctgctgtgcttcagagttccggcctgtattccctgagttctgtggtcactgttccaagctccagcctggggacccagacctacatctgcaatgtgaatcataaaccgtccaacacgaaagtggataaacgggttgaacccaagagctgcgataagacccatacatgcccaccatgtcccgctccagaggccgccggaggtccatccgtattcttgtttcctcccaaacccaaggataccctgatgatcagccggacacctgaagtcacttgtgtggttgtggacgtatcccatgaagatccagaggtgaagttcaactggtacgtcgacggtgtcgaagtccataatgccaaaaccaaacctagggaggaacagtacaacagtacctaccgagtagtgtcagtcctgactgtgttgcaccaggactggctgaatggtaaggagtacaagtgtaaggtgtccaataaggcccttcctgctcccattgaaaagaccatctccaaagcaaaagggcagccaagagagccccaggtgtatacactgcctccatctagagaggagatgaccaagaatcaggttagtctgacatgcctggttaaggggttttatccctcagatattgccgtggagtgggagtccaatggccaacccgagaataactacaagaccacgcctcccgtgcttgacagcgacgggagtttcttcctgtattccaagctgactgttgacaagtcccgttggcagcagggaaacgtgtttagctgttccgtgatgcacgaagccctgcacaaccactacacccagaaaagcctctctctctctccagggaag

SEQ ID NO: 85 - DNA, 1740 bp, Artificial Sequence
caggttcaactcgtccagagtggaggcggggttgtacagccagggagaagcctcaggcttagttgtaaagcatctggctataccttcacacgctataccatgcactgggtgagacaggctccagggaagggactggagtggatagggtatatcaatccctctcgtggttatacaaactataaccagaaggtgaaggatcggttcactatcagccgagataattcaaagaacacagcatttctgcagatggatagcctgcgacctgaagataccggtgtctacttttgcgccaggtattacgacgatcattatagcttggactactggggccaaggcacccctgtgacggtttccagcggcggaggaggcagtggaggaggaggctccggaggtggcggatctgacatccaaatgacccaaagccccagttctttgagcgcctcagttggagatcgggtgaccattacttgcagcgccagcagtagcgtgtcttacatgaactggtatcagcagaccccggggaaggctccaaagcgctggatctacgatacgtccaagctggcttccggcgtgccctctagattctcagggtctggcagtggtactgactacactttcacgatctcctctttgcagccagaggatatagcgacctactactgtcagcagtggtcctctaatcccttcacttttggtcaaggtaccaagctgcagattacaagaggcggtggaggcagccaggtgcagctccagcagtcaggggccgagctggtaaaaccgggttcatcagtgaagattagctgcaaagcctccggttacacctttacaaggaacttcattcactggatcaagcagcaacccgggaatgggctcgagtggattgggtggatattcccaggggacggagacacagagtacaaccagaaatttaacggcaaagctacactgacagccgacaaatcatcaagtacagcatacatgcagctctcctcactgacttccgaggacagcgcggtgtacttctgtgcgcgcggaaattataactacgaatactttgactattggggtcaaggcgtgatggtaacagtcagttctgcatcaacgaaaggccctagcgtctttcctctggcccctagctctaagtctacttccggcggaacagccgctctggggtgtcttgtcaaggactatttccctgaacccgtcacagtgagctggaatagcggggcccttacttcaggcgtccacacctttcctgctgtgcttcagagttccggcctgtattccctgagttctgtggtcactgttccaagctccagcctggggacccagacctacatctgcaatgtgaatcataaaccgtccaacacgaaagtggataaacgggttgaacccaagagctgcgctgcagccggaggcgggcagccaagagagccccaggtgtatacactgcctccatctagagaggagatgaccaagaatcaggttagtctgacatgcctggttaaggggttttatccctcagatattgccgtggagtgggagtccaatggccaacccgagaataactacaagaccacgcctcccgtgcttgacagcgacgggagtttcttcctgtattccaagctgactgttgacaagtcccgttggcagcagggaaacgtgtttagctgttccgtgatgcacgaagccctgcacaaccactacacccagaaaagcctctctctctctccagggaag

SEQ ID NO: 86 - DNA, 684 bp, Artificial Sequence
caggttcagcttcagcagtccggtgcagagctggtgaaaccagggtcatctgtgaagattagctgcaaagcctctggctatacctttacacgcaatttcatccactggatcaagcaacagcctggaaatggcctcgaatggattggctggatctttcctggagatggggataccgagtacaaccagaagttcaatggcaaagccacattgacagccgacaaatcctccagtaccgcctatatgcagctcagctctctgacttcagaggattccgctgtatacttctgtgcgagagggaactacaactatgagtacttcgattattggggtcaaggcgtcatggtgaccgtgagttcagccagcaccaagggaccatctgtgtttccactggcaccctccagcaagagtactagcggtggaactgctgcgttgggatgtctggtgaaggactactttcccgaaccggttactgtgagttggaactcaggcgcccttacgtccggcgtccacacctttcctgctgttctgcaaagctctgggctgtatagcctgtcaagcgtcgtgactgtgccttcctccagtctggggacacagacgtacatttgcaacgtcaatcacaaacccagcaataccaaggtcgacaaacgggttgaacccaagagctgccatcatcaccatcaccat

SEQ ID NO: 87 - DNA, 1380 bp, Artificial Sequence
caggtgcagctcgtccaaagcggcggaggtgtggtccaaccagggagatccctgaggctgtcctgcaaagccagtgggtacacattcacccgatatacaatgcactgggtacggcaagctcctggcaaaggcctggagtggataggctacatcaatccttcccgtggctatacgaactacaaccagaaagtgaaggaccggtttacgattagcagagacaactctaagaataccgcctttctgcagatggacagtctgcgaccagaggatactggcgtctatttctgtgctcgctattacgatgaccactattccctggattattggggccagggaacacctgtgacagtgagtagcggtggaggtgggtcaggaggtggagggagtggaggcggcggcagcgatatccagatgacgcagagtccttcatctttgtcagcctccgttggggacagggtcaccattacttgctcagccagcagctccgtgtcatacatgaattggtatcaacagactcccggcaaggctccaaaacggtggatttacgatacatccaaactggcaagcggtgtaccctccaggttttctggcagcgggtctggaacagactacaccttcaccattagctccttgcagccagaagatattgcaacctactactgtcagcagtggtctagcaacccctttaccttcgggcagggaaccaagctgcagataactcggggcggcggtggatctgacatccaaatgactcagtccccagctagcctgagtgctagccttggagagactgtgtcaatcgagtgtcttgcctctgaggacatctacagctatctcgcctggtaccaacagaagcccggaaagagccctcagctgctgatctttgccgccaatcgcctccaggatggcgtacctagccgtttctccggatcaggttcagggactcagttttcactgaagatatcaggtatgcagcccgaggacgaaggcgattacttttgcctgcaagggtctaagttcccgtatacttttgggcccggcaccaaattggagctgaacaggacagtcgcggcacctagtgtctttatcttcccacccagcgatgaacagctgaagtctgggaccgcaagcgttgtgtgcctgctgaataacttctatccgagagaagccaaggttcagtggaaagttgacaatgcgttgcagagtggcaatagccaggaatccgtgaccgagcaggattccaaagactccacatactctcttagtagcacactcaccctcagtaaagctgattacgagaagcacaaggtgtatgcctgtgaagtgacccatcaagggctttcttctccggtgacaaaatccttcaacagaggggaatgc

SEQ ID NO: 88 - DNA, 1347 bp, Artificial Sequence
caggtacagttgcagcaatctggggcagaactggtcaaacccgggagttctgtgaaaatctcctgtaaggccagtggatataccttcacccgtaatttcatccactggatcaaacaacagcctggcaatggcctcgaatggatcggatggatttttcccggtgatggcgataccgagtataaccagaagttcaatgggaaggcaacactaacagccgacaaatcctcatccacagcctatatgcaacttagtagcctcacatctgaagatagcgccgtgtacttttgcgcaaggggcaactataactacgagtatttcgactactggggtcagggggtgatggtgaccgtatcttccgctagtactaaaggacccagcgtgtttccactggcaccatcctctaaatctacaagcggaggcactgccgcacttggctgcctggtcaaagactattttcctgaacccgtcactgtgtcttggaactctggagctttgacatctggcgttcacacttttcccgcagtactccagtcatctggcctgtattctctgtcaagtgttgtgactgttcccagcagtagtctgggaacccagacctacatatgcaacgtcaaccataaacccagcaacacaaaggtggataagcgcgtcgagcctaagagctgcgataagacccatacatgcccaccatgtcccgctccagaggccgccggaggtccatccgtattcttgtttcctcccaaacccaaggataccctgatgatcagccggacacctgaagtcacttgtgtggttgtggacgtatcccatgaagatccagaggtgaagttcaactggtacgtcgacggtgtcgaagtccataatgccaaaaccaaacctagggaggaacagtacaacagtacctaccgagtagtgtcagtcctgactgtgttgcaccaggactggctgaatggtaaggagtacaagtgtaaggtgtccaataaggcccttcctgctcccattgaaaagaccatctccaaagcaaaagggcagccaagagagccccaggtgtatacactgcctccatctagagaggagatgaccaagaatcaggttagtctgacatgcctggttaaggggttttatccctcagatattgccgtggagtgggagtccaatggccaacccgagaataactacaagaccacgcctcccgtgcttgacagcgacgggagtttcttcctgtattccaagctgactgttgacaagtcccgttggcagcagggaaacgtgtttagctgttccgtgatgcacgaagccctgcacaaccactacacccagaaaagcctctctctctctccagggaag

SEQ ID NO: 89 - DNA, 1002 bp, Artificial Sequence
caggtacagttgcagcaatctggggcagaactggtcaaacccgggagttctgtgaaaatctcctgtaaggccagtggatataccttcacccgtaatttcatccactggatcaaacaacagcctggcaatggcctcgaatggatcggatggatttttcccggtgatggcgataccgagtataaccagaagttcaatgggaaggcaacactaacagccgacaaatcctcatccacagcctatatgcaacttagtagcctcacatctgaagatagcgccgtgtacttttgcgcaaggggcaactataactacgagtatttcgactactggggtcagggggtgatggtgaccgtatcttccgctagtactaaaggacccagcgtgtttccactggcaccatcctctaaatctacaagcggaggcactgccgcacttggctgcctggtcaaagactattttcctgaacccgtcactgtgtcttggaactctggagctttgacatctggcgttcacacttttcccgcagtactccagtcatctggcctgtattctctgtcaagtgttgtgactgttcccagcagtagtctgggaacccagacctacatatgcaacgtcaaccataaacccagcaacacaaaggtggataagcgcgtcgagcctaagagctgcgctgcagccggaggcgggcagccaagagagccccaggtgtatacactgcctccatctagagaggagatgaccaagaatcaggttagtctgacatgcctggttaaggggttttatccctcagatattgccgtggagtgggagtccaatggccaacccgagaataactacaagaccacgcctcccgtgcttgacagcgacgggagtttcttcctgtattccaagctgactgttgacaagtcccgttggcagcagggaaacgtgtttagctgttccgtgatgcacgaagccctgcacaaccactacacccagaaaagcctctctctctctccagggaag

SEQ ID NO: 90 - protein, 119 aa, Artificial Sequence
QVQLVQSGAEVKKPGASVKVSCKASGYTFTRNFIHWVRQAPGQGLEWMGWIFPGDGDTEYNQKFNGRVTMTRDTSISTAYMELSRLRSDDTAVYYCARGNYNYEYFDYWGQGTMVTVSS

SEQ ID NO: 91 - protein, 119 aa, Artificial Sequence
QVQLQESGAEVKKPGASVKVSCKASGYTFTRNFIHWVRQAPGQRLEWMGWIFPGDGDTEYNQKFNGRVTITRDTSASTAYMELSSLRSEDTAVYYCARGNYNYEYFDYWGQGTLVTVSS

SEQ ID NO: 92 - protein, 119 aa, Artificial Sequence
QVQLVQSGAEVKKPGASVKISCKASGYTFTRNFIHWVRQAPGQSLEWVGWIFPGDGDTEYNQKFNGRITITRDTSANTAYMELSSLKSEDTAVYYCARGNYNYEYFDYWGQGTLVTVSS

SEQ ID NO: 93 - protein, 119 aa, Artificial Sequence
QMQLVQSGAEVKKTGSSVKVSCKASGYTFTRNFIHWVRQAPGQALEWMGWIFPGDGDTEYNQKFNGRVTITRDRSMSTAYMELSSLRSEDTAMYYCARGNYNYEYFDYWGQGTLVTVSS

SEQ ID NO: 94 - protein, 119 aa, Artificial Sequence
QVQLVQSGAEVKKPGSSVKVSCKASGYTFTRNFIHWVRQQPGQGLEWMGWIFPGDGDTEYNQKFNGRVTITADKSTSTAYMQLSSLTSEDTAVYFCARGNYNYEYFDYWGQGVMVTVSS

SEQ ID NO: 95 - protein, 107 aa, Artificial Sequence
DIQMTQSPSFVSASVGDRVTITCLASEDIYSYLAWYQQKPGKAPKLLIFAANRLQDGVPSRFSGGGSGTGFTLTISSLQPEDFATYFCLQGSKFPYTFGQGTKLEIN

SEQ ID NO: 96 - protein, 107 aa, Artificial Sequence
DIQLTQSPAFLSASLGDRVTITCLASEDIYSYLAWYQQKPGKAPKLLISAANRLQDGVPSRFSGSGSGTEFTLTISSLQPEDFATYSCLQGSKFPYTFGQGTKLEIK

SEQ ID NO: 97 - protein, 107 aa, Artificial Sequence
DIQLTQSPSSLSASVGDRVTITCLASEDIYSYLAWYQQKPGKGPKLLIYAANRLQDGVPSRFSGSGSGTDFSLTISSLQPEDLATYYCLQGSKFPYTFGGGTKVEIK

SEQ ID NO: 98 - protein, 107 aa, Artificial Sequence
DIQMTQSPSSLSASVGDTVTIACLASEDIYSYLAWYQQKPGKAPKLLIYAANRLQDGVPSRFSGSGSFTDFTLTINSLQPDDSATYYCLQGSKFPYTFGGGTKVDIK

SEQ ID NO: 99 - protein, 107 aa, Artificial Sequence
DIQMTQSPSSVSASVGDSVTIECLASEDIYSYLAWYQQKPGKSPKLLIFAANRLQDGVPSRFSGSGSGTQFTLKISSLQPEDFAEYFCLQASKFPYTFGPGTKLELN

SEQ ID NO: 100 - DNA, 357 bp, Artificial Sequence
caggttcagctcgttcagtctggcgcggaagtcaagaaaccaggagcgtctgtgaaagtgagttgcaaagcatccggttacacgtttacccgcaacttcattcactgggttaggcaagcacctggccaagggttggagtggatgggatggatttttcctggagatggcgacactgagtacaaccagaagttcaatggcagagtgacaatgacacgcgatacatccatcagtacagcctacatggagctatcccggttacggtccgatgacactgccgtgtactactgtgccagagggaattacaactacgagtacttcgactattggggacaggggactatggtaaccgtgtcctca

SEQ ID NO: 101 - DNA, 357 bp, Artificial Sequence
caggttcagctgcaagaatcaggcgccgaagtcaagaaaccgggagcaagcgttaaggtgagttgtaaagcgtctggctatacattcacccgtaattttatccattgggtgagacaggcccctggccagcgcttagagtggatgggctggattttccccggcgacggcgatacggagtataaccagaagttcaatggacgggtgacaatcacaagagacactagcgcctcaaccgcgtacatggagctgagttccctccgatcagaggatacagccgtttactactgcgcaagggggaattacaactacgagtacttcgactattgggggcaggggactcttgtgacggtttcgtcc

SEQ ID NO: 102 - DNA, 357 bp, Artificial Sequence
caagtccagctggtacagtccggtgctgaagtaaagaaaccaggcgcctcagttaagatcagctgcaaggcttctggttacaccttcactcgcaacttcatccactgggtgagacaagcccctgggcagtctctcgaatgggttggctggatatttcccggggacggagatactgaatacaaccaaaagttcaatggccggattaccataacacgagatacttctgcgaatactgcctatatggaactgagctctcttaaaagcgaggacactgcagtctactattgcgctagagggaattacaattacgagtactttgactactggggacagggaacactggtgacagttagctcc

SEQ ID NO: 103 - DNA, 357 bp, Artificial Sequence
cagatgcagctcgtacagagcggtgccgaggtgaagaaaaccgggagcagcgttaaagtctcctgtaaagcctccggctacacctttacccggaatttcatccattgggtacggcaggcacccggccaagcactggaatggatggggtggatattcccgggtgacggagatactgagtacaaccagaagttcaatggaagagtgactattacgagagatcgctcaatgagtactgcgtatatggaactgtcctcattgcgcagcgaagatacggcgatgtattactgtgcacgcgggaactacaactacgagtacttcgattactggggccaagggacccttgtcacggtttcatcc

SEQ ID NO: 104 - DNA, 357 bp, Artificial Sequence
caggttcaactggttcagtcaggtgcagaggtaaagaagccagggagctcagtgaaagtctcatgcaaagccagcggatacacctttactcggaactttatccactgggtgagacagcagcctgggcaaggcttggagtggatgggctggatctttccaggcgatggagacaccgagtataaccagaagttcaatggcagagtgactattaccgccgataaaagcacatctacagcctatatgcagctgagcagcctgacaagtgaagataccgccgtctacttctgtgccagaggcaactacaactacgagtatttcgactactggggtcagggggtaatggtcacggtgagcagt

SEQ ID NO: 105 - DNA, 321 bp, Artificial Sequence
gacatccagatgacccaatccccttcattcgtgagtgcctcagtgggcgacagagtcaccattacgtgtcttgcttcagaggacatttacagctatctcgcatggtatcagcagaaacctgggaaagcacccaaactgctgatattcgctgccaatcggctgcaagatggcgtaccatccaggttttctggaggaggatctggtactgggtttaccctgactatcagctcccttcagcccgaggattttgccacatacttctgcctccaaggcagcaaattcccgtacacatttgggcagggtaccaagctggagatcaac

SEQ ID NO: 106 - DNA, 321 bp, Artificial Sequence
gacattcagctcactcagagtcctgcgtttctgtccgcatcacttggcgacagagtcaccatcacttgcttggccagtgaggacatctacagctatctggcttggtaccagcagaaacccggaaaagccccgaagctgttgatctctgctgcgaatcggttgcaggatggagtaccatcacgcttctcaggctctggaagcggtacagagttcacccttaccattagctctctccaacccgaagattttgccacctactcttgcctgcaagggagcaaattcccctatacctttggccaagggaccaaactggagattaag

SEQ ID NO: 107 - DNA, 321 bp, Artificial Sequence
gacattcagctgacccagtcaccaagctcactgagtgcttctgtgggtgatcgtgtgacgattacttgcctggctagtgaggacatctacagctacttggcctggtatcagcagaaacctgggaaaggccccaagctgctgatctacgctgccaataggctgcaagacggggtacctagccgcttttccggatctggctcaggcacagacttcagccttaccatatccagcctccaaccagaggatcttgccacctattactgccttcagggctccaagtttccctacacgtttggaggtggtactaaggtggagatcaaa

SEQ ID NO: 108 - DNA, 321 bp, Artificial Sequence
gacatccagatgactcaatccccaagcagtctgagcgcctctgtaggcgataccgtgacgattgcgtgtctggcttccgaggacatctacagttacctcgcatggtatcagcagaaaccggggaaagcacctaagctgctgatttatgcggctaacagactgcaggatggcgtacccagtcgcttctcaggttccggcagctttaccgactttaccctgaccatcaacagccttcagcccgatgatagcgccacttactactgtctgcaaggctctaagttcccctatacgtttggaggaggcactaaggtcgacataaag

SEQ ID NO: 109 - DNA, 321 bp, Artificial Sequence
gatatccagatgacacagagccctagcagcgttagcgcatcagtaggggacagtgtgaccattgaatgccttgcaagcgaggacatctacagctatttggcgtggtatcagcaaaagccaggcaaatctcccaaactgctcattttcgccgccaataggctccaagatggtgtcccttcccgattttccgggtcaggctcaggaacccagttcacactgaagatttcctctcttcagccagaggactttgcagagtacttctgtctccaggccagtaagtttccctacacctttgggcctggaacgaaactggaactgaat

SEQ ID NO: 110 - protein, 472 aa, Artificial Sequence
QVTLKESGPVLVKPTETLTLTCTVSGYSITSDYAWNWIRQPPGKALEWLAYISYSGSTSYNPSLKSRLSITKDTSKSQVVLTMTNMDPVDTATYYCARDPPYYYGSWGQGTTVTVSSASTKGPSVFPLAPSSKSTSGGTAALGCLVKDYFPEPVTVSWNSGALTSGVHTFPAVLQSSGLYSLSSVVTVPSSSLGTQTYICNVNHKPSNTKVDKRVEPKSCGGGGSQVQLVQSGGGVVQPGRSLRLSCKASGYTFTRYTMHWVRQAPGKGLEWIGYINPSRGYTNYNQKVKDRFTISRDNSKNTAFLQMDSLRPEDTGVYFCARYYDDHYSLDYWGQGTPVTVSSGGGGSGGGGSGGGGSDIQMTQSPSSLSASVGDRVTITCSASSSVSYMNWYQQTPGKAPKRWIYDTSKLASGVPSRFSGSGSGTDYTFTISSLQPEDIATYYCQQWSSNPFTFGQGTKLQITRHHHHHH

SEQ ID NO: 111 - protein, 219 aa, Artificial Sequence
DVVMTQSPLSLPVTLGQPASISCKSSQSLLDSDGKTYLNWLQQRPGQSPRRLIYLVSKLDSGVPDRFSGSGSGTDFTLKISRVEAEDVGVYHCWQGTHFPYTFGGGTKVEIKRTVAAPSVFIFPPSDEQLKSGTASVVCLLNNFYPREAKVQWKVDNALQSGNSQESVTEQDSKDSTYSLSSTLTLSKADYEKHKVYACEVTHQGLSSPVTKSFNRGEC

SEQ ID NO: 112 - protein, 468 aa, Artificial Sequence
QVQLVQSGAEVKKPGASVKVSCKASGYSFTGYYIHWVRQAPGQGLEWIGYISAYNGASSYNQKFKGRATFTVDTSISTAYMELSRLRSDDTAVYYCASSMDYWGQGTLVTVSSASTKGPSVFPLAPSSKSTSGGTAALGCLVKDYFPEPVTVSWNSGALTSGVHTFPAVLQSSGLYSLSSVVTVPSSSLGTQTYICNVNHKPSNTKVDKRVEPKSCGGGGSQVQLVQSGGGVVQPGRSLRLSCKASGYTFTRYTMHWVRQAPGKGLEWIGYINPSRGYTNYNQKVKDRFTISRDNSKNTAFLQMDSLRPEDTGVYFCARYYDDHYSLDYWGQGTPVTVSSGGGGSGGGGSGGGGSDIQMTQSPSSLSASVGDRVTITCSASSSVSYMNWYQQTPGKAPKRWIYDTSKLASGVPSRFSGSGSGTDYTFTISSLQPEDIATYYCQQWSSNPFTFGQGTKLQITRHHHHHH

SEQ ID NO: 113 - protein, 219 aa, Artificial Sequence
DVVMTQSPLSLPVTLGQPASISCKSSQSLLDSDGKTYLNWLQQRPGQSPKRLIYLVSKLDSGVPDRFSGSGSGTDFTLKISRVEAEDVGVYHCWQGTHFPYTFGQGTKLEIKRTVAAPSVFIFPPSDEQLKSGTASVVCLLNNFYPREAKVQWKVDNALQSGNSQESVTEQDSKDSTYSLSSTLTLSKADYEKHKVYACEVTHQGLSSPVTKSFNRGEC

SEQ ID NO: 114 - protein, 471 aa, Artificial Sequence
DVQLKLQESGPGLVKNSQSLSLTCTVTGYSITSDYAWNWIRQFPGNKLEWMGYISYSGSTSYNPSLKSRISITRDTSKNQFFLQLNSVTPEDTATYYCARDPPYYYGSNGTLTVSSASTKGPSVFPLAPSSKSTSGGTAALGCLVKDYFPEPVTVSWNSGALTSGVHTFPAVLQSSGLYSLSSVVTVPSSSLGTQTYICNVNHKPSNTKVDKRVEPKSCGGGGSQVQLVQSGGGVVQPGRSLRLSCKASGYTFTRYTMHWVRQAPGKGLEWIGYINPSRGYTNYNQKVKDRFTISRDNSKNTAFLQMDSLRPEDTGVYFCARYYDDHYSLDYWGQGTPVTVSSGGGGSGGGGSGGGGSDIQMTQSPSSLSASVGDRVTITCSASSSVSYMNWYQQTPGKAPKRWIYDTSKLASGVPSRFSGSGSGTDYTFTISSLQPEDIATYYCQQWSSNPFTFGQGTKLQITRHHHHHH

SEQ ID NO: 115 - protein, 219 aa, Artificial Sequence
DVVMTQTPLTLSVTIGQPASISCKSSQSLLDSDGKTYLNWLLQRPGQSPKRLIYLVSKLDSGVPDRFTGSGSGTDFTLKISRVEAEDLGVYHCWQGTHFPYTFGGGTKLEIKRTVAAPSVFIFPPSDEQLKSGTASVVCLLNNFYPREAKVQWKVDNALQSGNSQESVTEQDSKDSTYSLSSTLTLSKADYEKHKVYACEVTHQGLSSPVTKSFNRGEC

SEQ ID NO: 116 - protein, 474 aa, Artificial Sequence
QVQLVQSGAEVKKPGASVKVSCKASGYTFTRNFIHWVRQAPGQGLEWMGWIFPGDGDTEYNQKFNGRVTMTRDTSISTAYMELSRLRSDDTAVYYCARGNYNYEYFDYWGQGTMVTVSSASTKGPSVFPLAPSSKSTSGGTAALGCLVKDYFPEPVTVSWNSGALTSGVHTFPAVLQSSGLYSLSSVVTVPSSSLGTQTYICNVNHKPSNTKVDKRVEPKSCGGGGSQVQLVQSGGGVVQPGRSLRLSCKASGYTFTRYTMHWVRQAPGKGLEWIGYINPSRGYTNYNQKVKDRFTISRDNSKNTAFLQMDSLRPEDTGVYFCARYYDDHYSLDYWGQGTPVTVSSGGGGSGGGGSGGGGSDIQMTQSPSSLSASVGDRVTITCSASSSVSYMNWYQQTPGKAPKRWIYDTSKLASGVPSRFSGSGSGTDYTFTISSLQPEDIATYYCQQWSSNPFTFGQGTKLQITRHHHHHH

SEQ ID NO: 117 - protein, 474 aa, Artificial Sequence
QVQLQESGAEVKKPGASVKVSCKASGYTFTRNFIHWVRQAPGQRLEWMGWIFPGDGDTEYNQKFNGRVTITRDTSASTAYMELSSLRSEDTAVYYCARGNYNYEYFDYWGQGTLVTVSSASTKGPSVFPLAPSSKSTSGGTAALGCLVKDYFPEPVTVSWNSGALTSGVHTFPAVLQSSGLYSLSSVVTVPSSSLGTQTYICNVNHKPSNTKVDKRVEPKSCGGGGSQVQLVQSGGGVVQPGRSLRLSCKASGYTFTRYTMHWVRQAPGKGLEWIGYINPSRGYTNYNQKVKDRFTISRDNSKNTAFLQMDSLRPEDTGVYFCARYYDDHYSLDYWGQGTPVTVSSGGGGSGGGGSGGGGSDIQMTQSPSSLSASVGDRVTITCSASSSVSYMNWYQQTPGKAPKRWIYDTSKLASGVPSRFSGSGSGTDYTFTISSLQPEDIATYYCQQWSSNPFTFGQGTKLQITRHHHHHH

SEQ ID NO: 118 - protein, 474 aa, Artificial Sequence
QVQLVQSGAEVKKPGASVKISCKASGYTFTRNFIHWVRQAPGQSLEWVGWIFPGDGDTEYNQKFNGRITITRDTSANTAYMELSSLKSEDTAVYYCARGNYNYEYFDYWGQGTLVTVSSASTKGPSVFPLAPSSKSTSGGTAALGCLVKDYFPEPVTVSWNSGALTSGVHTFPAVLQSSGLYSLSSVVTVPSSSLGTQTYICNVNHKPSNTKVDKRVEPKSCGGGGSQVQLVQSGGGVVQPGRSLRLSCKASGYTFTRYTMHWVRQAPGKGLEWIGYINPSRGYTNYNQKVKDRFTISRDNSKNTAFLQMDSLRPEDTGVYFCARYYDDHYSLDYWGQGTPVTVSSGGGGSGGGGSGGGGSDIQMTQSPSSLSASVGDRVTITCSASSSVSYMNWYQQTPGKAPKRWIYDTSKLASGVPSRFSGSGSGTDYTFTISSLQPEDIATYYCQQWSSNPFTFGQGTKLQITRHHHHHH

SEQ ID NO: 119 - protein, 474 aa, Artificial Sequence
QMQLVQSGAEVKKTGSSVKVSCKASGYTFTRNFIHWVRQAPGQALEWMGWIFPGDGDTEYNQKFNGRVTITRDRSMSTAYMELSSLRSEDTAMYYCARGNYNYEYFDYWGQGTLVTVSSASTKGPSVFPLAPSSKSTSGGTAALGCLVKDYFPEPVTVSWNSGALTSGVHTFPAVLQSSGLYSLSSVVTVPSSSLGTQTYICNVNHKPSNTKVDKRVEPKSCGGGGSQVQLVQSGGGVVQPGRSLRLSCKASGYTFTRYTMHWVRQAPGKGLEWIGYINPSRGYTNYNQKVKDRFTISRDNSKNTAFLQMDSLRPEDTGVYFCARYYDDHYSLDYWGQGTPVTVSSGGGGSGGGGSGGGGSDIQMTQSPSSLSASVGDRVTITCSASSSVSYMNWYQQTPGKAPKRWIYDTSKLASGVPSRFSGSGSGTDYTFTISSLQPEDIATYYCQQWSSNPFTFGQGTKLQITRHHHHHH

SEQ ID NO: 120 - protein, 474 aa, Artificial Sequence
QVQLVQSGAEVKKPGSSVKVSCKASGYTFTRNFIHWVRQQPGQGLEWMGWIFPGDGDTEYNQKFNGRVTITADKSTSTAYMQLSSLTSEDTAVYFCARGNYNYEYFDYWGQGVMVTVSSASTKGPSVFPLAPSSKSTSGGTAALGCLVKDYFPEPVTVSWNSGALTSGVHTFPAVLQSSGLYSLSSVVTVPSSSLGTQTYICNVNHKPSNTKVDKRVEPKSCGGGGSQVQLVQSGGGVVQPGRSLRLSCKASGYTFTRYTMHWVRQAPGKGLEWIGYINPSRGYTNYNQKVKDRFTISRDNSKNTAFLQMDSLRPEDTGVYFCARYYDDHYSLDYWGQGTPVTVSSGGGGSGGGGSGGGGSDIQMTQSPSSLSASVGDRVTITCSASSSVSYMNWYQQTPGKAPKRWIYDTSKLASGVPSRFSGSGSGTDYTFTISSLQPEDIATYYCQQWSSNPFTFGQGTKLQITRHHHHHH

SEQ ID NO: 121 - protein, 214 aa, Artificial Sequence
DIQMTQSPSFVSASVGDRVTITCLASEDIYSYLAWYQQKPGKAPKLLIFAANRLQDGVPSRFSGGGSGTGFTLTISSLQPEDFATYFCLQGSKFPYTFGQGTKLEINRTVAAPSVFIFPPSDEQLKSGTASVVCLLNNFYPREAKVQWKVDNALQSGNSQESVTEQDSKDSTYSLSSTLTLSKADYEKHKVYACEVTHQGLSSPVTKSFNRGEC

SEQ ID NO: 122 - protein, 214 aa, Artificial Sequence
DIQLTQSPAFLSASLGDRVTITCLASEDIYSYLAWYQQKPGKAPKLLISAANRLQDGVPSRFSGSGSGTEFTLTISSLQPEDFATYSCLQGSKFPYTFGQGTKLEIKRTVAAPSVFIFPPSDEQLKSGTASVVCLLNNFYPREAKVQWKVDNALQSGNSQESVTEQDSKDSTYSLSSTLTLSKADYEKHKVYACEVTHQGLSSPVTKSFNRGEC

SEQ ID NO: 123 - protein, 214 aa, Artificial Sequence
DIQLTQSPSSLSASVGDRVTITCLASEDIYSYLAWYQQKPGKGPKLLIYAANRLQDGVPSRFSGSGSGTDFSLTISSLQPEDLATYYCLQGSKFPYTFGGGTKVEIKRTVAAPSVFIFPPSDEQLKSGTASVVCLLNNFYPREAKVQWKVDNALQSGNSQESVTEQDSKDSTYSLSSTLTLSKADYEKHKVYACEVTHQGLSSPVTKSFNRGEC

SEQ ID NO: 124 - protein, 214 aa, Artificial Sequence
DIQMTQSPSSLSASVGDTVTIACLASEDIYSYLAWYQQKPGKAPKLLIYAANRLQDGVPSRFSGSGSFTDFTLTINSLQPDDSATYYCLQGSKFPYTFGGGTKVDIKRTVAAPSVFIFPPSDEQLKSGTASVVCLLNNFYPREAKVQWKVDNALQSGNSQESVTEQDSKDSTYSLSSTLTLSKADYEKHKVYACEVTHQGLSSPVTKSFNRGEC

SEQ ID NO: 125 - protein, 214 aa, Artificial Sequence
DIQMTQSPSSVSASVGDSVTIECLASEDIYSYLAWYQQKPGKSPKLLIFAANRLQDGVPSRFSGSGSGTQFTLKISSLQPEDFAEYFCLQASKFPYTFGPGTKLELNRTVAAPSVFIFPPSDEQLKSGTASVVCLLNNFYPREAKVQWKVDNALQSGNSQESVTEQDSKDSTYSLSSTLTLSKADYEKHKVYACEVTHQGLSSPVTKSFNRGEC

SEQ ID NO: 126 - protein, 17 aa, Artificial Sequence
WIFPGDADTEYNQKFSG

SEQ ID NO: 127 - protein, 7 aa, Artificial Sequence
AANRLQS

SEQ ID NO: 128 - protein, 17 aa, Artificial Sequence
YINPSMGATNYNQKVKD

SEQ ID NO: 129 - protein, 10 aa, Artificial Sequence
YYNDHYSLDY

SEQ ID NO: 130 - protein, 10 aa, Artificial Sequence
YYDDHFSLDY

SEQ ID NO: 131 - protein, 10 aa, Artificial Sequence
SASSSVAYMN

SEQ ID NO: 132 - protein, 7 aa, Artificial Sequence
NTSKLAS

SEQ ID NO: 133 - protein, 119 aa, Artificial Sequence
QMQLVQSGAEVKKTGSSVKVSCKASGYTFTRNFIHWVRQAPGQALEWMGWIFPGDADTEYNQKFSGRVTITRDRSMSTAYMELSSLRSEDTAMYYCARGNYNYEYFDYWGQGTLVTVSS

SEQ ID NO: 134 - protein, 119 aa, Artificial Sequence
QVQLVQSGAEVKKPGSSVKVSCKASGYTFTRNFIHWIRQAPGQGLEWIGWIFPGDADTEYNQKFSGRATITADKSTSTAYMELSSLRSEDTAVYYCARGNYNYEYFDYWGQGTMVTVSS

SEQ ID NO: 135 - protein, 119 aa, Artificial Sequence
QVQLVQSGAEVKKPGSSVKVSCKASGYTFTRNFIHWIRQAPGQGLEWIGWIFPGDADTEYNQKFSGRVTITADKSTSTAYMELSSLRSEDTAVYYCARGNYNYEYFDYWGQGTMVTVSS

SEQ ID NO: 136 - protein, 119 aa, Artificial Sequence
QVQLVQSGAEVKKPGSSVKVSCKASGYTFTRNFIHWIRQAPGQGLEWIGWIFPGDGDTEYNQKFNGRATITADKSTSTAYMELSSLRSEDTAVYYCARGNYNYEYFDYWGQGTMVTVSS

SEQ ID NO: 137 - protein, 107 aa, Artificial Sequence
DIQMTQSPSFVSASVGDRVTITCLASEDIYSYLAWYQQKPGKAPKLLIFAANRLQSGVPSRFSGGGSGTGFTLTISSLQPEDFATYFCLQGSKFPYTFGQGTKLEIN

SEQ ID NO: 138 - protein, 107 aa, Artificial Sequence
DIQMTQSPSFVSASVGDRVTITCLASEDIYSYLAWYQQKPGKAPKLLIFAANRLQSGVPSRFSGGGSGTGFTLTISSLQPEDFATYFCLQGSKFPYTFGQGTKLEIK

SEQ ID NO: 139 - protein, 107 aa, Artificial Sequence
DIQMTQSPSFVSASVGDRVTITCLASEDIYSYLAWYQQKPGKAPKLLIFAANRLQDGVPSRFSGGGSGTGFTLTISSLQPEDFATYFCLQGSKFPYTFGQGTKLEIK

SEQ ID NO: 140 - protein, 107 aa, Artificial Sequence
DIQMTQSPSSLSASVGDRVTITCLASEDIYSYLAWYQQKPGKAPKLLIFAANRLQDGVPSRFSGSGSGTDFTLTISSLQPEDFATYYCLQGSKFPYTFGPGTKVDIK

SEQ ID NO: 141 - protein, 107 aa, Artificial Sequence
DIQMTQSPSSLSASVGDRVTITCLASEDIYSYLAWYQQKPGKAPKLLIFAANRLQSGVPSRFSGSGSGTDFTLTISSLQPEDFATYYCLQGSKFPYTFGPGTKVDIK

SEQ ID NO: 142 - DNA, 357 bp, Artificial Sequence
caaatgcagctcgtacagtcgggagcagaagtcaagaagaccggcagctcagttaaggtgtcgtgcaaagcctctggatatacattcacgcggaatttcattcactgggtgagacaggcaccaggccaggccttggaatggatgggctggatttttcctggggatgccgacacagagtataaccagaaattctcgggcagggtaacaattactcgggatagatcaatgtctacggcgtatatggagctcagcagcctgagatccgaagatacagccatgtattactgtgccagaggcaattacaattatgagtacttcgactattggggccaagggacactggtcaccgtttcatcc

SEQ ID NO: 143 - DNA, 357 bp, Artificial Sequence
caagttcagctggttcaatctggggctgaagtcaagaagcctgggtcctcagtgaaagtttcctgcaaggcttctggctacaccttcacccgtaactttatccactggatcagacaggcacctggacaaggccttgagtggattgggtggatttttcctggagatgcagatacagagtacaatcaaaagttcagtgggagagcaacaatcacagcagacaaatcaaccagcacagcctatatggagctcagcagcctgagatctgaggacactgcagtctattactgtgcaagaggaaattacaactacgagtactttgattactggggccaaggaaccatggtcacagtctcctca

SEQ ID NO: 144 - DNA, 357 bp, Artificial Sequence
caagttcagctggttcaatctggggctgaagtcaagaagcctgggtcctcagtgaaagtttcctgcaaggcttctggctacaccttcacccgtaactttatccactggatcagacaggcacctggacaaggccttgagtggattgggtggatttttcctggagatgcagatacagagtacaatcaaaagttcagtgggagagtgacaatcacagcagacaaatcaaccagcacagcctatatggagctcagcagcctgagatctgaggacactgcagtctattactgtgcaagaggaaattacaactacgagtactttgattactggggccaaggaaccatggtcacagtctcctca

SEQ ID NO: 145 - DNA, 357 bp, Artificial Sequence
caagttcagctggttcaatctggggctgaagtcaagaagcctgggtcctcagtgaaagtttcctgcaaggcttctggctacaccttcacccgtaactttatccactggatcagacaggcacctggacaaggccttgagtggattgggtggatttttcctggagatggagatacagagtacaatcaaaagttcaatgggagagcaacaatcacagcagacaaatcaaccagcacagcctatatggagctcagcagcctgagatctgaggacactgcagtctattactgtgcaagaggaaattacaactacgagtactttgattactggggccaaggaaccatggtcacagtctcctca

SEQ ID NO: 146 - DNA, 321 bp, Artificial Sequence
gacatccagatgacccaatccccttcattcgtgagtgcctcagtgggcgacagagtcaccattacgtgtcttgcttcagaggacatttacagctatctcgcatggtatcagcagaaacctgggaaagcacccaaactgctgatattcgctgccaatcggctgcaaagcggcgtaccatccaggttttctggaggaggatctggtactgggtttaccctgactatcagctcccttcagcccgaggattttgccacatacttctgcctccaaggcagcaaattcccgtacacatttgggcagggtaccaagctggagatcaac

SEQ ID NO: 147 - DNA, 321 bp, Artificial Sequence
gacatccagatgacccaatccccttcattcgtgagtgcctcagtgggcgacagagtcaccattacgtgtcttgcttcagaggacatttacagctatctcgcatggtatcagcagaaacctgggaaagcacccaaactgctgatattcgctgccaatcggctgcaaagcggcgtaccatccaggttttctggaggaggatctggtactgggtttaccctgactatcagctcccttcagcccgaggattttgccacatacttctgcctccaaggcagcaaattcccgtacacatttgggcagggtaccaagctggagatcaag

SEQ ID NO: 148 - DNA, 321 bp, Artificial Sequence
gacatccagatgacccaatccccttcattcgtgagtgcctcagtgggcgacagagtcaccattacgtgtcttgcttcagaggacatttacagctatctcgcatggtatcagcagaaacctgggaaagcacccaaactgctgatattcgctgccaatcggctgcaagatggcgtaccatccaggttttctggaggaggatctggtactgggtttaccctgactatcagctcccttcagcccgaggattttgccacatacttctgcctccaaggcagcaaattcccgtacacatttgggcagggtaccaagctggagatcaag

SEQ ID NO: 149 - DNA, 321 bp, Artificial Sequence
gacatccagatgacacagtctccatcttccctgtctgcatctgtgggagacagagtcaccatcacttgtctggcaagcgaggacatttacagttatcttgcatggtatcaacagaagccagggaaagctcctaagctcctgatctttgctgcaaataggctgcaagatggggtcccatcacggttcagtggcagtggatctggcacagactttactctcaccatcagcagtctgcaacctgaagatttcgcaacttattactgtcttcagggttccaagtttccctacacctttggacctgggaccaaggtggacatcaaa

SEQ ID NO: 150 - DNA, 321 bp, Artificial Sequence
gacatccagatgacacagtctccatcttccctgtctgcatctgtgggagacagagtcaccatcacttgtctggcaagcgaggacatttacagttatcttgcatggtatcaacagaagccagggaaagctcctaagctcctgatctttgctgcaaataggctgcaaagcggggtcccatcacggttcagtggcagtggatctggcacagactttactctcaccatcagcagtctgcaacctgaagatttcgcaacttattactgtcttcagggttccaagtttccctacacctttggacctgggaccaaggtggacatcaaa

SEQ ID NO: 151 - protein, 695 aa, Artificial Sequence
QMQLVQSGAEVKKTGSSVKVSCKASGYTFTRNFIHWVRQAPGQALEWMGWIFPGDGDTEYNQKFNGRVTITRDRSMSTAYMELSSLRSEDTAMYYCARGNYNYEYFDYWGQGTLVTVSSASTKGPSVFPLAPSSKSTSGGTAALGCLVKDYFPEPVTVSWNSGALTSGVHTFPAVLQSSGLYSLSSVVTVPSSSLGTQTYICNVNHKPSNTKVDKRVEPKSCGGGGSQVQLVQSGGGVVQPGRSLRLSCKASGYTFTRYTMHWVRQAPGKGLEWIGYINPSRGYTNYNQKVKDRFTISRDNSKNTAFLQMDSLRPEDTGVYFCARYYDDHYSLDYWGQGTPVTVSSGGGGSGGGGSGGGGSDIQMTQSPSSLSASVGDRVTITCSASSSVSYMNWYQQTPGKAPKRWIYDTSKLASGVPSRFSGSGSGTDYTFTISSLQPEDIATYYCQQWSSNPFTFGQGTKLQITRDKTHTCPPCPAPEAAGGPSVFLFPPKPKDTLMISRTPEVTCVVVDVSHEDPEVKFNWYVDGVEVHNAKTKPREEQYNSTYRVVSVLTVLHQDWLNGKEYKCKVSNKALPAPIEKTISKAKGQPREPQVYTLPPSREEMTKNQVSLTCLVKGFYPSDIAVEWESNGQPENNYKTTPPVLDSDGSFFLYSKLTVDKSRWQQGNVFSCSVMHEALHNHYTQKSLSLSPGK

SEQ ID NO: 152 - protein, 695 aa, Artificial Sequence
QMQLVQSGAEVKKTGSSVKVSCKASGYTFTRNFIHWVRQAPGQALEWMGWIFPGDGDTEYNQKFNGRVTITRDRSMSTAYMELSSLRSEDTAMYYCARGNYNYEYFDYWGQGTLVTVSSASTKGPSVFPLAPSSKSTSGGTAALGCLVKDYFPEPVTVSWNSGALTSGVHTFPAVLQSSGLYSLSSVVTVPSSSLGTQTYICNVNHKPSNTKVDKRVEPKSCGGGGSQVQLVQSGGGVVQPGRSLRLSCKASGYTFTRYTMHWVRQAPGKGLEWIGYINPSRGYTNYNQKVKDRFTISRDNSKNTAFLQMDSLRPEDTGVYFCARYYDDHYSLDYWGQGTPVTVSSGGGGSGGGGSGGGGSDIQMTQSPSSLSASVGDRVTITCSASSSVAYMNWYQQTPGKAPKRWIYDTSKLASGVPSRFSGSGSGTDYTFTISSLQPEDIATYYCQQWSSNPFTFGQGTKLQITRDKTHTCPPCPAPEAAGGPSVFLFPPKPKDTLMISRTPEVTCVVVDVSHEDPEVKFNWYVDGVEVHNAKTKPREEQYNSTYRVVSVLTVLHQDWLNGKEYKCKVSNKALPAPIEKTISKAKGQPREPQVYTLPPSREEMTKNQVSLTCLVKGFYPSDIAVEWESNGQPENNYKTTPPVLDSDGSFFLYSKLTVDKSRWQQGNVFSCSVMHEALHNHYTQKSLSLSPGK

SEQ ID NO: 153 - protein, 695 aa, Artificial Sequence
QMQLVQSGAEVKKTGSSVKVSCKASGYTFTRNFIHWVRQAPGQALEWMGWIFPGDGDTEYNQKFNGRVTITRDRSMSTAYMELSSLRSEDTAMYYCARGNYNYEYFDYWGQGTLVTVSSASTKGPSVFPLAPSSKSTSGGTAALGCLVKDYFPEPVTVSWNSGALTSGVHTFPAVLQSSGLYSLSSVVTVPSSSLGTQTYICNVNHKPSNTKVDKRVEPKSCGGGGSQVQLVQSGGGVVQPGRSLRLSCKASGYTFTRYTMHWVRQAPGKGLEWIGYINPSRGYTNYNQKVKDRFTISRDNSKNTAFLQMDSLRPEDTGVYFCARYYDDHYSLDYWGQGTPVTVSSGGGGSGGGGSGGGGSDIQMTQSPSSLSASVGDRVTITCSASSSVSYMNWYQQTPGKAPKRWIYNTSKLASGVPSRFSGSGSGTDYTFTISSLQPEDIATYYCQQWSSNPFTFGQGTKLQITRDKTHTCPPCPAPEAAGGPSVFLFPPKPKDTLMISRTPEVTCVVVDVSHEDPEVKFNWYVDGVEVHNAKTKPREEQYNSTYRVVSVLTVLHQDWLNGKEYKCKVSNKALPAPIEKTISKAKGQPREPQVYTLPPSREEMTKNQVSLTCLVKGFYPSDIAVEWESNGQPENNYKTTPPVLDSDGSFFLYSKLTVDKSRWQQGNVFSCSVMHEALHNHYTQKSLSLSPGK

SEQ ID NO: 154 - protein, 695 aa, Artificial Sequence
QMQLVQSGAEVKKTGSSVKVSCKASGYTFTRNFIHWVRQAPGQALEWMGWIFPGDGDTEYNQKFNGRVTITRDRSMSTAYMELSSLRSEDTAMYYCARGNYNYEYFDYWGQGTLVTVSSASTKGPSVFPLAPSSKSTSGGTAALGCLVKDYFPEPVTVSWNSGALTSGVHTFPAVLQSSGLYSLSSVVTVPSSSLGTQTYICNVNHKPSNTKVDKRVEPKSCGGGGSQVQLVQSGGGVVQPGRSLRLSCKASGYTFTRYTMHWVRQAPGKGLEWIGYINPSRGYTNYNQKVKDRFTISRDNSKNTAFLQMDSLRPEDTGVYFCARYYNDHYSLDYWGQGTPVTVSSGGGGSGGGGSGGGGSDIQMTQSPSSLSASVGDRVTITCSASSSVSYMNWYQQTPGKAPKRWIYDTSKLASGVPSRFSGSGSGTDYTFTISSLQPEDIATYYCQQWSSNPFTFGQGTKLQITRDKTHTCPPCPAPEAAGGPSVFLFPPKPKDTLMISRTPEVTCVVVDVSHEDPEVKFNWYVDGVEVHNAKTKPREEQYNSTYRVVSVLTVLHQDWLNGKEYKCKVSNKALPAPIEKTISKAKGQPREPQVYTLPPSREEMTKNQVSLTCLVKGFYPSDIAVEWESNGQPENNYKTTPPVLDSDGSFFLYSKLTVDKSRWQQGNVFSCSVMHEALHNHYTQKSLSLSPGK

SEQ ID NO: 155 - protein, 695 aa, Artificial Sequence
QMQLVQSGAEVKKTGSSVKVSCKASGYTFTRNFIHWVRQAPGQALEWMGWIFPGDGDTEYNQKFNGRVTITRDRSMSTAYMELSSLRSEDTAMYYCARGNYNYEYFDYWGQGTLVTVSSASTKGPSVFPLAPSSKSTSGGTAALGCLVKDYFPEPVTVSWNSGALTSGVHTFPAVLQSSGLYSLSSVVTVPSSSLGTQTYICNVNHKPSNTKVDKRVEPKSCGGGGSQVQLVQSGGGVVQPGRSLRLSCKASGYTFTRYTMHWVRQAPGKGLEWIGYINPSRGYTNYNQKVKDRFTISRDNSKNTAFLQMDSLRPEDTGVYFCARYYDDHFSLDYWGQGTPVTVSSGGGGSGGGGSGGGGSDIQMTQSPSSLSASVGDRVTITCSASSSVSYMNWYQQTPGKAPKRWIYDTSKLASGVPSRFSGSGSGTDYTFTISSLQPEDIATYYCQQWSSNPFTFGQGTKLQITRDKTHTCPPCPAPEAAGGPSVFLFPPKPKDTLMISRTPEVTCVVVDVSHEDPEVKFNWYVDGVEVHNAKTKPREEQYNSTYRVVSVLTVLHQDWLNGKEYKCKVSNKALPAPIEKTISKAKGQPREPQVYTLPPSREEMTKNQVSLTCLVKGFYPSDIAVEWESNGQPENNYKTTPPVLDSDGSFFLYSKLTVDKSRWQQGNVFSCSVMHEALHNHYTQKSLSLSPGK

SEQ ID NO: 156 - protein, 695 aa, Artificial Sequence
QMQLVQSGAEVKKTGSSVKVSCKASGYTFTRNFIHWVRQAPGQALEWMGWIFPGDGDTEYNQKFNGRVTITRDRSMSTAYMELSSLRSEDTAMYYCARGNYNYEYFDYWGQGTLVTVSSASTKGPSVFPLAPSSKSTSGGTAALGCLVKDYFPEPVTVSWNSGALTSGVHTFPAVLQSSGLYSLSSVVTVPSSSLGTQTYICNVNHKPSNTKVDKRVEPKSCGGGGSQVQLVQSGGGVVQPGRSLRLSCKASGYTFTRYTMHWVRQAPGKGLEWIGYINPSMGATNYNQKVKDRFTISRDNSKNTAFLQMDSLRPEDTGVYFCARYYDDHYSLDYWGQGTPVTVSSGGGGSGGGGSGGGGSDIQMTQSPSSLSASVGDRVTITCSASSSVSYMNWYQQTPGKAPKRWIYDTSKLASGVPSRFSGSGSGTDYTFTISSLQPEDIATYYCQQWSSNPFTFGQGTKLQITRDKTHTCPPCPAPEAAGGPSVFLFPPKPKDTLMISRTPEVTCVVVDVSHEDPEVKFNWYVDGVEVHNAKTKPREEQYNSTYRVVSVLTVLHQDWLNGKEYKCKVSNKALPAPIEKTISKAKGQPREPQVYTLPPSREEMTKNQVSLTCLVKGFYPSDIAVEWESNGQPENNYKTTPPVLDSDGSFFLYSKLTVDKSRWQQGNVFSCSVMHEALHNHYTQKSLSLSPGK

SEQ ID NO: 157 - protein, 695 aa, Artificial Sequence
QMQLVQSGAEVKKTGSSVKVSCKASGYTFTRNFIHWVRQAPGQALEWMGWIFPGDADTEYNQKFSGRVTITRDRSMSTAYMELSSLRSEDTAMYYCARGNYNYEYFDYWGQGTLVTVSSASTKGPSVFPLAPSSKSTSGGTAALGCLVKDYFPEPVTVSWNSGALTSGVHTFPAVLQSSGLYSLSSVVTVPSSSLGTQTYICNVNHKPSNTKVDKRVEPKSCGGGGSQVQLVQSGGGVVQPGRSLRLSCKASGYTFTRYTMHWVRQAPGKGLEWIGYINPSRGYTNYNQKVKDRFTISRDNSKNTAFLQMDSLRPEDTGVYFCARYYDDHYSLDYWGQGTPVTVSSGGGGSGGGGSGGGGSDIQMTQSPSSLSASVGDRVTITCSASSSVSYMNWYQQTPGKAPKRWIYDTSKLASGVPSRFSGSGSGTDYTFTISSLQPEDIATYYCQQWSSNPFTFGQGTKLQITRDKTHTCPPCPAPEAAGGPSVFLFPPKPKDTLMISRTPEVTCVVVDVSHEDPEVKFNWYVDGVEVHNAKTKPREEQYNSTYRVVSVLTVLHQDWLNGKEYKCKVSNKALPAPIEKTISKAKGQPREPQVYTLPPSREEMTKNQVSLTCLVKGFYPSDIAVEWESNGQPENNYKTTPPVLDSDGSFFLYSKLTVDKSRWQQGNVFSCSVMHEALHNHYTQKSLSLSPGK

SEQ ID NO: 158 - protein, 695 aa, Artificial Sequence
QMQLVQSGAEVKKTGSSVKVSCKASGYTFTRNFIHWVRQAPGQALEWMGWIFPGDADTEYNQKFSGRVTITRDRSMSTAYMELSSLRSEDTAMYYCARGNYNYEYFDYWGQGTLVTVSSASTKGPSVFPLAPSSKSTSGGTAALGCLVKDYFPEPVTVSWNSGALTSGVHTFPAVLQSSGLYSLSSVVTVPSSSLGTQTYICNVNHKPSNTKVDKRVEPKSCGGGGSQVQLVQSGGGVVQPGRSLRLSCKASGYTFTRYTMHWVRQAPGKGLEWIGYINPSRGYTNYNQKVKDRFTISRDNSKNTAFLQMDSLRPEDTGVYFCARYYDDHYSLDYWGQGTPVTVSSGGGGSGGGGSGGGGSDIQMTQSPSSLSASVGDRVTITCSASSSVAYMNWYQQTPGKAPKRWIYDTSKLASGVPSRFSGSGSGTDYTFTISSLQPEDIATYYCQQWSSNPFTFGQGTKLQITRDKTHTCPPCPAPEAAGGPSVFLFPPKPKDTLMISRTPEVTCVVVDVSHEDPEVKFNWYVDGVEVHNAKTKPREEQYNSTYRVVSVLTVLHQDWLNGKEYKCKVSNKALPAPIEKTISKAKGQPREPQVYTLPPSREEMTKNQVSLTCLVKGFYPSDIAVEWESNGQPENNYKTTPPVLDSDGSFFLYSKLTVDKSRWQQGNVFSCSVMHEALHNHYTQKSLSLSPGK

SEQ ID NO: 159 - protein, 695 aa, Artificial Sequence
QMQLVQSGAEVKKTGSSVKVSCKASGYTFTRNFIHWVRQAPGQALEWMGWIFPGDADTEYNQKFSGRVTITRDRSMSTAYMELSSLRSEDTAMYYCARGNYNYEYFDYWGQGTLVTVSSASTKGPSVFPLAPSSKSTSGGTAALGCLVKDYFPEPVTVSWNSGALTSGVHTFPAVLQSSGLYSLSSVVTVPSSSLGTQTYICNVNHKPSNTKVDKRVEPKSCGGGGSQVQLVQSGGGVVQPGRSLRLSCKASGYTFTRYTMHWVRQAPGKGLEWIGYINPSRGYTNYNQKVKDRFTISRDNSKNTAFLQMDSLRPEDTGVYFCARYYDDHYSLDYWGQGTPVTVSSGGGGSGGGGSGGGGSDIQMTQSPSSLSASVGDRVTITCSASSSVSYMNWYQQTPGKAPKRWIYNTSKLASGVPSRFSGSGSGTDYTFTISSLQPEDIATYYCQQWSSNPFTFGQGTKLQITRDKTHTCPPCPAPEAAGGPSVFLFPPKPKDTLMISRTPEVTCVVVDVSHEDPEVKFNWYVDGVEVHNAKTKPREEQYNSTYRVVSVLTVLHQDWLNGKEYKCKVSNKALPAPIEKTISKAKGQPREPQVYTLPPSREEMTKNQVSLTCLVKGFYPSDIAVEWESNGQPENNYKTTPPVLDSDGSFFLYSKLTVDKSRWQQGNVFSCSVMHEALHNHYTQKSLSLSPGK

SEQ ID NO: 160 - protein, 695 aa, Artificial Sequence
QMQLVQSGAEVKKTGSSVKVSCKASGYTFTRNFIHWVRQAPGQALEWMGWIFPGDADTEYNQKFSGRVTITRDRSMSTAYMELSSLRSEDTAMYYCARGNYNYEYFDYWGQGTLVTVSSASTKGPSVFPLAPSSKSTSGGTAALGCLVKDYFPEPVTVSWNSGALTSGVHTFPAVLQSSGLYSLSSVVTVPSSSLGTQTYICNVNHKPSNTKVDKRVEPKSCGGGGSQVQLVQSGGGVVQPGRSLRLSCKASGYTFTRYTMHWVRQAPGKGLEWIGYINPSRGYTNYNQKVKDRFTISRDNSKNTAFLQMDSLRPEDTGVYFCARYYNDHYSLDYWGQGTPVTVSSGGGGSGGGGSGGGGSDIQMTQSPSSLSASVGDRVTITCSASSSVSYMNWYQQTPGKAPKRWIYDTSKLASGVPSRFSGSGSGTDYTFTISSLQPEDIATYYCQQWSSNPFTFGQGTKLQITRDKTHTCPPCPAPEAAGGPSVFLFPPKPKDTLMISRTPEVTCVVVDVSHEDPEVKFNWYVDGVEVHNAKTKPREEQYNSTYRVVSVLTVLHQDWLNGKEYKCKVSNKALPAPIEKTISKAKGQPREPQVYTLPPSREEMTKNQVSLTCLVKGFYPSDIAVEWESNGQPENNYKTTPPVLDSDGSFFLYSKLTVDKSRWQQGNVFSCSVMHEALHNHYTQKSLSLSPGK

SEQ ID NO: 161 - protein, 695 aa, Artificial Sequence
QMQLVQSGAEVKKTGSSVKVSCKASGYTFTRNFIHWVRQAPGQALEWMGWIFPGDADTEYNQKFSGRVTITRDRSMSTAYMELSSLRSEDTAMYYCARGNYNYEYFDYWGQGTLVTVSSASTKGPSVFPLAPSSKSTSGGTAALGCLVKDYFPEPVTVSWNSGALTSGVHTFPAVLQSSGLYSLSSVVTVPSSSLGTQTYICNVNHKPSNTKVDKRVEPKSCGGGGSQVQLVQSGGGVVQPGRSLRLSCKASGYTFTRYTMHWVRQAPGKGLEWIGYINPSRGYTNYNQKVKDRFTISRDNSKNTAFLQMDSLRPEDTGVYFCARYYDDHFSLDYWGQGTPVTVSSGGGGSGGGGSGGGGSDIQMTQSPSSLSASVGDRVTITCSASSSVSYMNWYQQTPGKAPKRWIYDTSKLASGVPSRFSGSGSGTDYTFTISSLQPEDIATYYCQQWSSNPFTFGQGTKLQITRDKTHTCPPCPAPEAAGGPSVFLFPPKPKDTLMISRTPEVTCVVVDVSHEDPEVKFNWYVDGVEVHNAKTKPREEQYNSTYRVVSVLTVLHQDWLNGKEYKCKVSNKALPAPIEKTISKAKGQPREPQVYTLPPSREEMTKNQVSLTCLVKGFYPSDIAVEWESNGQPENNYKTTPPVLDSDGSFFLYSKLTVDKSRWQQGNVFSCSVMHEALHNHYTQKSLSLSPGK

SEQ ID NO: 162 - protein, 695 aa, Artificial Sequence
QMQLVQSGAEVKKTGSSVKVSCKASGYTFTRNFIHWVRQAPGQALEWMGWIFPGDADTEYNQKFSGRVTITRDRSMSTAYMELSSLRSEDTAMYYCARGNYNYEYFDYWGQGTLVTVSSASTKGPSVFPLAPSSKSTSGGTAALGCLVKDYFPEPVTVSWNSGALTSGVHTFPAVLQSSGLYSLSSVVTVPSSSLGTQTYICNVNHKPSNTKVDKRVEPKSCGGGGSQVQLVQSGGGVVQPGRSLRLSCKASGYTFTRYTMHWVRQAPGKGLEWIGYINPSMGATNYNQKVKDRFTISRDNSKNTAFLQMDSLRPEDTGVYFCARYYDDHYSLDYWGQGTPVTVSSGGGGSGGGGSGGGGSDIQMTQSPSSLSASVGDRVTITCSASSSVSYMNWYQQTPGKAPKRWIYDTSKLASGVPSRFSGSGSGTDYTFTISSLQPEDIATYYCQQWSSNPFTFGQGTKLQITRDKTHTCPPCPAPEAAGGPSVFLFPPKPKDTLMISRTPEVTCVVVDVSHEDPEVKFNWYVDGVEVHNAKTKPREEQYNSTYRVVSVLTVLHQDWLNGKEYKCKVSNKALPAPIEKTISKAKGQPREPQVYTLPPSREEMTKNQVSLTCLVKGFYPSDIAVEWESNGQPENNYKTTPPVLDSDGSFFLYSKLTVDKSRWQQGNVFSCSVMHEALHNHYTQKSLSLSPGK

SEQ ID NO: 163 - protein, 449 aa, Artificial Sequence
QMQLVQSGAEVKKTGSSVKVSCKASGYTFTRNFIHWVRQAPGQALEWMGWIFPGDGDTEYNQKFNGRVTITRDRSMSTAYMELSSLRSEDTAMYYCARGNYNYEYFDYWGQGTLVTVSSASTKGPSVFPLAPSSKSTSGGTAALGCLVKDYFPEPVTVSWNSGALTSGVHTFPAVLQSSGLYSLSSVVTVPSSSLGTQTYICNVNHKPSNTKVDKRVEPKSCDKTHTCPPCPAPEAAGGPSVFLFPPKPKDTLMISRTPEVTCVVVDVSHEDPEVKFNWYVDGVEVHNAKTKPREEQYNSTYRVVSVLTVLHQDWLNGKEYKCKVSNKALPAPIEKTISKAKGQPREPQVYTLPPSREEMTKNQVSLTCLVKGFYPSDIAVEWESNGQPENNYKTTPPVLDSDGSFFLYSKLTVDKSRWQQGNVFSCSVMHEALHNHYTQKSLSLSPGK

SEQ ID NO: 164 - protein, 449 aa, Artificial Sequence
QMQLVQSGAEVKKTGSSVKVSCKASGYTFTRNFIHWVRQAPGQALEWMGWIFPGDADTEYNQKFSGRVTITRDRSMSTAYMELSSLRSEDTAMYYCARGNYNYEYFDYWGQGTLVTVSSASTKGPSVFPLAPSSKSTSGGTAALGCLVKDYFPEPVTVSWNSGALTSGVHTFPAVLQSSGLYSLSSVVTVPSSSLGTQTYICNVNHKPSNTKVDKRVEPKSCDKTHTCPPCPAPEAAGGPSVFLFPPKPKDTLMISRTPEVTCVVVDVSHEDPEVKFNWYVDGVEVHNAKTKPREEQYNSTYRVVSVLTVLHQDWLNGKEYKCKVSNKALPAPIEKTISKAKGQPREPQVYTLPPSREEMTKNQVSLTCLVKGFYPSDIAVEWESNGQPENNYKTTPPVLDSDGSFFLYSKLTVDKSRWQQGNVFSCSVMHEALHNHYTQKSLSLSPGK

SEQ ID NO: 165 - protein, 214 aa, Artificial Sequence
DIQMTQSPSFVSASVGDRVTITCLASEDIYSYLAWYQQKPGKAPKLLIFAANRLQSGVPSRFSGGGSGTGFTLTISSLQPEDFATYFCLQGSKFPYTFGQGTKLEINRTVAAPSVFIFPPSDEQLKSGTASVVCLLNNFYPREAKVQWKVDNALQSGNSQESVTEQDSKDSTYSLSSTLTLSKADYEKHKVYACEVTHQGLSSPVTKSFNRGEC

SEQ ID NO: 166 - protein, 214 aa, Artificial Sequence
DIQMTQSPSFVSASVGDRVTITCLASEDIYSYLAWYQQKPGKAPKLLIFAANRLQDGVPSRFSGGGSGTGFTLTISSLQPEDFATYFCLQGSKFPYTFGQGTKLEIKRTVAAPSVFIFPPSDEQLKSGTASVVCLLNNFYPREAKVQWKVDNALQSGNSQESVTEQDSKDSTYSLSSTLTLSKADYEKHKVYACEVTHQGLSSPVTKSFNRGEC

SEQ ID NO: 167 - protein, 214 aa, Artificial Sequence
DIQMTQSPSFVSASVGDRVTITCLASEDIYSYLAWYQQKPGKAPKLLIFAANRLQSGVPSRFSGGGSGTGFTLTISSLQPEDFATYFCLQGSKFPYTFGQGTKLEIKRTVAAPSVFIFPPSDEQLKSGTASVVCLLNNFYPREAKVQWKVDNALQSGNSQESVTEQDSKDSTYSLSSTLTLSKADYEKHKVYACEVTHQGLSSPVTKSFNRGEC

SEQ ID NO: 168 - protein, 465 aa, Artificial Sequence
DIQMTQSPSFVSASVGDRVTITCLASEDIYSYLAWYQQKPGKAPKLLIFAANRLQDGVPSRFSGGGSGTGFTLTISSLQPEDFATYFCLQGSKFPYTFGQGTKLEINRTVAAPSVFIFPPSDEQLKSGTASVVCLLNNFYPREAKVQWKVDNALQSGNSQESVTEQDSKDSTYSLSSTLTLSKADYEKHKVYACEVTHQGLSSPVTKSFNRGECGGGGSGGGGSQVQLVQSGGGVVQPGRSLRLSCKASGYTFTRYTMHWVRQAPGKGLEWIGYINPSRGYTNYNQKVKDRFTISRDNSKNTAFLQMDSLRPEDTGVYFCARYYDDHYSLDYWGQGTPVTVSSGGGGSGGGGSGGGGSDIQMTQSPSSLSASVGDRVTITCSASSSVSYMNWYQQTPGKAPKRWIYDTSKLASGVPSRFSGSGSGTDYTFTISSLQPEDIATYYCQQWSSNPFTFGQGTKLQITR

SEQ ID NO: 169 - protein, 465 aa, Artificial Sequence
DIQMTQSPSFVSASVGDRVTITCLASEDIYSYLAWYQQKPGKAPKLLIFAANRLQSGVPSRFSGGGSGTGFTLTISSLQPEDFATYFCLQGSKFPYTFGQGTKLEINRTVAAPSVFIFPPSDEQLKSGTASVVCLLNNFYPREAKVQWKVDNALQSGNSQESVTEQDSKDSTYSLSSTLTLSKADYEKHKVYACEVTHQGLSSPVTKSFNRGECGGGGSGGGGSQVQLVQSGGGVVQPGRSLRLSCKASGYTFTRYTMHWVRQAPGKGLEWIGYINPSRGYTNYNQKVKDRFTISRDNSKNTAFLQMDSLRPEDTGVYFCARYYDDHYSLDYWGQGTPVTVSSGGGGSGGGGSGGGGSDIQMTQSPSSLSASVGDRVTITCSASSSVSYMNWYQQTPGKAPKRWIYDTSKLASGVPSRFSGSGSGTDYTFTISSLQPEDIATYYCQQWSSNPFTFGQGTKLQITR

SEQ ID NO: 170 - protein, 695 aa, Artificial Sequence
QVQLVQSGAEVKKPGSSVKVSCKASGYTFTRNFIHWIRQAPGQGLEWIGWIFPGDADTEYNQKFSGRATITADKSTSTAYMELSSLRSEDTAVYYCARGNYNYEYFDYWGQGTMVTVSSASTKGPSVFPLAPSSKSTSGGTAALGCLVKDYFPEPVTVSWNSGALTSGVHTFPAVLQSSGLYSLSSVVTVPSSSLGTQTYICNVNHKPSNTKVDKRVEPKSCGGGGSQVQLVQSGGGVVQPGRSLRLSCKASGYTFTRYTMHWVRQAPGKGLEWIGYINPSRGYTNYNQKVKDRFTISRDNSKNTAFLQMDSLRPEDTGVYFCARYYDDHYSLDYWGQGTPVTVSSGGGGSGGGGSGGGGSDIQMTQSPSSLSASVGDRVTITCSASSSVSYMNWYQQTPGKAPKRWIYDTSKLASGVPSRFSGSGSGTDYTFTISSLQPEDIATYYCQQWSSNPFTFGQGTKLQITRDKTHTCPPCPAPEAAGGPSVFLFPPKPKDTLMISRTPEVTCVVVDVSHEDPEVKFNWYVDGVEVHNAKTKPREEQYNSTYRVVSVLTVLHQDWLNGKEYKCKVSNKALPAPIEKTISKAKGQPREPQVYTLPPSREEMTKNQVSLTCLVKGFYPSDIAVEWESNGQPENNYKTTPPVLDSDGSFFLYSKLTVDKSRWQQGNVFSCSVMHEALHNHYTQKSLSLSPGK

SEQ ID NO: 171 - protein, 695 aa, Artificial Sequence
QVQLVQSGAEVKKPGSSVKVSCKASGYTFTRNFIHWIRQAPGQGLEWIGWIFPGDADTEYNQKFSGRATITADKSTSTAYMELSSLRSEDTAVYYCARGNYNYEYFDYWGQGTMVTVSSASTKGPSVFPLAPSSKSTSGGTAALGCLVKDYFPEPVTVSWNSGALTSGVHTFPAVLQSSGLYSLSSVVTVPSSSLGTQTYICNVNHKPSNTKVDKRVEPKSCGGGGSQVQLVQSGGGVVQPGRSLRLSCKASGYTFTRYTMHWVRQAPGKGLEWIGYINPSRGYTNYNQKVKDRFTISRDNSKNTAFLQMDSLRPEDTGVYFCARYYDDHYSLDYWGQGTPVTVSSGGGGSGGGGSGGGGSDIQMTQSPSSLSASVGDRVTITCSASSSVAYMNWYQQTPGKAPKRWIYDTSKLASGVPSRFSGSGSGTDYTFTISSLQPEDIATYYCQQWSSNPFTFGQGTKLQITRDKTHTCPPCPAPEAAGGPSVFLFPPKPKDTLMISRTPEVTCVVVDVSHEDPEVKFNWYVDGVEVHNAKTKPREEQYNSTYRVVSVLTVLHQDWLNGKEYKCKVSNKALPAPIEKTISKAKGQPREPQVYTLPPSREEMTKNQVSLTCLVKGFYPSDIAVEWESNGQPENNYKTTPPVLDSDGSFFLYSKLTVDKSRWQQGNVFSCSVMHEALHNHYTQKSLSLSPGK

SEQ ID NO: 172 - protein, 695 aa, Artificial Sequence
QVQLVQSGAEVKKPGSSVKVSCKASGYTFTRNFIHWIRQAPGQGLEWIGWIFPGDADTEYNQKFSGRATITADKSTSTAYMELSSLRSEDTAVYYCARGNYNYEYFDYWGQGTMVTVSSASTKGPSVFPLAPSSKSTSGGTAALGCLVKDYFPEPVTVSWNSGALTSGVHTFPAVLQSSGLYSLSSVVTVPSSSLGTQTYICNVNHKPSNTKVDKRVEPKSCGGGGSQVQLVQSGGGVVQPGRSLRLSCKASGYTFTRYTMHWVRQAPGKGLEWIGYINPSRGYTNYNQKVKDRFTISRDNSKNTAFLQMDSLRPEDTGVYFCARYYDDHYSLDYWGQGTPVTVSSGGGGSGGGGSGGGGSDIQMTQSPSSLSASVGDRVTITCSASSSVSYMNWYQQTPGKAPKRWIYNTSKLASGVPSRFSGSGSGTDYTFTISSLQPEDIATYYCQQWSSNPFTFGQGTKLQITRDKTHTCPPCPAPEAAGGPSVFLFPPKPKDTLMISRTPEVTCVVVDVSHEDPEVKFNWYVDGVEVHNAKTKPREEQYNSTYRVVSVLTVLHQDWLNGKEYKCKVSNKALPAPIEKTISKAKGQPREPQVYTLPPSREEMTKNQVSLTCLVKGFYPSDIAVEWESNGQPENNYKTTPPVLDSDGSFFLYSKLTVDKSRWQQGNVFSCSVMHEALHNHYTQKSLSLSPGK

SEQ ID NO: 173 - protein, 695 aa, Artificial Sequence
QVQLVQSGAEVKKPGSSVKVSCKASGYTFTRNFIHWIRQAPGQGLEWIGWIFPGDADTEYNQKFSGRATITADKSTSTAYMELSSLRSEDTAVYYCARGNYNYEYFDYWGQGTMVTVSSASTKGPSVFPLAPSSKSTSGGTAALGCLVKDYFPEPVTVSWNSGALTSGVHTFPAVLQSSGLYSLSSVVTVPSSSLGTQTYICNVNHKPSNTKVDKRVEPKSCGGGGSQVQLVQSGGGVVQPGRSLRLSCKASGYTFTRYTMHWVRQAPGKGLEWIGYINPSRGYTNYNQKVKDRFTISRDNSKNTAFLQMDSLRPEDTGVYFCARYYNDHYSLDYWGQGTPVTVSSGGGGSGGGGSGGGGSDIQMTQSPSSLSASVGDRVTITCSASSSVSYMNWYQQTPGKAPKRWIYDTSKLASGVPSRFSGSGSGTDYTFTISSLQPEDIATYYCQQWSSNPFTFGQGTKLQITRDKTHTCPPCPAPEAAGGPSVFLFPPKPKDTLMISRTPEVTCVVVDVSHEDPEVKFNWYVDGVEVHNAKTKPREEQYNSTYRVVSVLTVLHQDWLNGKEYKCKVSNKALPAPIEKTISKAKGQPREPQVYTLPPSREEMTKNQVSLTCLVKGFYPSDIAVEWESNGQPENNYKTTPPVLDSDGSFFLYSKLTVDKSRWQQGNVFSCSVMHEALHNHYTQKSLSLSPGK

SEQ ID NO: 174 - protein, 695 aa, Artificial Sequence
QVQLVQSGAEVKKPGSSVKVSCKASGYTFTRNFIHWIRQAPGQGLEWIGWIFPGDADTEYNQKFSGRATITADKSTSTAYMELSSLRSEDTAVYYCARGNYNYEYFDYWGQGTMVTVSSASTKGPSVFPLAPSSKSTSGGTAALGCLVKDYFPEPVTVSWNSGALTSGVHTFPAVLQSSGLYSLSSVVTVPSSSLGTQTYICNVNHKPSNTKVDKRVEPKSCGGGGSQVQLVQSGGGVVQPGRSLRLSCKASGYTFTRYTMHWVRQAPGKGLEWIGYINPSRGYTNYNQKVKDRFTISRDNSKNTAFLQMDSLRPEDTGVYFCARYYDDHFSLDYWGQGTPVTVSSGGGGSGGGGSGGGGSDIQMTQSPSSLSASVGDRVTITCSASSSVSYMNWYQQTPGKAPKRWIYDTSKLASGVPSRFSGSGSGTDYTFTISSLQPEDIATYYCQQWSSNPFTFGQGTKLQITRDKTHTCPPCPAPEAAGGPSVFLFPPKPKDTLMISRTPEVTCVVVDVSHEDPEVKFNWYVDGVEVHNAKTKPREEQYNSTYRVVSVLTVLHQDWLNGKEYKCKVSNKALPAPIEKTISKAKGQPREPQVYTLPPSREEMTKNQVSLTCLVKGFYPSDIAVEWESNGQPENNYKTTPPVLDSDGSFFLYSKLTVDKSRWQQGNVFSCSVMHEALHNHYTQKSLSLSPGK

SEQ ID NO: 175 - protein, 695 aa, Artificial Sequence
QVQLVQSGAEVKKPGSSVKVSCKASGYTFTRNFIHWIRQAPGQGLEWIGWIFPGDADTEYNQKFSGRATITADKSTSTAYMELSSLRSEDTAVYYCARGNYNYEYFDYWGQGTMVTVSSASTKGPSVFPLAPSSKSTSGGTAALGCLVKDYFPEPVTVSWNSGALTSGVHTFPAVLQSSGLYSLSSVVTVPSSSLGTQTYICNVNHKPSNTKVDKRVEPKSCGGGGSQVQLVQSGGGVVQPGRSLRLSCKASGYTFTRYTMHWVRQAPGKGLEWIGYINPSMGATNYNQKVKDRFTISRDNSKNTAFLQMDSLRPEDTGVYFCARYYDDHYSLDYWGQGTPVTVSSGGGGSGGGGSGGGGSDIQMTQSPSSLSASVGDRVTITCSASSSVSYMNWYQQTPGKAPKRWIYDTSKLASGVPSRFSGSGSGTDYTFTISSLQPEDIATYYCQQWSSNPFTFGQGTKLQITRDKTHTCPPCPAPEAAGGPSVFLFPPKPKDTLMISRTPEVTCVVVDVSHEDPEVKFNWYVDGVEVHNAKTKPREEQYNSTYRVVSVLTVLHQDWLNGKEYKCKVSNKALPAPIEKTISKAKGQPREPQVYTLPPSREEMTKNQVSLTCLVKGFYPSDIAVEWESNGQPENNYKTTPPVLDSDGSFFLYSKLTVDKSRWQQGNVFSCSVMHEALHNHYTQKSLSLSPGK

SEQ ID NO: 176 - protein, 695 aa, Artificial Sequence
QVQLVQSGAEVKKPGSSVKVSCKASGYTFTRNFIHWIRQAPGQGLEWIGWIFPGDADTEYNQKFSGRVTITADKSTSTAYMELSSLRSEDTAVYYCARGNYNYEYFDYWGQGTMVTVSSASTKGPSVFPLAPSSKSTSGGTAALGCLVKDYFPEPVTVSWNSGALTSGVHTFPAVLQSSGLYSLSSVVTVPSSSLGTQTYICNVNHKPSNTKVDKRVEPKSCGGGGSQVQLVQSGGGVVQPGRSLRLSCKASGYTFTRYTMHWVRQAPGKGLEWIGYINPSRGYTNYNQKVKDRFTISRDNSKNTAFLQMDSLRPEDTGVYFCARYYDDHYSLDYWGQGTPVTVSSGGGGSGGGGSGGGGSDIQMTQSPSSLSASVGDRVTITCSASSSVSYMNWYQQTPGKAPKRWIYDTSKLASGVPSRFSGSGSGTDYTFTISSLQPEDIATYYCQQWSSNPFTFGQGTKLQITRDKTHTCPPCPAPEAAGGPSVFLFPPKPKDTLMISRTPEVTCVVVDVSHEDPEVKFNWYVDGVEVHNAKTKPREEQYNSTYRVVSVLTVLHQDWLNGKEYKCKVSNKALPAPIEKTISKAKGQPREPQVYTLPPSREEMTKNQVSLTCLVKGFYPSDIAVEWESNGQPENNYKTTPPVLDSDGSFFLYSKLTVDKSRWQQGNVFSCSVMHEALHNHYTQKSLSLSPGK

SEQ ID NO: 177 - protein, 695 aa, Artificial Sequence
QVQLVQSGAEVKKPGSSVKVSCKASGYTFTRNFIHWIRQAPGQGLEWIGWIFPGDADTEYNQKFSGRVTITADKSTSTAYMELSSLRSEDTAVYYCARGNYNYEYFDYWGQGTMVTVSSASTKGPSVFPLAPSSKSTSGGTAALGCLVKDYFPEPVTVSWNSGALTSGVHTFPAVLQSSGLYSLSSVVTVPSSSLGTQTYICNVNHKPSNTKVDKRVEPKSCGGGGSQVQLVQSGGGVVQPGRSLRLSCKASGYTFTRYTMHWVRQAPGKGLEWIGYINPSRGYTNYNQKVKDRFTISRDNSKNTAFLQMDSLRPEDTGVYFCARYYDDHYSLDYWGQGTPVTVSSGGGGSGGGGSGGGGSDIQMTQSPSSLSASVGDRVTITCSASSSVAYMNWYQQTPGKAPKRWIYDTSKLASGVPSRFSGSGSGTDYTFTISSLQPEDIATYYCQQWSSNPFTFGQGTKLQITRDKTHTCPPCPAPEAAGGPSVFLFPPKPKDTLMISRTPEVTCVVVDVSHEDPEVKFNWYVDGVEVHNAKTKPREEQYNSTYRVVSVLTVLHQDWLNGKEYKCKVSNKALPAPIEKTISKAKGQPREPQVYTLPPSREEMTKNQVSLTCLVKGFYPSDIAVEWESNGQPENNYKTTPPVLDSDGSFFLYSKLTVDKSRWQQGNVFSCSVMHEALHNHYTQKSLSLSPGK

SEQ ID NO: 178 - protein, 695 aa, Artificial Sequence
QVQLVQSGAEVKKPGSSVKVSCKASGYTFTRNFIHWIRQAPGQGLEWIGWIFPGDADTEYNQKFSGRVTITADKSTSTAYMELSSLRSEDTAVYYCARGNYNYEYFDYWGQGTMVTVSSASTKGPSVFPLAPSSKSTSGGTAALGCLVKDYFPEPVTVSWNSGALTSGVHTFPAVLQSSGLYSLSSVVTVPSSSLGTQTYICNVNHKPSNTKVDKRVEPKSCGGGGSQVQLVQSGGGVVQPGRSLRLSCKASGYTFTRYTMHWVRQAPGKGLEWIGYINPSRGYTNYNQKVKDRFTISRDNSKNTAFLQMDSLRPEDTGVYFCARYYDDHYSLDYWGQGTPVTVSSGGGGSGGGGSGGGGSDIQMTQSPSSLSASVGDRVTITCSASSSVSYMNWYQQTPGKAPKRWIYNTSKLASGVPSRFSGSGSGTDYTFTISSLQPEDIATYYCQQWSSNPFTFGQGTKLQITRDKTHTCPPCPAPEAAGGPSVFLFPPKPKDTLMISRTPEVTCVVVDVSHEDPEVKFNWYVDGVEVHNAKTKPREEQYNSTYRVVSVLTVLHQDWLNGKEYKCKVSNKALPAPIEKTISKAKGQPREPQVYTLPPSREEMTKNQVSLTCLVKGFYPSDIAVEWESNGQPENNYKTTPPVLDSDGSFFLYSKLTVDKSRWQQGNVFSCSVMHEALHNHYTQKSLSLSPGK

SEQ ID NO: 179 - protein, 695 aa, Artificial Sequence
QVQLVQSGAEVKKPGSSVKVSCKASGYTFTRNFIHWIRQAPGQGLEWIGWIFPGDADTEYNQKFSGRVTITADKSTSTAYMELSSLRSEDTAVYYCARGNYNYEYFDYWGQGTMVTVSSASTKGPSVFPLAPSSKSTSGGTAALGCLVKDYFPEPVTVSWNSGALTSGVHTFPAVLQSSGLYSLSSVVTVPSSSLGTQTYICNVNHKPSNTKVDKRVEPKSCGGGGSQVQLVQSGGGVVQPGRSLRLSCKASGYTFTRYTMHWVRQAPGKGLEWIGYINPSRGYTNYNQKVKDRFTISRDNSKNTAFLQMDSLRPEDTGVYFCARYYNDHYSLDYWGQGTPVTVSSGGGGSGGGGSGGGGSDIQMTQSPSSLSASVGDRVTITCSASSSVSYMNWYQQTPGKAPKRWIYDTSKLASGVPSRFSGSGSGTDYTFTISSLQPEDIATYYCQQWSSNPFTFGQGTKLQITRDKTHTCPPCPAPEAAGGPSVFLFPPKPKDTLMISRTPEVTCVVVDVSHEDPEVKFNWYVDGVEVHNAKTKPREEQYNSTYRVVSVLTVLHQDWLNGKEYKCKVSNKALPAPIEKTISKAKGQPREPQVYTLPPSREEMTKNQVSLTCLVKGFYPSDIAVEWESNGQPENNYKTTPPVLDSDGSFFLYSKLTVDKSRWQQGNVFSCSVMHEALHNHYTQKSLSLSPGK

SEQ ID NO: 180 - protein, 695 aa, Artificial Sequence
QVQLVQSGAEVKKPGSSVKVSCKASGYTFTRNFIHWIRQAPGQGLEWIGWIFPGDADTEYNQKFSGRVTITADKSTSTAYMELSSLRSEDTAVYYCARGNYNYEYFDYWGQGTMVTVSSASTKGPSVFPLAPSSKSTSGGTAALGCLVKDYFPEPVTVSWNSGALTSGVHTFPAVLQSSGLYSLSSVVTVPSSSLGTQTYICNVNHKPSNTKVDKRVEPKSCGGGGSQVQLVQSGGGVVQPGRSLRLSCKASGYTFTRYTMHWVRQAPGKGLEWIGYINPSRGYTNYNQKVKDRFTISRDNSKNTAFLQMDSLRPEDTGVYFCARYYDDHFSLDYWGQGTPVTVSSGGGGSGGGGSGGGGSDIQMTQSPSSLSASVGDRVTITCSASSSVSYMNWYQQTPGKAPKRWIYDTSKLASGVPSRFSGSGSGTDYTFTISSLQPEDIATYYCQQWSSNPFTFGQGTKLQITRDKTHTCPPCPAPEAAGGPSVFLFPPKPKDTLMISRTPEVTCVVVDVSHEDPEVKFNWYVDGVEVHNAKTKPREEQYNSTYRVVSVLTVLHQDWLNGKEYKCKVSNKALPAPIEKTISKAKGQPREPQVYTLPPSREEMTKNQVSLTCLVKGFYPSDIAVEWESNGQPENNYKTTPPVLDSDGSFFLYSKLTVDKSRWQQGNVFSCSVMHEALHNHYTQKSLSLSPGK

SEQ ID NO: 181 - protein, 695 aa, Artificial Sequence
QVQLVQSGAEVKKPGSSVKVSCKASGYTFTRNFIHWIRQAPGQGLEWIGWIFPGDADTEYNQKFSGRVTITADKSTSTAYMELSSLRSEDTAVYYCARGNYNYEYFDYWGQGTMVTVSSASTKGPSVFPLAPSSKSTSGGTAALGCLVKDYFPEPVTVSWNSGALTSGVHTFPAVLQSSGLYSLSSVVTVPSSSLGTQTYICNVNHKPSNTKVDKRVEPKSCGGGGSQVQLVQSGGGVVQPGRSLRLSCKASGYTFTRYTMHWVRQAPGKGLEWIGYINPSMGATNYNQKVKDRFTISRDNSKNTAFLQMDSLRPEDTGVYFCARYYDDHYSLDYWGQGTPVTVSSGGGGSGGGGSGGGGSDIQMTQSPSSLSASVGDRVTITCSASSSVSYMNWYQQTPGKAPKRWIYDTSKLASGVPSRFSGSGSGTDYTFTISSLQPEDIATYYCQQWSSNPFTFGQGTKLQITRDKTHTCPPCPAPEAAGGPSVFLFPPKPKDTLMISRTPEVTCVVVDVSHEDPEVKFNWYVDGVEVHNAKTKPREEQYNSTYRVVSVLTVLHQDWLNGKEYKCKVSNKALPAPIEKTISKAKGQPREPQVYTLPPSREEMTKNQVSLTCLVKGFYPSDIAVEWESNGQPENNYKTTPPVLDSDGSFFLYSKLTVDKSRWQQGNVFSCSVMHEALHNHYTQKSLSLSPGK

SEQ ID NO: 182 - protein, 695 aa, Artificial Sequence
QVQLVQSGAEVKKPGSSVKVSCKASGYTFTRNFIHWIRQAPGQGLEWIGWIFPGDGDTEYNQKFNGRATITADKSTSTAYMELSSLRSEDTAVYYCARGNYNYEYFDYWGQGTMVTVSSASTKGPSVFPLAPSSKSTSGGTAALGCLVKDYFPEPVTVSWNSGALTSGVHTFPAVLQSSGLYSLSSVVTVPSSSLGTQTYICNVNHKPSNTKVDKRVEPKSCGGGGSQVQLVQSGGGVVQPGRSLRLSCKASGYTFTRYTMHWVRQAPGKGLEWIGYINPSRGYTNYNQKVKDRFTISRDNSKNTAFLQMDSLRPEDTGVYFCARYYDDHYSLDYWGQGTPVTVSSGGGGSGGGGSGGGGSDIQMTQSPSSLSASVGDRVTITCSASSSVSYMNWYQQTPGKAPKRWIYDTSKLASGVPSRFSGSGSGTDYTFTISSLQPEDIATYYCQQWSSNPFTFGQGTKLQITRDKTHTCPPCPAPEAAGGPSVFLFPPKPKDTLMISRTPEVTCVVVDVSHEDPEVKFNWYVDGVEVHNAKTKPREEQYNSTYRVVSVLTVLHQDWLNGKEYKCKVSNKALPAPIEKTISKAKGQPREPQVYTLPPSREEMTKNQVSLTCLVKGFYPSDIAVEWESNGQPENNYKTTPPVLDSDGSFFLYSKLTVDKSRWQQGNVFSCSVMHEALHNHYTQKSLSLSPGK

SEQ ID NO: 183 - protein, 695 aa, Artificial Sequence
QVQLVQSGAEVKKPGSSVKVSCKASGYTFTRNFIHWIRQAPGQGLEWIGWIFPGDGDTEYNQKFNGRATITADKSTSTAYMELSSLRSEDTAVYYCARGNYNYEYFDYWGQGTMVTVSSASTKGPSVFPLAPSSKSTSGGTAALGCLVKDYFPEPVTVSWNSGALTSGVHTFPAVLQSSGLYSLSSVVTVPSSSLGTQTYICNVNHKPSNTKVDKRVEPKSCGGGGSQVQLVQSGGGVVQPGRSLRLSCKASGYTFTRYTMHWVRQAPGKGLEWIGYINPSRGYTNYNQKVKDRFTISRDNSKNTAFLQMDSLRPEDTGVYFCARYYDDHYSLDYWGQGTPVTVSSGGGGSGGGGSGGGGSDIQMTQSPSSLSASVGDRVTITCSASSSVAYMNWYQQTPGKAPKRWIYDTSKLASGVPSRFSGSGSGTDYTFTISSLQPEDIATYYCQQWSSNPFTFGQGTKLQITRDKTHTCPPCPAPEAAGGPSVFLFPPKPKDTLMISRTPEVTCVVVDVSHEDPEVKFNWYVDGVEVHNAKTKPREEQYNSTYRVVSVLTVLHQDWLNGKEYKCKVSNKALPAPIEKTISKAKGQPREPQVYTLPPSREEMTKNQVSLTCLVKGFYPSDIAVEWESNGQPENNYKTTPPVLDSDGSFFLYSKLTVDKSRWQQGNVFSCSVMHEALHNHYTQKSLSLSPGK

SEQ ID NO: 184 - protein, 695 aa, Artificial Sequence
QVQLVQSGAEVKKPGSSVKVSCKASGYTFTRNFIHWIRQAPGQGLEWIGWIFPGDGDTEYNQKFNGRATITADKSTSTAYMELSSLRSEDTAVYYCARGNYNYEYFDYWGQGTMVTVSSASTKGPSVFPLAPSSKSTSGGTAALGCLVKDYFPEPVTVSWNSGALTSGVHTFPAVLQSSGLYSLSSVVTVPSSSLGTQTYICNVNHKPSNTKVDKRVEPKSCGGGGSQVQLVQSGGGVVQPGRSLRLSCKASGYTFTRYTMHWVRQAPGKGLEWIGYINPSRGYTNYNQKVKDRFTISRDNSKNTAFLQMDSLRPEDTGVYFCARYYDDHYSLDYWGQGTPVTVSSGGGGSGGGGSGGGGSDIQMTQSPSSLSASVGDRVTITCSASSSVSYMNWYQQTPGKAPKRWIYNTSKLASGVPSRFSGSGSGTDYTFTISSLQPEDIATYYCQQWSSNPFTFGQGTKLQITRDKTHTCPPCPAPEAAGGPSVFLFPPKPKDTLMISRTPEVTCVVVDVSHEDPEVKFNWYVDGVEVHNAKTKPREEQYNSTYRVVSVLTVLHQDWLNGKEYKCKVSNKALPAPIEKTISKAKGQPREPQVYTLPPSREEMTKNQVSLTCLVKGFYPSDIAVEWESNGQPENNYKTTPPVLDSDGSFFLYSKLTVDKSRWQQGNVFSCSVMHEALHNHYTQKSLSLSPGK

SEQ ID NO: 185 - protein, 695 aa, Artificial Sequence
QVQLVQSGAEVKKPGSSVKVSCKASGYTFTRNFIHWIRQAPGQGLEWIGWIFPGDGDTEYNQKFNGRATITADKSTSTAYMELSSLRSEDTAVYYCARGNYNYEYFDYWGQGTMVTVSSASTKGPSVFPLAPSSKSTSGGTAALGCLVKDYFPEPVTVSWNSGALTSGVHTFPAVLQSSGLYSLSSVVTVPSSSLGTQTYICNVNHKPSNTKVDKRVEPKSCGGGGSQVQLVQSGGGVVQPGRSLRLSCKASGYTFTRYTMHWVRQAPGKGLEWIGYINPSRGYTNYNQKVKDRFTISRDNSKNTAFLQMDSLRPEDTGVYFCARYYNDHYSLDYWGQGTPVTVSSGGGGSGGGGSGGGGSDIQMTQSPSSLSASVGDRVTITCSASSSVSYMNWYQQTPGKAPKRWIYDTSKLASGVPSRFSGSGSGTDYTFTISSLQPEDIATYYCQQWSSNPFTFGQGTKLQITRDKTHTCPPCPAPEAAGGPSVFLFPPKPKDTLMISRTPEVTCVVVDVSHEDPEVKFNWYVDGVEVHNAKTKPREEQYNSTYRVVSVLTVLHQDWLNGKEYKCKVSNKALPAPIEKTISKAKGQPREPQVYTLPPSREEMTKNQVSLTCLVKGFYPSDIAVEWESNGQPENNYKTTPPVLDSDGSFFLYSKLTVDKSRWQQGNVFSCSVMHEALHNHYTQKSLSLSPGK

SEQ ID NO: 186 - protein, 695 aa, Artificial Sequence
QVQLVQSGAEVKKPGSSVKVSCKASGYTFTRNFIHWIRQAPGQGLEWIGWIFPGDGDTEYNQKFNGRATITADKSTSTAYMELSSLRSEDTAVYYCARGNYNYEYFDYWGQGTMVTVSSASTKGPSVFPLAPSSKSTSGGTAALGCLVKDYFPEPVTVSWNSGALTSGVHTFPAVLQSSGLYSLSSVVTVPSSSLGTQTYICNVNHKPSNTKVDKRVEPKSCGGGGSQVQLVQSGGGVVQPGRSLRLSCKASGYTFTRYTMHWVRQAPGKGLEWIGYINPSRGYTNYNQKVKDRFTISRDNSKNTAFLQMDSLRPEDTGVYFCARYYDDHFSLDYWGQGTPVTVSSGGGGSGGGGSGGGGSDIQMTQSPSSLSASVGDRVTITCSASSSVSYMNWYQQTPGKAPKRWIYDTSKLASGVPSRFSGSGSGTDYTFTISSLQPEDIATYYCQQWSSNPFTFGQGTKLQITRDKTHTCPPCPAPEAAGGPSVFLFPPKPKDTLMISRTPEVTCVVVDVSHEDPEVKFNWYVDGVEVHNAKTKPREEQYNSTYRVVSVLTVLHQDWLNGKEYKCKVSNKALPAPIEKTISKAKGQPREPQVYTLPPSREEMTKNQVSLTCLVKGFYPSDIAVEWESNGQPENNYKTTPPVLDSDGSFFLYSKLTVDKSRWQQGNVFSCSVMHEALHNHYTQKSLSLSPGK

SEQ ID NO: 187 - protein, 695 aa, Artificial Sequence
QVQLVQSGAEVKKPGSSVKVSCKASGYTFTRNFIHWIRQAPGQGLEWIGWIFPGDGDTEYNQKFNGRATITADKSTSTAYMELSSLRSEDTAVYYCARGNYNYEYFDYWGQGTMVTVSSASTKGPSVFPLAPSSKSTSGGTAALGCLVKDYFPEPVTVSWNSGALTSGVHTFPAVLQSSGLYSLSSVVTVPSSSLGTQTYICNVNHKPSNTKVDKRVEPKSCGGGGSQVQLVQSGGGVVQPGRSLRLSCKASGYTFTRYTMHWVRQAPGKGLEWIGYINPSMGATNYNQKVKDRFTISRDNSKNTAFLQMDSLRPEDTGVYFCARYYDDHYSLDYWGQGTPVTVSSGGGGSGGGGSGGGGSDIQMTQSPSSLSASVGDRVTITCSASSSVSYMNWYQQTPGKAPKRWIYDTSKLASGVPSRFSGSGSGTDYTFTISSLQPEDIATYYCQQWSSNPFTFGQGTKLQITRDKTHTCPPCPAPEAAGGPSVFLFPPKPKDTLMISRTPEVTCVVVDVSHEDPEVKFNWYVDGVEVHNAKTKPREEQYNSTYRVVSVLTVLHQDWLNGKEYKCKVSNKALPAPIEKTISKAKGQPREPQVYTLPPSREEMTKNQVSLTCLVKGFYPSDIAVEWESNGQPENNYKTTPPVLDSDGSFFLYSKLTVDKSRWQQGNVFSCSVMHEALHNHYTQKSLSLSPGK

SEQ ID NO: 188 - protein, 714 aa, Artificial Sequence
QVQLVQSGGGVVQPGRSLRLSCKASGYTFTRYTMHWVRQAPGKGLEWIGYINPSRGYTNYNQKVKDRFTISRDNSKNTAFLQMDSLRPEDTGVYFCARYYDDHYSLDYWGQGTPVTVSSGGGGSGGGGSGGGGSDIQMTQSPSSLSASVGDRVTITCSASSSVSYMNWYQQTPGKAPKRWIYDTSKLASGVPSRFSGSGSGTDYTFTISSLQPEDIATYYCQQWSSNPFTFGQGTKLQITRGGGGSDIQMTQSPSSLSASVGDRVTITCLASEDIYSYLAWYQQKPGKAPKLLIFAANRLQDGVPSRFSGSGSGTDFTLTISSLQPEDFATYYCLQGSKFPYTFGPGTKVDIKGGGGSGGGGSGGGGSQVQLVQSGAEVKKPGSSVKVSCKASGYTFTRNFIHWIRQAPGQGLEWIGWIFPGDADTEYNQKFSGRATITADKSTSTAYMELSSLRSEDTAVYYCARGNYNYEYFDYWGQGTMVTVSSDKTHTCPPCPAPEAAGGPSVFLFPPKPKDTLMISRTPEVTCVVVDVSHEDPEVKFNWYVDGVEVHNAKTKPREEQYNSTYRVVSVLTVLHQDWLNGKEYKCKVSNKALPAPIEKTISKAKGQPREPQVYTLPPSREEMTKNQVSLTCLVKGFYPSDIAVEWESNGQPENNYKTTPPVLDSDGSFFLYSKLTVDKSRWQQGNVFSCSVMHEALHNHYTQKSLSLSPGK

SEQ ID NO: 189 - protein, 449 aa, Artificial Sequence
QVQLVQSGAEVKKPGSSVKVSCKASGYTFTRNFIHWIRQAPGQGLEWIGWIFPGDADTEYNQKFSGRATITADKSTSTAYMELSSLRSEDTAVYYCARGNYNYEYFDYWGQGTMVTVSSASTKGPSVFPLAPSSKSTSGGTAALGCLVKDYFPEPVTVSWNSGALTSGVHTFPAVLQSSGLYSLSSVVTVPSSSLGTQTYICNVNHKPSNTKVDKRVEPKSCDKTHTCPPCPAPEAAGGPSVFLFPPKPKDTLMISRTPEVTCVVVDVSHEDPEVKFNWYVDGVEVHNAKTKPREEQYNSTYRVVSVLTVLHQDWLNGKEYKCKVSNKALPAPIEKTISKAKGQPREPQVYTLPPSREEMTKNQVSLTCLVKGFYPSDIAVEWESNGQPENNYKTTPPVLDSDGSFFLYSKLTVDKSRWQQGNVFSCSVMHEALHNHYTQKSLSLSPGK

SEQ ID NO: 190 - protein, 449 aa, Artificial Sequence
QVQLVQSGAEVKKPGSSVKVSCKASGYTFTRNFIHWIRQAPGQGLEWIGWIFPGDADTEYNQKFSGRVTITADKSTSTAYMELSSLRSEDTAVYYCARGNYNYEYFDYWGQGTMVTVSSASTKGPSVFPLAPSSKSTSGGTAALGCLVKDYFPEPVTVSWNSGALTSGVHTFPAVLQSSGLYSLSSVVTVPSSSLGTQTYICNVNHKPSNTKVDKRVEPKSCDKTHTCPPCPAPEAAGGPSVFLFPPKPKDTLMISRTPEVTCVVVDVSHEDPEVKFNWYVDGVEVHNAKTKPREEQYNSTYRVVSVLTVLHQDWLNGKEYKCKVSNKALPAPIEKTISKAKGQPREPQVYTLPPSREEMTKNQVSLTCLVKGFYPSDIAVEWESNGQPENNYKTTPPVLDSDGSFFLYSKLTVDKSRWQQGNVFSCSVMHEALHNHYTQKSLSLSPGK

SEQ ID NO: 191 - protein, 695 aa, Artificial Sequence
QVQLVQSGAEVKKPGSSVKVSCKASGYTFTRNFIHWIRQAPGQGLEWIGWIFPGDADTEYNQKFSGRATITADKSTSTAYMELSSLRSEDTAVYYCARGNYNYEYFDYWGQGTMVTVSSASTKGPSVFPLAPSSKSTSGGTAALGCLVKDYFPEPVTVSWNSGALTSGVHTFPAVLQSSGLYSLSSVVTVPSSSLGTQTYICNVNHKPSNTKVDKRVEPKSCGGGGSQVQLVQSGGGVVQPGRSLRLSCKASGYTFTRYTMHWVRQAPGKGLEWIGYINPSRGYTNYNQKVKDRFTISRDNSKNTAFLQMDSLRPEDTGVYFCARYYDDHYSLDYWGQGTPVTVSSGGGGSGGGGSGGGGSDIQMTQSPSSLSASVGDRVTITCSASSSVSYMNWYQQTPGKAPKRWIYDTSKLASGVPSRFSGSGSGTDYTFTISSLQPEDIATYYCQQWSSNPFTFGQGTKLQITRDKTHTCPPCPAPEAAGGPSVFLFPPKPKDTLMISRTPEVTCVVVDVSHEDPEVKFNWYVDGVEVHNAKTKPREEQYNSTYRVVSVLTVLHQDWLNGKEYKCKVSNKALPAPIEKTISKAKGQPREPQVYTLPPCREEMTKNQVSLWCLVKGFYPSDIAVEWESNGQPENNYKTTPPVLDSDGSFFLYSKLTVDKSRWQQGNVFSCSVMHEALHNHYTQKSLSLSPGK

SEQ ID NO: 192 - protein, 705 aa, Artificial Sequence
QVQLVQSGAEVKKPGSSVKVSCKASGYTFTRNFIHWIRQAPGQGLEWIGWIFPGDADTEYNQKFSGRATITADKSTSTAYMELSSLRSEDTAVYYCARGNYNYEYFDYWGQGTMVTVSSASTKGPSVFPLAPSSKSTSGGTAALGCLVKDYFPEPVTVSWNSGALTSGVHTFPAVLQSSGLYSLSSVVTVPSSSLGTQTYICNVNHKPSNTKVDKRVEPKSCGGGGSQVQLVQSGGGVVQPGRSLRLSCKASGYTFTRYTMHWVRQAPGKGLEWIGYINPSRGYTNYNQKVKDRFTISRDNSKNTAFLQMDSLRPEDTGVYFCARYYDDHYSLDYWGQGTPVTVSSGGGGSGGGGSGGGGSDIQMTQSPSSLSASVGDRVTITCSASSSVSYMNWYQQTPGKAPKRWIYDTSKLASGVPSRFSGSGSGTDYTFTISSLQPEDIATYYCQQWSSNPFTFGQGTKLQITRGGGGSGGGGSDKTHTCPPCPAPEAAGGPSVFLFPPKPKDTLMISRTPEVTCVVVDVSHEDPEVKFNWYVDGVEVHNAKTKPREEQYNSTYRVVSVLTVLHQDWLNGKEYKCKVSNKALPAPIEKTISKAKGQPREPQVYTLPPCREEMTKNQVSLWCLVKGFYPSDIAVEWESNGQPENNYKTTPPVLDSDGSFFLYSKLTVDKSRWQQGNVFSCSVMHEALHNHYTQKSLSLSPGK

SEQ ID NO: 193 - protein, 700 aa, Artificial Sequence
QVQLVQSGAEVKKPGSSVKVSCKASGYTFTRNFIHWIRQAPGQGLEWIGWIFPGDADTEYNQKFSGRATITADKSTSTAYMELSSLRSEDTAVYYCARGNYNYEYFDYWGQGTMVTVSSASTKGPSVFPLAPSSKSTSGGTAALGCLVKDYFPEPVTVSWNSGALTSGVHTFPAVLQSSGLYSLSSVVTVPSSSLGTQTYICNVNHKPSNTKVDKRVEPKSCGGGGSQVQLVQSGGGVVQPGRSLRLSCKASGYTFTRYTMHWVRQAPGKGLEWIGYINPSRGYTNYNQKVKDRFTISRDNSKNTAFLQMDSLRPEDTGVYFCARYYDDHYSLDYWGQGTPVTVSSGGGGSGGGGSGGGGSDIQMTQSPSSLSASVGDRVTITCSASSSVSYMNWYQQTPGKAPKRWIYDTSKLASGVPSRFSGSGSGTDYTFTISSLQPEDIATYYCQQWSSNPFTFGQGTKLQITREPKSVDKTHTCPPCPAPEAAGGPSVFLFPPKPKDTLMISRTPEVTCVVVDVSHEDPEVKFNWYVDGVEVHNAKTKPREEQYNSTYRVVSVLTVLHQDWLNGKEYKCKVSNKALPAPIEKTISKAKGQPREPQVYTLPPCREEMTKNQVSLWCLVKGFYPSDIAVEWESNGQPENNYKTTPPVLDSDGSFFLYSKLTVDKSRWQQGNVFSCSVMHEALHNHYTQKSLSLSPGK

SEQ ID NO: 194 - protein, 474 aa, Artificial Sequence
QVQLVQSGAEVKKPGSSVKVSCKASGYTFTRNFIHWIRQAPGQGLEWIGWIFPGDADTEYNQKFSGRATITADKSTSTAYMELSSLRSEDTAVYYCARGNYNYEYFDYWGQGTMVTVSSASTKGPSVFPLAPSSKSTSGGTAALGCLVKDYFPEPVTVSWNSGALTSGVHTFPAVLQSSGLYSLSSVVTVPSSSLGTQTYICNVNHKPSNTKVDKRVEPKSCGGGGSQVQLVQSGGGVVQPGRSLRLSCKASGYTFTRYTMHWVRQAPGKGLEWIGYINPSRGYTNYNQKVKDRFTISRDNSKNTAFLQMDSLRPEDTGVYFCARYYDDHYSLDYWGQGTPVTVSSGGGGSGGGGSGGGGSDIQMTQSPSSLSASVGDRVTITCSASSSVSYMNWYQQTPGKAPKRWIYDTSKLASGVPSRFSGSGSGTDYTFTISSLQPEDIATYYCQQWSSNPFTFGQGTKLQITRHHHHHH

SEQ ID NO: 195 - protein, 449 aa, Artificial Sequence
QVQLVQSGAEVKKPGSSVKVSCKASGYTFTRNFIHWIRQAPGQGLEWIGWIFPGDADTEYNQKFSGRATITADKSTSTAYMELSSLRSEDTAVYYCARGNYNYEYFDYWGQGTMVTVSSASTKGPSVFPLAPSSKSTSGGTAALGCLVKDYFPEPVTVSWNSGALTSGVHTFPAVLQSSGLYSLSSVVTVPSSSLGTQTYICNVNHKPSNTKVDKRVEPKSCDKTHTCPPCPAPEAAGGPSVFLFPPKPKDTLMISRTPEVTCVVVDVSHEDPEVKFNWYVDGVEVHNAKTKPREEQYNSTYRVVSVLTVLHQDWLNGKEYKCKVSNKALPAPIEKTISKAKGQPREPQVYTLPPCREEMTKNQVSLWCLVKGFYPSDIAVEWESNGQPENNYKTTPPVLDSDGSFFLYSKLTVDKSRWQQGNVFSCSVMHEALHNHYTQKSLSLSPGK

SEQ ID NO: 196 - protein, 483 aa, Artificial Sequence
DIQMTQSPSSLSASVGDRVTITCLASEDIYSYLAWYQQKPGKAPKLLIFAANRLQSGVPSRFSGSGSGTDFTLTISSLQPEDFATYYCLQGSKFPYTFGPGTKVDIKGGGGSGGGGSGGGGSQVQLVQSGAEVKKPGSSVKVSCKASGYTFTRNFIHWIRQAPGQGLEWIGWIFPGDADTEYNQKFSGRATITADKSTSTAYMELSSLRSEDTAVYYCARGNYNYEYFDYWGQGTMVTVSSGGGGSGGGGSGGGGSDKTHTCPPCPAPEAAGGPSVFLFPPKPKDTLMISRTPEVTCVVVDVSHEDPEVKFNWYVDGVEVHNAKTKPREEQYNSTYRVVSVLTVLHQDWLNGKEYKCKVSNKALPAPIEKTISKAKGQPREPQVCTLPPSREEMTKNQVSLSCAVKGFYPSDIAVEWESNGQPENNYKTTPPVLDSDGSFFLVSKLTVDKSRWQQGNVFSCSVMHEALHNHYTQKSLSLSPGK

SEQ ID NO: 197 - protein, 214 aa, Artificial Sequence
DIQMTQSPSSLSASVGDRVTITCLASEDIYSYLAWYQQKPGKAPKLLIFAANRLQDGVPSRFSGSGSGTDFTLTISSLQPEDFATYYCLQGSKFPYTFGPGTKVDIKRTVAAPSVFIFPPSDEQLKSGTASVVCLLNNFYPREAKVQWKVDNALQSGNSQESVTEQDSKDSTYSLSSTLTLSKADYEKHKVYACEVTHQGLSSPVTKSFNRGEC

SEQ ID NO: 198 - protein, 214 aa, Artificial Sequence
DIQMTQSPSSLSASVGDRVTITCLASEDIYSYLAWYQQKPGKAPKLLIFAANRLQSGVPSRFSGSGSGTDFTLTISSLQPEDFATYYCLQGSKFPYTFGPGTKVDIKRTVAAPSVFIFPPSDEQLKSGTASVVCLLNNFYPREAKVQWKVDNALQSGNSQESVTEQDSKDSTYSLSSTLTLSKADYEKHKVYACEVTHQGLSSPVTKSFNRGEC

SEQ ID NO: 199 - protein, 465 aa, Artificial Sequence
DIQMTQSPSSLSASVGDRVTITCLASEDIYSYLAWYQQKPGKAPKLLIFAANRLQSGVPSRFSGSGSGTDFTLTISSLQPEDFATYYCLQGSKFPYTFGPGTKVDIKRTVAAPSVFIFPPSDEQLKSGTASVVCLLNNFYPREAKVQWKVDNALQSGNSQESVTEQDSKDSTYSLSSTLTLSKADYEKHKVYACEVTHQGLSSPVTKSFNRGECGGGGSGGGGSQVQLVQSGGGVVQPGRSLRLSCKASGYTFTRYTMHWVRQAPGKGLEWIGYINPSRGYTNYNQKVKDRFTISRDNSKNTAFLQMDSLRPEDTGVYFCARYYDDHYSLDYWGQGTPVTVSSGGGGSGGGGSGGGGSDIQMTQSPSSLSASVGDRVTITCSASSSVSYMNWYQQTPGKAPKRWIYDTSKLASGVPSRFSGSGSGTDYTFTISSLQPEDIATYYCQQWSSNPFTFGQGTKLQITR

SEQ ID NO: 200 - protein, 227 aa, Artificial Sequence
DKTHTCPPCPAPEAAGGPSVFLFPPKPKDTLMISRTPEVTCVVVDVSHEDPEVKFNWYVDGVEVHNAKTKPREEQYNSTYRVVSVLTVLHQDWLNGKEYKCKVSNKALPAPIEKTISKAKGQPREPQVCTLPPSREEMTKNQVSLSCAVKGFYPSDIAVEWESNGQPENNYKTTPPVLDSDGSFFLVSKLTVDKSRWQQGNVFSCSVMHEALHNHYTQKSLSLSPGK

SEQ ID NO: 201 - protein, 483 aa, Artificial Sequence
QVQLVQSGGGVVQPGRSLRLSCKASGYTFTRYTMHWVRQAPGKGLEWIGYINPSRGYTNYNQKVKDRFTISRDNSKNTAFLQMDSLRPEDTGVYFCARYYDDHYSLDYWGQGTPVTVSSGGGGSGGGGSGGGGSDIQMTQSPSSLSASVGDRVTITCSASSSVSYMNWYQQTPGKAPKRWIYDTSKLASGVPSRFSGSGSGTDYTFTISSLQPEDIATYYCQQWSSNPFTFGQGTKLQITRGGGGSGGGGSGGGGSDKTHTCPPCPAPEAAGGPSVFLFPPKPKDTLMISRTPEVTCVVVDVSHEDPEVKFNWYVDGVEVHNAKTKPREEQYNSTYRVVSVLTVLHQDWLNGKEYKCKVSNKALPAPIEKTISKAKGQPREPQVYTLPPCREEMTKNQVSLWCLVKGFYPSDIAVEWESNGQPENNYKTTPPVLDSDGSFFLYSKLTVDKSRWQQGNVFSCSVMHEALHNHYTQKSLSLSPGK

SEQ ID NO: 202 - protein, 465 aa, Artificial Sequence
DIQMTQSPSSLSASVGDRVTITCLASEDIYSYLAWYQQKPGKAPKLLIFAANRLQDGVPSRFSGSGSGTDFTLTISSLQPEDFATYYCLQGSKFPYTFGPGTKVDIKRTVAAPSVFIFPPSDEQLKSGTASVVCLLNNFYPREAKVQWKVDNALQSGNSQESVTEQDSKDSTYSLSSTLTLSKADYEKHKVYACEVTHQGLSSPVTKSFNRGECGGGGSGGGGSQVQLVQSGGGVVQPGRSLRLSCKASGYTFTRYTMHWVRQAPGKGLEWIGYINPSRGYTNYNQKVKDRFTISRDNSKNTAFLQMDSLRPEDTGVYFCARYYDDHYSLDYWGQGTPVTVSSGGGGSGGGGSGGGGSDIQMTQSPSSLSASVGDRVTITCSASSSVSYMNWYQQTPGKAPKRWIYDTSKLASGVPSRFSGSGSGTDYTFTISSLQPEDIATYYCQQWSSNPFTFGQGTKLQITR

SEQ ID NO: 203 - protein, 468 aa, Artificial Sequence
DIQMTQSPSSLSASVGDRVTITCLASEDIYSYLAWYQQKPGKAPKLLIFAANRLQDGVPSRFSGSGSGTDFTLTISSLQPEDFATYYCLQGSKFPYTFGPGTKVDIKGGGGSGGGGSGGGGSQVQLVQSGAEVKKPGSSVKVSCKASGYTFTRNFIHWIRQAPGQGLEWIGWIFPGDADTEYNQKFSGRATITADKSTSTAYMELSSLRSEDTAVYYCARGNYNYEYFDYWGQGTMVTVSSDKTHTCPPCPAPEAAGGPSVFLFPPKPKDTLMISRTPEVTCVVVDVSHEDPEVKFNWYVDGVEVHNAKTKPREEQYNSTYRVVSVLTVLHQDWLNGKEYKCKVSNKALPAPIEKTISKAKGQPREPQVCTLPPSREEMTKNQVSLSCAVKGFYPSDIAVEWESNGQPENNYKTTPPVLDSDGSFFLVSKLTVDKSRWQQGNVFSCSVMHEALHNHYTQKSLSLSPGK

SEQ ID NO: 204 - protein, 119 aa, Artificial Sequence
QVQLVQSGGGVVQPGRSLRLSCKASGYTFTRYTMHWVRQAPGKGLEWIGYINPSRGYTNYNQKVKDRFTISRDNSKNTAFLQMDSLRPEDTGVYFCARYYNDHYSLDYWGQGTPVTVSS

SEQ ID NO: 205 - protein, 119 aa, Artificial Sequence
QVQLVQSGGGVVQPGRSLRLSCKASGYTFTRYTMHWVRQAPGKGLEWIGYINPSRGYTNYNQKVKDRFTISRDNSKNTAFLQMDSLRPEDTGVYFCARYYDDHFSLDYWGQGTPVTVSS

SEQ ID NO: 206 - protein, 119 aa, Artificial Sequence
QVQLVQSGGGVVQPGRSLRLSCKASGYTFTRYTMHWVRQAPGKGLEWIGYINPSMGATNYNQKVKDRFTISRDNSKNTAFLQMDSLRPEDTGVYFCARYYDDHYSLDYWGQGTPVTVSS

SEQ ID NO: 207 - protein, 107 aa, Artificial Sequence
DIQMTQSPSSLSASVGDRVTITCSASSSVAYMNWYQQTPGKAPKRWIYDTSKLASGVPSRFSGSGSGTDYTFTISSLQPEDIATYYCQQWSSNPFTFGQGTKLQITR

SEQ ID NO: 208 - protein, 107 aa, Artificial Sequence
DIQMTQSPSSLSASVGDRVTITCSASSSVSYMNWYQQTPGKAPKRWIYNTSKLASGVPSRFSGSGSGTDYTFTISSLQPEDIATYYCQQWSSNPFTFGQGTKLQITR

SEQ ID NO: 209 - protein, 217 aa, Artificial Sequence
APEAAGGPSVFLFPPKPKDTLMISRTPEVTCVVVDVSHEDPEVKFNWYVDGVEVHNAKTKPREEQYNSTYRVVSVLTVLHQDWLNGKEYKCKVSNKALPAPIEKTISKAKGQPREPQVCTLPPSREEMTKNQVSLSCAVKGFYPSDIAVEWESNGQPENNYKTTPPVLDSDGSFFLVSKLTVDKSRWQQGNVFSCSVMHEALHNHYTQKSLSLSPGK

SEQ ID NO: 210 - protein, 217 aa, Artificial Sequence
APEAAGGPSVFLFPPKPKDTLMISRTPEVTCVVVDVSHEDPEVKFNWYVDGVEVHNAKTKPREEQYNSTYRVVSVLTVLHQDWLNGKEYKCKVSNKALPAPIEKTISKAKGQPREPQVYTLPPCREEMTKNQVSLWCLVKGFYPSDIAVEWESNGQPENNYKTTPPVLDSDGSFFLYSKLTVDKSRWQQGNVFSCSVMHEALHNHYTQKSLSLSPGK

SEQ ID NO: 211 - protein, 217 aa, Artificial Sequence
APEAAGGPSVFLFPPKPKDTLMISRTPEVTCVVVDVSHEDPEVKFNWYVDGVEVHNAKTKPREEQYNSTYRVVSVLTVLHQDWLNGKEYKCKVSNKALPAPIEKTISKAKGQPREPQVYTLPPSREEMTKNQVSLTCLVKGFYPSDIAVEWESNGQPENNYKTTPPVLDSDGSFFLYSKLTVDKSRWQQGNVFSCSVMHEALHNHYTQKSLSLSPGK

SEQ ID NO: 212 - protein, 695 aa, Artificial Sequence
QVQLVQSGAEVKKPGSSVKVSCKASGYTFTRNFIHWIRQAPGQGLEWIGWIFPGDADTEYNQKFSGRVTITADKSTSTAYMELSSLRSEDTAVYYCARGNYNYEYFDYWGQGTMVTVSSASTKGPSVFPLAPSSKSTSGGTAALGCLVKDYFPEPVTVSWNSGALTSGVHTFPAVLQSSGLYSLSSVVTVPSSSLGTQTYICNVNHKPSNTKVDKRVEPKSCGGGGSQVQLVQSGGGVVQPGRSLRLSCKASGYTFTRYTMHWVRQAPGKGLEWIGYINPSRGYTNYNQKVKDRFTISRDNSKNTAFLQMDSLRPEDTGVYFCARYYDDHYSLDYWGQGTPVTVSSGGGGSGGGGSGGGGSDIQMTQSPSSLSASVGDRVTITCSASSSVSYMNWYQQTPGKAPKRWIYDTSKLASGVPSRFSGSGSGTDYTFTISSLQPEDIATYYCQQWSSNPFTFGQGTKLQITRDKTHTCPPCPAPEAAGGPSVFLFPPKPKDTLMISRTPEVTCVVVDVSHEDPEVKFNWYVDGVEVHNAKTKPREEQYNSTYRVVSVLTVLHQDWLNGKEYKCKVSNKALPAPIEKTISKAKGQPREPQVYTLPPCREEMTKNQVSLWCLVKGFYPSDIAVEWESNGQPENNYKTTPPVLDSDGSFFLYSKLTVDKSRWQQGNVFSCSVMHEALHNHYTQKSLSLSPGK